European Patent Specification EP 3 578 557 B1, published September 20, 2023. Title: CHEMICAL PROCESS FOR PREPARING SPIROINDOLONES AND INTERMEDIATES THEREOF. Applicant: Novartis AG CROWE, Michael FOULKES, Michael FRANCESE, Giancarlo GRIMLER, Dominique KUESTERS, Ernst LAUMEN, Kurt LI, Yunzhong LIN, Changxue NAZOR, Jovana RUCH, Thomas SMITH, Derek SONG, Shiwei TENG, Shangjun. The sequence listing filed with the application follows.

SEQUENCE LISTING (154 sequences)

SEQ ID NO: 1 - DNA, 1362 bp, Artificial Sequence
  Codon optimized transaminase gene from Vibrio fluvialis
atgaacaaaccgcagagctgggaagcgcgtgcggaaacctatagcctgtatggctttaccgatatgccgagcctgcatcagcgtggcaccgtggtggtgacccatggcgaaggcccgtatatcgtggatgtgaacggccgtcgttatctggatgcgaacagcggcctgtggaacatggtggcgggctttgatcataaaggcctgattgatgcggcgaaagcgcagtatgaacgttttccgggctatcatgcgttttttggccgtatgagcgatcagaccgtgatgctgtctgaaaaactggtggaagtgagcccgtttgatagcggccgtgtgttttataccaacagcggcagcgaagcgaacgataccatggtgaaaatgctgtggtttctgcatgcggcggaaggcaaaccgcagaaacgtaaaattctgacccgttggaacgcgtatcatggcgtgaccgcggtgagcgcgagcatgaccggcaaaccgtataacagcgtgtttggcctgccgctgccgggctttgtgcatctgacctgcccgcattattggcgttatggcgaagaaggcgaaaccgaagaacagtttgtggcgcgtctggcccgtgaactggaagaaaccattcagcgtgaaggcgcggataccattgcgggcttttttgcggaaccggtgatgggtgcgggcggtgttattccgccggcgaaaggctattttcaggcgattctgccgatcctgcgcaaatatgatattccggtgatcagcgatgaagtgatttgcggctttggccgtaccggcaacacctggggctgcgtgacctatgattttaccccggatgcgattattagcagcaaaaacctgaccgcgggtttttttccgatgggcgcggtgattctgggtccggaactgagcaaacgtctggaaaccgcgattgaagcgatcgaagaatttccgcatggttttaccgcgagcggccatccggtgggttgtgcgattgcgctgaaagcgattgatgtggtgatgaacgaaggcctggccgaaaacgtgcgtcgtctggccccgcgttttgaagaacgtctgaaacatattgcggaacgtccgaacattggcgaatatcgtggcattggctttatgtgggcgctggaagcggtgaaagataaagcgagcaaaaccccgtttgatggcaacctgagcgtgagcgaacgtattgcgaacacctgcaccgatctgggcctgatttgccgtccgctgggccagagcgtggttctgtgcccgccgtttattctgaccgaagcgcagatggatgaaatgttcgataaactggaaaaagcgctggataaagtgtttgcggaagtggcgtaa

SEQ ID NO: 2 - protein, 453 aa, Vibrio fluvialis
MNKPQSWEARAETYSLYGFTDMPSLHQRGTVVVTHGEGPYIVDVNGRRYLDANSGLWNMVAGFDHKGLIDAAKAQYERFPGYHAFFGRMSDQTVMLSEKLVEVSPFDSGRVFYTNSGSEANDTMVKMLWFLHAAEGKPQKRKILTRWNAYHGVTAVSASMTGKPYNSVFGLPLPGFVHLTCPHYWRYGEEGETEEQFVARLARELEETIQREGADTIAGFFAEPVMGAGGVIPPAKGYFQAILPILRKYDIPVISDEVICGFGRTGNTWGCVTYDFTPDAIISSKNLTAGFFPMGAVILGPELSKRLETAIEAIEEFPHGFTASGHPVGCAIALKAIDVVMNEGLAENVRRLAPRFEERLKHIAERPNIGEYRGIGFMWALEAVKDKASKTPFDGNLSVSERIANTCTDLGLICRPLGQSVVLCPPFILTEAQMDEMFDKLEKALDKVFAEVA

SEQ ID NO: 3 - DNA, 1362 bp, Artificial Sequence
  Engineered variant of V. fluvialis transaminase
atgaacaaaccgcagagctgggaaacgcgtgcggaaacctatagcctgtatgcctttacccacatgccgagcctacatcagcgtggcaccatggtggtgacccatggcgaaggcccgtatatcgtggatgtgcatggccgtcgttatctggatgcgaacagcggcctgtggaacatggtggcgggctttgatcataaaggcctgattgatgcggcgaaagcgcagtatgaacgttttccgggctatcatgcgttttacggccgtatgagcgatcagaccgtgatgctgtctgaaaaactggtggaagtgagcccgtttgatagcggccgtgtgttttataccaacagcggcagcgaagcgaacgataccatggtgaaaatgctgtggtttctgcatcgtgcggaaggcaaaccgcagaaacgtaaaattctgaccctgaagaacgcgtatcatggctccaccgcggtgagcgcgagcatgaccggctttccgtataacagcgtgtttggcctgccgctgccgggctttctgcatctgacctgcccgcattattggcgttatggcgaagaaggcgaaaccgaagaacagtttgtcgcgcgtctggcccgtgaactggaagaaaccattcagaaggaaggcgcggataccattgcgggcttttttgcggaaccggtgatgggtgcgggcggtgttattaccccgccaaaaggctattttcaggcgattctgaccatcctgcgcaaatatgatattccggtgatcagcgatgaagtgatttgcggctttggtcgtaccggcaacacctggggctgcgtgacctatgattttaccccggatgcgattattagcagtaaaaacctaaccgcgggtttttttccagtaggagcggtgattttggggccggaactgagcaaacgtctggaaaccgcgattgaagcgatcgaagaatttgatcatggttttaccacaggcggccatccggtgggttgtgcgattgcgctgaaagcgattgatgtggtgatgaacgaaggcctggccgaaaacgtgcgtcgtctggccccgcgttttgaagaacgtctgaaacatattgcggaacgtccgaacattggcgaatatcgtggtattggctttatgtgggcgctggaagtggtgaaagataaagcgagcaaagccccgtttgatggcaacctgagcgtgagcgaacgtattgcgaacacctgcaccgatctgggactgatttgccgaccgttgggccagagcgtggttctggcaccgccgtacattctgaccgaagcgcagatggatgaaatgttcgataaactggaaaaagcgctggataaagtgtttgcggaagtggcgtaa

SEQ ID NO: 4 - protein, 453 aa, Artificial Sequence
  Engineered variant of V. fluvialis transaminase
MNKPQSWETRAETYSLYAFTHMPSLHQRGTMVVTHGEGPYIVDVHGRRYLDANSGLWNMVAGFDHKGLIDAAKAQYERFPGYHAFYGRMSDQTVMLSEKLVEVSPFDSGRVFYTNSGSEANDTMVKMLWFLHRAEGKPQKRKILTLKNAYHGSTAVSASMTGFPYNSVFGLPLPGFLHLTCPHYWRYGEEGETEEQFVARLARELEETIQKEGADTIAGFFAEPVMGAGGVITPPKGYFQAILTILRKYDIPVISDEVICGFGRTGNTWGCVTYDFTPDAIISSKNLTAGFFPVGAVILGPELSKRLETAIEAIEEFDHGFTTGGHPVGCAIALKAIDVVMNEGLAENVRRLAPRFEERLKHIAERPNIGEYRGIGFMWALEVVKDKASKAPFDGNLSVSERIANTCTDLGLICRPLGQSVVLAPPYILTEAQMDEMFDKLEKALDKVFAEVA

SEQ ID NO: 5 - DNA, 1362 bp, Artificial Sequence
  Engineered variant of V. fluvialis transaminase
atgaacaaaccgcagagctgggaaacgcgtgcggaaacctatagcctgtatgcctttacccacatgccgagcctacatcagcgtggcaccatggtggtgacccatggcgaaggcccgtatatcgtggatgtgcatggccgtcgttatctggatgcgaacagcggcctgtggaacatggtggcgggctttgatcataaaggcctgattgatgcggcgaaagcgcagtatgaacgttttccgggctatcatgcgttttacggccgtatgagcgatcagaccgtgatgctgtctgaaaaactggtggaagtgagcccgtttgatagcggccgtgtgttttataccaacagcggcagcgaagcgaacgataccatggtgaaaatgctgtggtttctgcatcgtgcggaaggcaaaccgcagaaacgtaaaattctgaccctgaagaacgcgtatcatggctccaccgcggtgagcgcgagcatgaccggccttccgtataacagcgtgtttggcctgccgctgccgggctttctgcatctgacctgcccgcattattggcgttatggcgaagaaggcgaaaccgaagaacagtttgtcgcgcgtctggcccgtgaactggaagaaaccattcagaaggaaggcgcggataccattgcgggcttttttgcggaaccggtgatgggtgcgggcggtgttattaccccgccaaaaggctattttcaggcgattctgaccatcctgcgcaaatatgatattccggtgatcagcgatgaagtgatttgcggctttggtcgtaccggcaacacctggggctgcgtgacctatgattttaccccggatgcgattattagcagtaaaaacctaaccgcgggtttttttccagtaggagcggtgattttggggccggaactgagcaaacgtctggaaaccgcgattgaagcgatcgaagaatttgatcatggttttaccacaggcggccatccggtgggttgtgcgattgcgctgaaagcgattgatgtggtgatgaacgaaggcctggccgaaaacgtgcgtcgtctggccccgcgttttgaagaacgtctgaaacatattgcggaacgtccgaacattggcgaatatcgtggtattggctttatgtgggcgctggaagtggtgaaagataaagcgagcaaagccccgtttgatggcaacctgagcgtgagcgaacgtattgcgaacacctgcaccgatctgggactgatttgccgaccgttgggccagagcgtggttctggcaccgccgtacattctgaccgaagcgcagatggatgaaatgttcgataaactggaaaaagcgctggataaagtgtttgcggaagtggcgtaa

SEQ ID NO: 6 - protein, 453 aa, Artificial Sequence
  Engineered variant of V. fluvialis transaminase
MNKPQSWETRAETYSLYAFTHMPSLHQRGTMVVTHGEGPYIVDVHGRRYLDANSGLWNMVAGFDHKGLIDAAKAQYERFPGYHAFYGRMSDQTVMLSEKLVEVSPFDSGRVFYTNSGSEANDTMVKMLWFLHRAEGKPQKRKILTLKNAYHGSTAVSASMTGLPYNSVFGLPLPGFLHLTCPHYWRYGEEGETEEQFVARLARELEETIQKEGADTIAGFFAEPVMGAGGVITPPKGYFQAILTILRKYDIPVISDEVICGFGRTGNTWGCVTYDFTPDAIISSKNLTAGFFPVGAVILGPELSKRLETAIEAIEEFDHGFTTGGHPVGCAIALKAIDVVMNEGLAENVRRLAPRFEERLKHIAERPNIGEYRGIGFMWALEVVKDKASKAPFDGNLSVSERIANTCTDLGLICRPLGQSVVLAPPYILTEAQMDEMFDKLEKALDKVFAEVA

SEQ ID NO: 7 - DNA, 1362 bp, Artificial Sequence
  Engineered variant of V. fluvialis transaminase
atgaacaaaccgcagagctgggaaacgcgtgcggaaacctatagcctgtatgcctttacccacatgccgagcctacatcagcgtggcaccatggtggtgacccatggcgaaggcccgtatatcgtggatgtgcatggccgtcgttatctggatgcgaacagcggcctgtggaacatggtggcgggctttgatcataaaggcctgattgatgcggcgaaagcgcagtatgaacgttttccgggctatcatgcgttttacggccgtatgagcgatcagaccgtgatgctgtctgaaaaactggtggaagtgagcccgtttgatagcggccgtgtgttttataccaacagcggcagcgaagcgaacgataccatggtgaaaatgctgtggtttctgcatcgtgcggaaggcaaaccgcagaaacgtaaaattctgaccctgaagaacgcgtatcatggctccaccgcggtgagcgcgagcatgaccggcattccgtataacagcgtgtttggcctgccgctgccgggctttctgcatctgacctgcccgcattattggcgttatggcgaagaaggcgaaaccgaagaacagtttgtcgcgcgtctggcccgtgaactggaagaaaccattcagaaggaaggcgcggataccattgcgggcttttttgcggaaccggtgatgggtgcgggcggtgttattaccccgccaaaaggctattttcaggcgattctgaccatcctgcgcaaatatgatattccggtgatcagcgatgaagtgatttgcggctttggtcgtaccggcaacacctggggctgcgtgacctatgattttaccccggatgcgattattagcagtaaaaacctaaccgcgggtttttttccagtaggagcggtgattttggggccggaactgagcaaacgtctggaaaccgcgattgaagcgatcgaagaatttgatcatggttttaccacaggcggccatccggtgggttgtgcgattgcgctgaaagcgattgatgtggtgatgaacgaaggcctggccgaaaacgtgcgtcgtctggccccgcgttttgaagaacgtctgaaacatattgcggaacgtccgaacattggcgaatatcgtggtattggctttatgtgggcgctggaagtggtgaaagataaagcgagcaaagccccgtttgatggcaacctgagcgtgagcgaacgtattgcgaacacctgcaccgatctgggactgatttgccgaccgttgggccagagcgtggttctggcaccgccgtacattctgaccgaagcgcagatggatgaaatgttcgataaactggaaaaagcgctggataaagtgtttgcggaagtggcgtaa

SEQ ID NO: 8 - protein, 453 aa, Artificial Sequence
  Engineered variant of V. fluvialis transaminase
MNKPQSWETRAETYSLYAFTHMPSLHQRGTMVVTHGEGPYIVDVHGRRYLDANSGLWNMVAGFDHKGLIDAAKAQYERFPGYHAFYGRMSDQTVMLSEKLVEVSPFDSGRVFYTNSGSEANDTMVKMLWFLHRAEGKPQKRKILTLKNAYHGSTAVSASMTGIPYNSVFGLPLPGFLHLTCPHYWRYGEEGETEEQFVARLARELEETIQKEGADTIAGFFAEPVMGAGGVITPPKGYFQAILTILRKYDIPVISDEVICGFGRTGNTWGCVTYDFTPDAIISSKNLTAGFFPVGAVILGPELSKRLETAIEAIEEFDHGFTTGGHPVGCAIALKAIDVVMNEGLAENVRRLAPRFEERLKHIAERPNIGEYRGIGFMWALEVVKDKASKAPFDGNLSVSERIANTCTDLGLICRPLGQSVVLAPPYILTEAQMDEMFDKLEKALDKVFAEVA

SEQ ID NO: 9 - DNA, 1362 bp, Artificial Sequence
  Engineered variant of V. fluvialis transaminase
atgaacaaaccgcagagctgggaaacgcgtgcggaaacctatagcctgtatgcctttacccacatgccgagcctacatcagcgtggcaccatggtggtgacccatggcgaaggcccgtatatcgtggatgtgcatggccgtcgttatctggatgcgaacagcggcctgtggaacatggtggcgggctttgatcataaaggcctgattgatgcggcgaaagcgcagtatgaacgttttccgggctatcatgcgttttacggccgtatgagcgatcagaccgtgatgctgtctgaaaaactggtggaagtgagcccgtttgatagcggccgtgtgttttataccaacagcggcagcgaagcgaacgataccatggtgaaaatgctgtggtttctgcatcgtgcggaaggcaaaccgcagaaacgtaaaattctgaccctgaagaacgcgtatcatggctccaccgcggtgagcgcgagcatgaccggccgtccgtataacagcgtgtttggcctgccgctgccgggctttctgcatctgacctgcccgcattattggcgttatggcgaagaaggcgaaaccgaagaacagtttgtcgcgcgtctggcccgtgaactggaagaaaccattcagaaggaaggcgcggataccattgcgggcttttttgcggaaccggtgatgggtgcgggcggtgttattaccccgccaaaaggctattttcaggcgattctgaccatcctgcgcaaatatgatattccggtgatcagcgatgaagtgatttgcggctttggtcgtaccggcaacacctggggctgcgtgacctatgattttaccccggatgcgattattagcagtaaaaacctaaccgcgggtttttttccagtaggagcggtgattttggggccggaactgagcaaacgtctggaaaccgcgattgaagcgatcgaagaatttgatcatggttttaccacaggcggccatccggtgggttgtgcgattgcgctgaaagcgattgatgtggtgatgaacgaaggcctggccgaaaacgtgcgtcgtctggccccgcgttttgaagaacgtctgaaacatattgcggaacgtccgaacattggcgaatatcgtggtattggctttatgtgggcgctggaagtggtgaaagataaagcgagcaaagccccgtttgatggcaacctgagcgtgagcgaacgtattgcgaacacctgcaccgatctgggactgatttgccgaccgttgggccagagcgtggttctggcaccgccgtacattctgaccgaagcgcagatggatgaaatgttcgataaactggaaaaagcgctggataaagtgtttgcggaagtggcgtaa

SEQ ID NO: 10 - protein, 453 aa, Artificial Sequence
  Engineered variant of V. fluvialis transaminase
MNKPQSWETRAETYSLYAFTHMPSLHQRGTMVVTHGEGPYIVDVHGRRYLDANSGLWNMVAGFDHKGLIDAAKAQYERFPGYHAFYGRMSDQTVMLSEKLVEVSPFDSGRVFYTNSGSEANDTMVKMLWFLHRAEGKPQKRKILTLKNAYHGSTAVSASMTGRPYNSVFGLPLPGFLHLTCPHYWRYGEEGETEEQFVARLARELEETIQKEGADTIAGFFAEPVMGAGGVITPPKGYFQAILTILRKYDIPVISDEVICGFGRTGNTWGCVTYDFTPDAIISSKNLTAGFFPVGAVILGPELSKRLETAIEAIEEFDHGFTTGGHPVGCAIALKAIDVVMNEGLAENVRRLAPRFEERLKHIAERPNIGEYRGIGFMWALEVVKDKASKAPFDGNLSVSERIANTCTDLGLICRPLGQSVVLAPPYILTEAQMDEMFDKLEKALDKVFAEVA

SEQ ID NO: 11 - DNA, 1362 bp, Artificial Sequence
  Engineered variant of V. fluvialis transaminase
atgaacaaaccgcagagctgggaaacgcgtgcggaaacctatagcctgtatgcctttacccacatgccgagcctacatcagcgtggcaccatggtggtgacccatggcgaaggcccgtatatcgtggatgtgcatggccgtcgttatctggatgcgaacagcggcctgtggaacatggtggcgggctttgatcataaaggcctgattgatgcggcgaaagcgcagtatgaacgttttccgggctatcatgcgtttgatggccgtatgagcgatcagaccgtgatgctgtctgaaaaactggtggaagtgagcccgtttgatagcggccgtgtgttttataccaacagcggcagcgaagcgaacgataccatggtgaaaatgctgtggtttctgcatcgtgcggaaggcaaaccgcagaaacgtaaaattctgaccctgaagaacgcgtatcatggctccaccgcggtgagcgcgagcatgaccggctttccgtataacagcgtgtttggcctgccgctgccgggctttctgcatctgacctgcccgcattattggcgttatggcgaagaaggcgaaaccgaagaacagtttgtcgcgcgtctggcccgtgaactggaagaaaccattcagaaggaaggcgcggataccattgcgggcttttttgcggaaccggtgatgggtgcgggcggtgttattaccccgccaaaaggctattttcaggcgattctgaccatcctgcgcaaatatgatattccggtgatcagcgatgaagtgatttgcggctttggtcgtaccggcaacacctggggctgcgtgacctatgattttaccccggatgcgattattagcagtaaaaacctaaccgcgggtttttttccagtaggagcggtgattttggggccggaactgagcaaacgtctggaaaccgcgattgaagcgatcgaagaatttgatcatggttttaccacaggcggccatccggtgggttgtgcgattgcgctgaaagcgattgatgtggtgatgaacgaaggcctggccgaaaacgtgcgtcgtctggccccgcgttttgaagaacgtctgaaacatattgcggaacgtccgaacattggcgaatatcgtggtattggctttatgtgggcgctggaagtggtgaaagataaagcgagcaaagccccgtttgatggcaacctgagcgtgagcgaacgtattgcgaacacctgcaccgatctgggactgatttgccgaccgttgggccagagcgtggttctggcaccgccgtacattctgaccgaagcgcagatggatgaaatgttcgataaactggaaaaagcgctggataaagtgtttgcggaagtggcgtaa

SEQ ID NO: 12 - protein, 453 aa, Artificial Sequence
  Engineered variant of V. fluvialis transaminase
MNKPQSWETRAETYSLYAFTHMPSLHQRGTMVVTHGEGPYIVDVHGRRYLDANSGLWNMVAGFDHKGLIDAAKAQYERFPGYHAFDGRMSDQTVMLSEKLVEVSPFDSGRVFYTNSGSEANDTMVKMLWFLHRAEGKPQKRKILTLKNAYHGSTAVSASMTGFPYNSVFGLPLPGFLHLTCPHYWRYGEEGETEEQFVARLARELEETIQKEGADTIAGFFAEPVMGAGGVITPPKGYFQAILTILRKYDIPVISDEVICGFGRTGNTWGCVTYDFTPDAIISSKNLTAGFFPVGAVILGPELSKRLETAIEAIEEFDHGFTTGGHPVGCAIALKAIDVVMNEGLAENVRRLAPRFEERLKHIAERPNIGEYRGIGFMWALEVVKDKASKAPFDGNLSVSERIANTCTDLGLICRPLGQSVVLAPPYILTEAQMDEMFDKLEKALDKVFAEVA

SEQ ID NO: 13 - DNA, 1362 bp, Artificial Sequence
  Engineered variant of V. fluvialis transaminase
atgaacaaaccgcagagctgggaaacgcgtgcggaaacctatagcctgtatgcctttacccacatgccgagcctacatcagcgtggcaccatggtggtgacccatggcgaaggcccgtatatcgtggatgtgcatggccgtcgttatctggatgcgaacagcggcctgtggaacatggtggcgggctttgatcataaaggcctgattgatgcggcgaaagcgcagtatgaacgttttccgggctatcatgcgttttacggccgtatgagcgatcagaccgtgatgctgtctgaaaaactggtggaagtgagcccgtttgatagcggccgtgtgttttataccaacagcggcagcgaagcgaacgataccatggtgaaaatgctgtggtttctgcatcgtgcggaaggcaaaccgcagaaacgtaaaattctgaccctgaagaacgcgtatcatggctccaccgcggtgagcgcgagcatgaccggcgtgccgtataacagcgtgtttggcctgccgctgccgggctttctgcatctgacctgcccgcattattggcgttatggcgaagaaggcgaaaccgaagaacagtttgtcgcgcgtctggcccgtgaactggaagaaaccattcagaaggaaggcgcggataccattgcgggcttttttgcggaaccggtgatgggtgcgggcggtgttattaccccgccaaaaggctattttcaggcgattctgaccatcctgcgcaaatatgatattccggtgatcagcgatgaagtgatttgcggctttggtcgtaccggcaacacctggggctgcgtgacctatgattttaccccggatgcgattattagcagtaaaaacctaaccgcgggtttttttccagtaggagcggtgattttggggccggaactgagcaaacgtctggaaaccgcgattgaagcgatcgaagaatttgatcatggttttaccacaggcggccatccggtgggttgtgcgattgcgctgaaagcgattgatgtggtgatgaacgaaggcctggccgaaaacgtgcgtcgtctggccccgcgttttgaagaacgtctgaaacatattgcggaacgtccgaacattggcgaatatcgtggtattggctttatgtgggcgctggaagtggtgaaagataaagcgagcaaagccccgtttgatggcaacctgagcgtgagcgaacgtattgcgaacacctgcaccgatctgggactgatttgccgaccgttgggccagagcgtggttctggcaccgccgtacattctgaccgaagcgcagatggatgaaatgttcgataaactggaaaaagcgctggataaagtgtttgcggaagtggcgtaa

SEQ ID NO: 14 - protein, 453 aa, Artificial Sequence
  Engineered variant of V. fluvialis transaminase
MNKPQSWETRAETYSLYAFTHMPSLHQRGTMVVTHGEGPYIVDVHGRRYLDANSGLWNMVAGFDHKGLIDAAKAQYERFPGYHAFYGRMSDQTVMLSEKLVEVSPFDSGRVFYTNSGSEANDTMVKMLWFLHRAEGKPQKRKILTLKNAYHGSTAVSASMTGVPYNSVFGLPLPGFLHLTCPHYWRYGEEGETEEQFVARLARELEETIQKEGADTIAGFFAEPVMGAGGVITPPKGYFQAILTILRKYDIPVISDEVICGFGRTGNTWGCVTYDFTPDAIISSKNLTAGFFPVGAVILGPELSKRLETAIEAIEEFDHGFTTGGHPVGCAIALKAIDVVMNEGLAENVRRLAPRFEERLKHIAERPNIGEYRGIGFMWALEVVKDKASKAPFDGNLSVSERIANTCTDLGLICRPLGQSVVLAPPYILTEAQMDEMFDKLEKALDKVFAEVA

SEQ ID NO: 15 - DNA, 1362 bp, Artificial Sequence
  Engineered variant of V. fluvialis transaminase
atgaacaaaccgcagagctgggaaacgcgtgcggaaaccgtgagcctgtatgcctttacccacatgccgagcctacgtcagcgtggcaccatggtggtgacccatggcgaaggcccgtatatcgtggatgtgcatggccgtcgttatctggatgcgaacagcggcctgtggaacatggtggcgggctttgatcataaaggcctgattgatgcggcgaaagcgcagtatgaacgttttccgggctatcatgcgttttacggcctgatgagcgatcagaccgtgatgctgtctgaaaaactggtggaagtgagcccgtttgatagcggccgtgtgtttctgaccaacagcggcagcgaagcgaacgataccatggtgaaaatgctgtggtttctgcatcgtgcggaaggcaaaccgcagaaacgtaaaattctgaccctgaagaacgcgtatcatggctccaccgcggtgagcgcgagcatgaccggccttccgtataacagcgtgtttggcctgccgctgccgggctttctgcatctgacctgcccgcattattggcgttatggcgaagaaggcgaaaccgaagaacagtttgtcgcgcgtctggcccgtgaactggaagaaaccattcagaaggaaggcgcggataccattgcgggcttttttgcggaaccggtgatgggtgcgggcggtgttattaccccgccaaaaggctattttcaggcgattctgaccatcctgcgcaaatatgatattccggtgatcagcgatgaagtgatttgcggctttggtcgtaccggcaacacctggggctgcgtgacctatgattttaccccggatgcgattattagcagtaaaaacctaaccgcgggtttttttccagtaggagcggtgattttggggccggaactgagcaaacgtctggaaaccgcgattgaagcgatcgaagaatttgatcatggttttaccacaggcggccatccggtgggttgtgcgattgcgctgaaagcgattgatgtggtgatgaacgaaggcctggccgaaaacgtgcgtcgtctggccccgcgttttgaagaacgtctgaaacatattgcggaacgtccgaacattggcgaatatcgtggtattggctttatgtgggcgctggaagtggtgaaagataaagcgagcaaagccccgtttgatggcaacctgagcgtgagcgaacgtattgcgaacacctgcaccgatctgggactgatttgccgaccgttgggccagagcgtggttctggcaccgccgtacattctgaccgaagcgcagatggatgaaatgttcgataaactggaaaaagcgctggataaagtgtttgcggaagtggcgtaa

SEQ ID NO: 16 - protein, 453 aa, Artificial Sequence
  Engineered variant of V. fluvialis transaminase
MNKPQSWETRAETVSLYAFTHMPSLRQRGTMVVTHGEGPYIVDVHGRRYLDANSGLWNMVAGFDHKGLIDAAKAQYERFPGYHAFYGLMSDQTVMLSEKLVEVSPFDSGRVFLTNSGSEANDTMVKMLWFLHRAEGKPQKRKILTLKNAYHGSTAVSASMTGLPYNSVFGLPLPGFLHLTCPHYWRYGEEGETEEQFVARLARELEETIQKEGADTIAGFFAEPVMGAGGVITPPKGYFQAILTILRKYDIPVISDEVICGFGRTGNTWGCVTYDFTPDAIISSKNLTAGFFPVGAVILGPELSKRLETAIEAIEEFDHGFTTGGHPVGCAIALKAIDVVMNEGLAENVRRLAPRFEERLKHIAERPNIGEYRGIGFMWALEVVKDKASKAPFDGNLSVSERIANTCTDLGLICRPLGQSVVLAPPYILTEAQMDEMFDKLEKALDKVFAEVA

SEQ ID NO: 17 - DNA, 1362 bp, Artificial Sequence
  Engineered variant of V. fluvialis transaminase
atgaacaaaccgcagagctgggaaacgcgtgcggaaaccgtgagcctgtatgcctttacccacatgccgagcctacgtcagcgtggcaccatggtggtgacccatggcgaaggcccgtatatcgtggatgtgcatggccgtcgttatctggatgcgaacagcggcctgttcaacatggtggcgggctttgatcataaaggcctgattgatgcggcgaaagcgcagtatgaacgttttccgggctatcatgcgttttacggccgtatgagcgatcagaccgtgatgctgtctgaaaaactggtggaagtgagcccgtttgatagcggccgtgtgttttataccaacagcggcagcgaagcgaacgataccatggtgaaaatgctgtggtttctgcatcgtgcggaaggcaaaccgcagaaacgtaaaattctgaccctgaagaacgcgtatcatggctccaccgcggtgagcgcgagcatgaccggccttccgtataacagcgtgtttggcctgccgctgccgggctttctgcatctgacctgcccgcattattggcgttatggcgaagaaggcgaaaccgaagaacagtttgtcgcgcgtctggcccgtgaactggaagaaaccattcagaaggaaggcgcggataccattgcgggcttttttgcggaaccggtgatgggtgcgggcggtgttattaccccgccaaaaggctattttcaggcgattctgaccatcctgcgcaaatatgatattccggtgatcagcgatgaagtgatttgcggctttggtcgtaccggcaacacctggggctgcgtgacctatgattttaccccggatgcgattattagcagtaaaaacctaaccgcgggtttttttccagtaggagcggtgattttggggccggaactgagcaaacgtctggaaaccgcgattgaagcgatcgaagaatttgatcatggttttaccacaggcggccatccggtgggttgtgcgattgcgctgaaagcgattgatgtggtgatgaacgaaggcctggccgaaaacgtgcgtcgtctggccccgcgttttgaagaacgtctgaaacatattgcggaacgtccgaacattggcgaatatcgtggtattggctttatgtgggcgctggaagtggtgaaagataaagcgagcaaagccccgtttgatggcaacctgagcgtgagcgaacgtattgcgaacacctgcaccgatctgggactgatttgccgaccgttgggccagagcgtggttctggcaccgccgtacattctgaccgaagcgcagatggatgaaatgttcgataaactggaaaaagcgctggataaagtgtttgcggaagtggcgtaa

SEQ ID NO: 18 - protein, 453 aa, Artificial Sequence
  Engineered variant of V. fluvialis transaminase
MNKPQSWETRAETVSLYAFTHMPSLRQRGTMVVTHGEGPYIVDVHGRRYLDANSGLFNMVAGFDHKGLIDAAKAQYERFPGYHAFYGRMSDQTVMLSEKLVEVSPFDSGRVFYTNSGSEANDTMVKMLWFLHRAEGKPQKRKILTLKNAYHGSTAVSASMTGLPYNSVFGLPLPGFLHLTCPHYWRYGEEGETEEQFVARLARELEETIQKEGADTIAGFFAEPVMGAGGVITPPKGYFQAILTILRKYDIPVISDEVICGFGRTGNTWGCVTYDFTPDAIISSKNLTAGFFPVGAVILGPELSKRLETAIEAIEEFDHGFTTGGHPVGCAIALKAIDVVMNEGLAENVRRLAPRFEERLKHIAERPNIGEYRGIGFMWALEVVKDKASKAPFDGNLSVSERIANTCTDLGLICRPLGQSVVLAPPYILTEAQMDEMFDKLEKALDKVFAEVA

SEQ ID NO: 19 - DNA, 1362 bp, Artificial Sequence
  Engineered variant of V. fluvialis transaminase
atgaacaaaccgcagagctgggaaacgcgtgcggaaaccgtgagcctgtatgcctttacccacatgccgagcctacatcagcgtggcaccatggtgaccacccatggcgaaggcccgtatatcgtggatgtgcatggccgtcgttatctggatgcgaacagcggcctgttcaacatggtggcgggctttgatcataaaggcctgattgatgcggcgaaagcgcagtatgaacgttttccgggctatcatgcgttttacggcctgatgagcgatcagaccgtgatgctgtctgaaaaactggtggaagtgagcccgtttgatagcggccgtgtgtttctgaccaacagcggcagcgaagcgaacgataccatggtgaaaatgctgtggtttctgcatcgtgcggaaggcaaaccgcagaaacgtaaaattctgaccctgaagaacgcgtatcatggctccaccgcggtgagcgcgagcatgaccggccttccgtataacagcgtgtttggcctgccgctgccgggctttctgcatctgacctgcccgcattattggcgttatggcgaagaaggcgaaaccgaagaacagtttgtcgcgcgtctggcccgtgaactggaagaaaccattcagaaggaaggcgcggataccattgcgggcttttttgcggaaccggtgatgggtgcgggcggtgttattaccccgccaaaaggctattttcaggcgattctgaccatcctgcgcaaatatgatattccggtgatcagcgatgaagtgatttgcggctttggtcgtaccggcaacacctggggctgcgtgacctatgattttaccccggatgcgattattagcagtaaaaacctaaccgcgggtttttttccagtaggagcggtgattttggggccggaactgagcaaacgtctggaaaccgcgattgaagcgatcgaagaatttgatcatggttttaccacaggcggccatccggtgggttgtgcgattgcgctgaaagcgattgatgtggtgatgaacgaaggcctggccgaaaacgtgcgtcgtctggccccgcgttttgaagaacgtctgaaacatattgcggaacgtccgaacattggcgaatatcgtggtattggctttatgtgggcgctggaagtggtgaaagataaagcgagcaaagccccgtttgatggcaacctgagcgtgagcgaacgtattgcgaacacctgcaccgatctgggactgatttgccgaccgttgggccagagcgtggttctggcaccgccgtacattctgaccgaagcgcagatggatgaaatgttcgataaactggaaaaagcgctggataaagagtttgcggaagtggcgtaa

SEQ ID NO: 20 - protein, 453 aa, Artificial Sequence
  Engineered variant of V. fluvialis transaminase
MNKPQSWETRAETVSLYAFTHMPSLHQRGTMVTTHGEGPYIVDVHGRRYLDANSGLFNMVAGFDHKGLIDAAKAQYERFPGYHAFYGLMSDQTVMLSEKLVEVSPFDSGRVFLTNSGSEANDTMVKMLWFLHRAEGKPQKRKILTLKNAYHGSTAVSASMTGLPYNSVFGLPLPGFLHLTCPHYWRYGEEGETEEQFVARLARELEETIQKEGADTIAGFFAEPVMGAGGVITPPKGYFQAILTILRKYDIPVISDEVICGFGRTGNTWGCVTYDFTPDAIISSKNLTAGFFPVGAVILGPELSKRLETAIEAIEEFDHGFTTGGHPVGCAIALKAIDVVMNEGLAENVRRLAPRFEERLKHIAERPNIGEYRGIGFMWALEVVKDKASKAPFDGNLSVSERIANTCTDLGLICRPLGQSVVLAPPYILTEAQMDEMFDKLEKALDKEFAEVA

SEQ ID NO: 21 - DNA, 1362 bp, Artificial Sequence
  Engineered variant of V. fluvialis transaminase
atgaacaaaccgcagagctgggaaacgcgtgcggaaaccgtgagcctgtatgcctttacccacatgccgagcctacgtcagcgtggcaccatggtggtaacccatggcgaaggcccgtatatcgtggatgtgcatggccgtcgttatctggatgcgaacagcggcctgtggaacatggtggcgggctttgatcataaaggcctgattgatgcggcgaaagcgcagtatgaacgttttccgggctatcatgcgttttacggcgccatgagcgatcagaccgtgatgctgtctgaaaaactggtggaagtgagcccgtttgatagcggccgtgtgtttctgaccaacagcggcagcgaagcgaacgataccatggtgaaaatgctgtggtttctgcatcgtgcggaaggcaaaccgcagaaacgtaaaattctgaccctgaagcaggcgtatcatggctccaccgcggtgagcgcgagcatgaccggcatcccgtataacagcgtgtttggcctgccgctgccgggctttctgcatctgacctgcccgcattattggcgttatggcgaagaaggcgaaaccgaagaacagtttgtcgcgcgtctggccagtgaactggaagaaaccattcagaaggaaggcgcggataccattgcgggcttttttgcggaaccggtgatgggtgcgggcggtgttattaccccgccaaaaggctattttcaggcgattctgaccatcctgcgcaaatatgatattccggtgatcagcgatgaagtgatttgcggctttggtcgtaccggcaacacctggggctgcgtgacctatgattttaccccggatgcgattattagcagtaaaaacctaaccgcgggtttttttccagtaggagcggtgattttggggccggaactgagcaaacgtctggaaaccgcgattgaagcgatcgaagaatttgatcatggttttaccacaggcggccatccggtgggttgtgcgattgcgctgaaagcgattgatgtggtgatgaacgaaggcctggccgaaaacgtgcgtcgtctggccccgcgttttgaagaacgtctgaaacatattgcggaacgtccgaacattggcgaatatcgtggtattggctttatgtgggcgctggaagtggtgaaagataaagcgagcaaagccccgtttgatggcaacctgagcgtgagcgaacgtattgcgaacacctgcaccgatctgggactgatttgccgaccgttgggccagagcgtggttctggcaccgccgtacattctgaccgaagcgcagatggatgaaatgttcgataaactggaaaaagcgctggataaagtgtttgcggaagtggcgtaa

SEQ ID NO: 22 - protein, 453 aa, Artificial Sequence
  Engineered variant of V. fluvialis transaminase
MNKPQSWETRAETVSLYAFTHMPSLRQRGTMVVTHGEGPYIVDVHGRRYLDANSGLWNMVAGFDHKGLIDAAKAQYERFPGYHAFYGAMSDQTVMLSEKLVEVSPFDSGRVFLTNSGSEANDTMVKMLWFLHRAEGKPQKRKILTLKQAYHGSTAVSASMTGIPYNSVFGLPLPGFLHLTCPHYWRYGEEGETEEQFVARLASELEETIQKEGADTIAGFFAEPVMGAGGVITPPKGYFQAILTILRKYDIPVISDEVICGFGRTGNTWGCVTYDFTPDAIISSKNLTAGFFPVGAVILGPELSKRLETAIEAIEEFDHGFTTGGHPVGCAIALKAIDVVMNEGLAENVRRLAPRFEERLKHIAERPNIGEYRGIGFMWALEVVKDKASKAPFDGNLSVSERIANTCTDLGLICRPLGQSVVLAPPYILTEAQMDEMFDKLEKALDKVFAEVA

SEQ ID NO: 23 - DNA, 1362 bp, Artificial Sequence
  Engineered variant of V. fluvialis transaminase
atgaacaaaccgcagagctgggaaacgcgtgcggaaacctatagcctgtatgcctttacccacatgccgagcctacatcagcgtggcaccatggtggtgacccatggcgaaggcccgtatatcgtggatgtgcatggccgtcgttatctggatgcgaacagcggcctgttcaacatggtggcgggctttgatcataaaggcctgattgatgcggcgaaagcgcagtatgaacgttttccgggctatcatgcgttttacggcctgatgagcgatcagaccgtgatgctgtctgaaaaactggtggaagtgagcccgtttgatagcggccgtgtgtttctgaccaacagcggcagcgaagcgaacgataccatggtgaaaatgctgtggtttctgcatcgtgcggaaggcaaaccgcagaaacgtaaaattctgaccctgaagcaggcgtatcatggctccaccgcggtgagcgcgagcatgaccggcatcccgtataacagcgtgtttggcctgccgctgccgggctttctgcatctgacctgcccgcattattggcgttatggcgaagaaggcgaaaccgaagaacagtttgtcgcgcgtctggcccgtgaactggaagaaaccattcagaaggaaggcgcggataccattgcgggcttttttgcggaaccggtgatgggtgcgggcggtgttattaccccgccaaaaggctattttcaggcgattctgaccatcctgcgcaaatatgatattccggtgatcagcgatgaagtgatttgcggctttggtcgtaccggcaacacctggggctgcgtgacctatgattttaccccggatgcgattattagcagtaaaaacctaaccgcgggtttttttccagtaggagcggtgattttggggccggaactgagcaaacgtctggaaaccgcgattgaagcgatcgaagaatttgatcatggttttaccacaggcggccatccggtgggttgtgcgattgcgctgaaagcgattgatgtggtgatgaacgaaggcctggccgaaaacgtgcgtcgtctggccccgcgttttgaagaacgtctgaaacatattgcggaacgtccgaacattggcgaatatcgtggtattggctttatgtgggcgctggaagtggtgaaagataaagcgagcaaagccccgtttgatggcaacctgagcgtgagcgaacgtattgcgaacacctgcaccgatctgggactgatttgccgaccgttgggccagagcgtggttctggcaccgccgtacattctgaccgaagcgcagatggatgaaatgttcgataaactggaaaaagcgctggataaagagtttgcggaagtggcgtaa

SEQ ID NO: 24 - protein, 453 aa, Artificial Sequence
  Engineered variant of V. fluvialis transaminase
MNKPQSWETRAETYSLYAFTHMPSLHQRGTMVVTHGEGPYIVDVHGRRYLDANSGLFNMVAGFDHKGLIDAAKAQYERFPGYHAFYGLMSDQTVMLSEKLVEVSPFDSGRVFLTNSGSEANDTMVKMLWFLHRAEGKPQKRKILTLKQAYHGSTAVSASMTGIPYNSVFGLPLPGFLHLTCPHYWRYGEEGETEEQFVARLARELEETIQKEGADTIAGFFAEPVMGAGGVITPPKGYFQAILTILRKYDIPVISDEVICGFGRTGNTWGCVTYDFTPDAIISSKNLTAGFFPVGAVILGPELSKRLETAIEAIEEFDHGFTTGGHPVGCAIALKAIDVVMNEGLAENVRRLAPRFEERLKHIAERPNIGEYRGIGFMWALEVVKDKASKAPFDGNLSVSERIANTCTDLGLICRPLGQSVVLAPPYILTEAQMDEMFDKLEKALDKEFAEVA

SEQ ID NO: 25 - DNA, 1362 bp, Artificial Sequence
  Engineered variant of V. fluvialis transaminase
atgaacaaaccgcagagctgggaaacgcgtgcggaaaccgtgagcctgtatgcctttacccacatgccgagcctacatcagcgtggcaccatggtggtgacccatggcgaaggcccgtatatcgtggatgtgcatggccgtcgttatctggatgcgaacagcggcctgtggaacatggtggcgggctttgatcataaaggcctgattgatgcggcgaaagcgcagtatgaacgttttccgggctatcatgcgttttacggccgtatgagcgatcagaccgtgatgctgtctgaaaaactggtggaagtgagcccgtttgatagcggccgtgtgttttataccaacagcggcagcgaagcgaacgataccatggtgaaaatgctgtggtttctgcatcgtgcggaaggcaaaccgcagaaacgtaaaattctgaccctgaagaacgcgtatcatggctccaccgcggtgagcgcgagcatgaccggccttccgtataacagcgtgtttggcctgccgctgccgggctttctgcatctgacctgcccgcattattggcgttatggcgaagaaggcgaaaccgaagaacagtttgtcgcgcgtctggcccgtgaactggaagaaaccattcagaaggaaggcgcggataccattgcgggcttttttgcggaaccggtgatgggtgcgggcggtgttattaccccgccaaaaggctattttcaggcgattctgaccatcctgcgcaaatatgatattccggtgatcagcgatgaagtgatttgcggctttggtcgtaccggcaacacctggggctgcgtgacctatgattttaccccggatgcgattattagcagtaaaaacctaaccgcgggtttttttccagtaggagcggtgattttggggccggaactgagcaaacgtctggaaaccgcgattgaagcgatcgaagaatttgatcatggttttaccacaggcggccatccggtgggttgtgcgattgcgctgaaagcgattgatgtggtgatgaacgaaggcctggccgaaaacgtgcgtcgtctggccccgcgttttgaagaacgtctgaaacatattgcggaacgtccgaacattggcgaatatcgtggtattggctttatgtgggcgctggaagtggtgaaagataaagcgagcaaagccccgtttgatggcaacctgagcgtgagcgaacgtattgcgaacacctgcaccgatctgggactgatttgccgaccgttgggccagagcgtggttctggcaccgccgtacattctgaccgaagcgcagatggatgaaatgttcgataaactggaaaaagcgctggataaagtgtttgcggaagtggcgtaa

SEQ ID NO: 26 - protein, 453 aa, Artificial Sequence
  Engineered variant of V. fluvialis transaminase
MNKPQSWETRAETVSLYAFTHMPSLHQRGTMVVTHGEGPYIVDVHGRRYLDANSGLWNMVAGFDHKGLIDAAKAQYERFPGYHAFYGRMSDQTVMLSEKLVEVSPFDSGRVFYTNSGSEANDTMVKMLWFLHRAEGKPQKRKILTLKNAYHGSTAVSASMTGLPYNSVFGLPLPGFLHLTCPHYWRYGEEGETEEQFVARLARELEETIQKEGADTIAGFFAEPVMGAGGVITPPKGYFQAILTILRKYDIPVISDEVICGFGRTGNTWGCVTYDFTPDAIISSKNLTAGFFPVGAVILGPELSKRLETAIEAIEEFDHGFTTGGHPVGCAIALKAIDVVMNEGLAENVRRLAPRFEERLKHIAERPNIGEYRGIGFMWALEVVKDKASKAPFDGNLSVSERIANTCTDLGLICRPLGQSVVLAPPYILTEAQMDEMFDKLEKALDKVFAEVA

SEQ ID NO: 27 - DNA, 1362 bp, Artificial Sequence
  Engineered variant of V. fluvialis transaminase
atgaacaaaccgcagagctgggaaacgcgtgcggaaaccgtgagcctgtatgcctttacccacatgccgagcctacgtcagcgtggcaccatggtggtgacccatggcgaaggcccgtatatcgtggatgtgcatggccgtcgttatctggatgcgaacagcggcctgtggaacatggtggcgggctttgatcataaaggcctgattgatgcggcgaaagcgcagtatgaacgttttccgggctatcatgcgttttacggcgccatgagcgatcagaccgtgatgctgtctgaaaaactggtggaagtgagcccgtttgatagcggccgtgtgttttataccaacagcggcagcgaagcgaacgataccatggtgaaaatgctgtggtttctgcatcgtgcggaaggcaaaccgcagaaacgtaaaattctgaccctgaagcaggcgtatcatggctccaccgcggtgagcgcgagcatgaccggcatcccgtataacagcgtgtttggcctgccgctgccgggctttctgcatctgacctgcccgcattattggcgttatggcgaagaaggcgaaaccgaagaacagtttgtcgcgcgtctggcccgtgaactggaagaaaccattcagaaggaaggcgcggataccattgcgggcttttttgcggaaccggtgatgggtgcgggcggtgttattaccccgccaaaaggctattttcaggcgattctgaccatcctgcgcaaatatgatattccggtgatcagcgatgaagtgatttgcggctttggtcgtaccggcaacacctggggctgcgtgacctatgattttaccccggatgcgattattagcagtaaaaacctaaccgcgggtttttttccagtaggagcggtgattttggggccggaactgagcaaacgtctggaaaccgcgattgaagcgatcgaagaatttgatcatggttttaccacaggcggccatccggtgggttgtgcgattgcgctgaaagcgattgatgtggtgatgaacgaaggcctggccgaaaacgtgcgtcgtctggccccgcgttttgaagaacgtctgaaacatattgcggaacgtccgaacattggcgaatatcgtggtattggctttatgtgggcgctggaagtggtgaaagataaagcgagcaaagccccgtttgatggcaacctgagcgtgagcgaacgtattgcgaacacctgcaccgatctgggactgatttgccgaccgttgggccagagcgtggttctggcaccgccgtacattctgaccgaagcgcagatggatgaaatgttcgataaactggaaaaagcgctggataaagtgtttgcggaagtggcgtaa

SEQ ID NO: 28 - protein, 453 aa, Artificial Sequence
  Engineered variant of V. fluvialis transaminase
MNKPQSWETRAETVSLYAFTHMPSLRQRGTMVVTHGEGPYIVDVHGRRYLDANSGLWNMVAGFDHKGLIDAAKAQYERFPGYHAFYGAMSDQTVMLSEKLVEVSPFDSGRVFYTNSGSEANDTMVKMLWFLHRAEGKPQKRKILTLKQAYHGSTAVSASMTGIPYNSVFGLPLPGFLHLTCPHYWRYGEEGETEEQFVARLARELEETIQKEGADTIAGFFAEPVMGAGGVITPPKGYFQAILTILRKYDIPVISDEVICGFGRTGNTWGCVTYDFTPDAIISSKNLTAGFFPVGAVILGPELSKRLETAIEAIEEFDHGFTTGGHPVGCAIALKAIDVVMNEGLAENVRRLAPRFEERLKHIAERPNIGEYRGIGFMWALEVVKDKASKAPFDGNLSVSERIANTCTDLGLICRPLGQSVVLAPPYILTEAQMDEMFDKLEKALDKVFAEVA

SEQ ID NO: 29 - DNA, 1362 bp, Artificial Sequence
  Engineered variant of V. fluvialis transaminase
atgaacaaaccgcagagctgggaaacgcgtgcggaaaccgtgagcctgtatgcctttacccacatgccgagcctacgtcagcgtggcaccatggtggtgacccatggcgaaggcccgtatatcgtggatgtgcatggccgtcgttatctggatgcgaacagcggcctgtggaacatggtggcgggctttgatcataaaggcctgattgatgcggcgaaagcgcagtatgaacgttttccgggctatcatgcgttttacggcctgatgagcgatcagaccgtgatgctgtctgaaaaactggtggaagtgagcccgtttgatagcggccgtgtgtttgtgaccaacagcggcagcgaagcgaacgataccatggtgaaaatgctgtggtttctgcatcgtgcggaaggcaaaccgcagaaacgtaaaattctgaccctgaagaacgcgtatcatggctccaccgcggtgagcgcgagcatgaccggccttccgtataacagcgtgtttggcctgccgctgccgggctttctgcatctgacctgcccgcattattggcgttatggcgaagaaggcgaaaccgaagaacagtttgtcgcgcgtctggcccgtgaactggaagaaaccattcagaaggaaggcgcggataccattgcgggcttttttgcggaaccggtgatgggtgcgggcggtgttattaccccgccaaaaggctattttcaggcgattctgaccatcctgcgcaaatatgatattccggtgatcagcgatgaagtgatttgcggctttggtcgtaccggcaacacctggggctgcgtgacctatgattttaccccggatgcgattattagcagtaaaaacctaaccgcgggtttttttccagtaggagcggtgattttggggccggaactgagcaaacgtctggaaaccgcgattgaagcgatcgaagaatttgatcatggttttaccacaggcggccatccggtgggttgtgcgattgcgctgaaagcgattgatgtggtgatgaacgaaggcctggccgaaaacgtgcgtcgtctggccccgcgttttgaagaacgtctgaaacatattgcggaacgtccgaacattggcgaatatcgtggtattggctttatgtgggcgctggaagtggtgaaagataaagcgagcaaagccccgtttgatggcaacctgagcgtgagcgaacgtattgcgaacacctgcaccgatctgggactgatttgccgaccgttgggccagagcgtggttctggcaccgccgtacattctgaccgaagcgcagatggatgaaatgttcgataaactggaaaaagcgctggataaagtgtttgcggaagtggcgtaa

SEQ ID NO: 30 - protein, 453 aa, Artificial Sequence
  Engineered variant of V. fluvialis transaminase
MNKPQSWETRAETVSLYAFTHMPSLRQRGTMVVTHGEGPYIVDVHGRRYLDANSGLWNMVAGFDHKGLIDAAKAQYERFPGYHAFYGLMSDQTVMLSEKLVEVSPFDSGRVFVTNSGSEANDTMVKMLWFLHRAEGKPQKRKILTLKNAYHGSTAVSASMTGLPYNSVFGLPLPGFLHLTCPHYWRYGEEGETEEQFVARLARELEETIQKEGADTIAGFFAEPVMGAGGVITPPKGYFQAILTILRKYDIPVISDEVICGFGRTGNTWGCVTYDFTPDAIISSKNLTAGFFPVGAVILGPELSKRLETAIEAIEEFDHGFTTGGHPVGCAIALKAIDVVMNEGLAENVRRLAPRFEERLKHIAERPNIGEYRGIGFMWALEVVKDKASKAPFDGNLSVSERIANTCTDLGLICRPLGQSVVLAPPYILTEAQMDEMFDKLEKALDKVFAEVA

SEQ ID NO: 31 - DNA, 1362 bp, Artificial Sequence
  Engineered variant of V. fluvialis transaminase
atgaacaaaccgcagagctgggaaacgcgtgcggaaaccgtgagcctgtatgcctttacccacatgccgagcctacatcagcgtggcaccatggtggtgacccatggcgaaggcccgtatatcgtggatgtgcatggccgtcgttatctggatgcgaacagcggcctgttcaacatggtggcgggctttgatcataaaggcctgattgatgcggcgaaagcgcagtatgaacgttttccgggctatcatgcgttttacggccgcatgagcgatcagaccgtgatgctgtctgaaaaactggtggaagtgagcccgtttgatagcggccgtgtgtttgtgaccaacagcggcagcgaagcgaacgataccatggtgaaaatgctgtggtttctgcatcgtgcggaaggcaaaccgcagaaacgtaaaattctgaccctgaagcaggcgtatcatggctccaccgcggtgagcgcgagcatgaccggccttccgtataacagcgtgtttggcctgccgctgccgggctttctgcatctgacctgcccgcattattggcgttatggcgaagaaggcgaaaccgaagaacagtttgtcgcgcgtctggcccgtgaactggaagaaaccattcagaaggaaggcgcggataccattgcgggcttttttgcggaaccggtgatgggtgcgggcggtgttattaccccgccaaaaggctattttcaggcgattctgaccatcctgcgcaaatatgatattccggtgatcagcgatgaagtgatttgcggctttggtcgtaccggcaacacctggggctgcgtgacctatgattttaccccggatgcgattattagcagtaaaaacctaaccgcgggtttttttccagtaggagcggtgattttggggccggaactgagcaaacgtctggaaaccgcgattgaagcgatcgaagaatttgatcatggttttaccacaggcggccatccggtgggttgtgcgattgcgctgaaagcgattgatgtggtgatgaacgaaggcctggccgaaaacgtgcgtcgtctggccccgcgttttgaagaacgtctgaaacatattgcggaacgtccgaacattggcgaatatcgtggtattggctttatgtgggcgctggaagtggtgaaagataaagcgagcaaagccccgtttgatggcaacctgagcgtgagcgaacgtattgcgaacacctgcaccgatctgggactgatttgccgaccgttgggccagagcgtggttctggcaccgccgtacattctgaccgaagcgcagatggatgaaatgttcgataaactggaaaaagcgctggataaagtgtttgcggaagtggcgtaa

SEQ ID NO: 32 - protein, 453 aa, Artificial Sequence
  Engineered variant of V. fluvialis transaminase
MNKPQSWETRAETVSLYAFTHMPSLHQRGTMVVTHGEGPYIVDVHGRRYLDANSGLFNMVAGFDHKGLIDAAKAQYERFPGYHAFYGRMSDQTVMLSEKLVEVSPFDSGRVFVTNSGSEANDTMVKMLWFLHRAEGKPQKRKILTLKQAYHGSTAVSASMTGLPYNSVFGLPLPGFLHLTCPHYWRYGEEGETEEQFVARLARELEETIQKEGADTIAGFFAEPVMGAGGVITPPKGYFQAILTILRKYDIPVISDEVICGFGRTGNTWGCVTYDFTPDAIISSKNLTAGFFPVGAVILGPELSKRLETAIEAIEEFDHGFTTGGHPVGCAIALKAIDVVMNEGLAENVRRLAPRFEERLKHIAERPNIGEYRGIGFMWALEVVKDKASKAPFDGNLSVSERIANTCTDLGLICRPLGQSVVLAPPYILTEAQMDEMFDKLEKALDKVFAEVA

SEQ ID NO: 33 - DNA, 1362 bp, Artificial Sequence
  Engineered variant of V. fluvialis transaminase
atgaacaaaccgcagagctgggaaacgcgtgcggaaaccgtgagcctgtatgcctttacccacatgccgagcctacgtcagcgtggcaccatggtggtgacccatggcgaaggcccgtatatcgtggatgtgcatggccgtcgttatctggatgcgaacagcggcctgttcaacatggtggcgggctttgatcataaaggcctgattgatgcggcgaaagcgcagtatgaacgttttccgggctatcatgcgttttacggccgtatgagcgatcagaccgtgatgctgtctgaaaaactggtggaagtgagcccgtttgatagcggccgtgtgttttataccaacagcggcagcgaagcgaacgataccatggtgaaaatgctgtggtttctgcatcgtgcggaaggcaaaccgcagaaacgtaaaattctgaccctgaagcaggcgtatcatggctccaccgcggtgagcgcgagcatgaccggcatcccgtataacagcgtgtttggcctgccgctgccgggctttctgcatctgacctgcccgcattattggcgttatggcgaagaaggcgaaaccgaagaacagtttgtcgcgcgtctggcccgtgaactggaagaaaccattcagaaggaaggcgcggataccattgcgggcttttttgcggaaccggtgatgggtgcgggcggtgttattaccccgccaaaaggctattttcaggcgattctgaccatcctgcgcaaatatgatattccggtgatcagcgatgaagtgatttgcggctttggtcgtaccggcaacacctggggctgcgtgacctatgattttaccccggatgcgattattagcagtaaaaacctaaccgcgggtttttttccagtaggagcggtgattttggggccggaactgagcaaacgtctggaaaccgcgattgaagcgatcgaagaatttgatcatggttttaccacaggcggccatccggtgggttgtgcgattgcgctgaaagcgattgatgtggtgatgaacgaaggcctggccgaaaacgtgcgtcgtctggccccgcgttttgaagaacgtctgaaacatattgcggaacgtccgaacattggcgaatatcgtggtattggctttatgtgggcgctggaagtggtgaaagataaagcgagcaaagccccgtttgatggcaacctgagcgtgagcgaacgtattgcgaacacctgcaccgatctgggactgatttgccgaccgttgggccagagcgtggttctggcaccgccgtacattctgaccgaagcgcagatggatgaaatgttcgataaactggaaaaagcgctggataaagtgtttgcggaagtggcgtaa

SEQ ID NO: 34 - protein, 453 aa, Artificial Sequence
  Engineered variant of V. fluvialis transaminase
MNKPQSWETRAETVSLYAFTHMPSLRQRGTMVVTHGEGPYIVDVHGRRYLDANSGLFNMVAGFDHKGLIDAAKAQYERFPGYHAFYGRMSDQTVMLSEKLVEVSPFDSGRVFYTNSGSEANDTMVKMLWFLHRAEGKPQKRKILTLKQAYHGSTAVSASMTGIPYNSVFGLPLPGFLHLTCPHYWRYGEEGETEEQFVARLARELEETIQKEGADTIAGFFAEPVMGAGGVITPPKGYFQAILTILRKYDIPVISDEVICGFGRTGNTWGCVTYDFTPDAIISSKNLTAGFFPVGAVILGPELSKRLETAIEAIEEFDHGFTTGGHPVGCAIALKAIDVVMNEGLAENVRRLAPRFEERLKHIAERPNIGEYRGIGFMWALEVVKDKASKAPFDGNLSVSERIANTCTDLGLICRPLGQSVVLAPPYILTEAQMDEMFDKLEKALDKVFAEVA

SEQ ID NO: 35 - DNA, 1362 bp, Artificial Sequence
  Engineered variant of V. fluvialis transaminase
atgaacaaaccgcagagctgggaaacgcgtgcggaaaccgtgagcctgtatgcctttacccacatgccgagcctacgtcagcgtggcaccatggtggtgacccatggcgaaggcccgtatatcgtggatgtgcatggccgtcgttatctggatgcgaacagcggcctgtggaacatggtggcgggctttgatcataaaggcctgattgatgcggcgaaagcgcagtatgaacgttttccgggctatcatgcgttttacggccgtatgagcgatcagaccgtgatgctgtctgaaaaactggtggaagtgagcccgtttgatagcggccgtgtgttttataccaacagcggcagcgaagcgaacgataccatggtgaaaatgctgtggtttctgcatcgtgcggaaggcaaaccgcagaaacgtaaaattctgaccctgaagaacgcgtatcatggctccaccgcggtgagcgcgagcatgaccggccttccgtataacagcgtgtttggcctgccgctgccgggctttctgcatctgacctgcccgcattattggcgttatggcgaagaaggcgaaaccgaagaacagtttgtcgcgcgtctggcccgtgaactggaagaaaccattcagaaggaaggcgcggataccattgcgggcttttttgcggaaccggtgatgggtgcgggcggtgttattaccccgccaaaaggctattttcaggcgattctgaccatcctgcgcaaatatgatattccggtgatcagcgatgaagtgatttgcggctttggtcgtaccggcaacacctggggctgcgtgacctatgattttaccccggatgcgattattagcagtaaaaacctaaccgcgggtttttttccagtaggagcggtgattttggggccggaactgagcaaacgtctggaaaccgcgattgaagcgatcgaagaatttgatcatggttttaccacaggcggccatccggtgggttgtgcgattgcgctgaaagcgattgatgtggtgatgaacgaaggcctggccgaaaacgtgcgtcgtctggccccgcgttttgaagaacgtctgaaacatattgcggaacgtccgaacattggcgaatatcgtggtattggctttatgtgggcgctggaagtggtgaaagataaagcgagcaaagccccgtttgatggcaacctgagcgtgagcgaacgtattgcgaacacctgcaccgatctgggactgatttgccgaccgttgggccagagcgtggttctggcaccgccgtacattctgaccgaagcgcagatggatgaaatgttcgataaactggaaaaagcgctggataaagtgtttgcggaagtggcgtaa

SEQ ID NO: 36 - protein, 453 aa, Artificial Sequence
  Engineered variant of V. fluvialis transaminase
MNKPQSWETRAETVSLYAFTHMPSLRQRGTMVVTHGEGPYIVDVHGRRYLDANSGLWNMVAGFDHKGLIDAAKAQYERFPGYHAFYGRMSDQTVMLSEKLVEVSPFDSGRVFYTNSGSEANDTMVKMLWFLHRAEGKPQKRKILTLKNAYHGSTAVSASMTGLPYNSVFGLPLPGFLHLTCPHYWRYGEEGETEEQFVARLARELEETIQKEGADTIAGFFAEPVMGAGGVITPPKGYFQAILTILRKYDIPVISDEVICGFGRTGNTWGCVTYDFTPDAIISSKNLTAGFFPVGAVILGPELSKRLETAIEAIEEFDHGFTTGGHPVGCAIALKAIDVVMNEGLAENVRRLAPRFEERLKHIAERPNIGEYRGIGFMWALEVVKDKASKAPFDGNLSVSERIANTCTDLGLICRPLGQSVVLAPPYILTEAQMDEMFDKLEKALDKVFAEVA

SEQ ID NO: 37 - DNA, 1362 bp, Artificial Sequence
  Engineered variant of V. fluvialis transaminase
atgaacaaaccgcagagctgggaaacgcgtgcggaaaccgtgagcctgtatgcctttacccacatgccgagcctacgtcagcgtggcaccatggtggtgacccatggcgaaggcccgtatatcgtggatgtgcatggccgtcgttatctggatgcgaacagcggcctgttcaacatggtggcgggctttgatcataaaggcctgattgatgcggcgaaagcgcagtatgaacgttttccgggctatcatgcgttttacggccgcatgagcgatcagaccgtgatgctgtctgaaaaactggtggaagtgagcccgtttgatagcggccgtgtgtttctgaccaacagcggcagcgaagcgaacgataccatggtgaaaatgctgtggtttctgcatcgtgcggaaggcaaaccgcagaaacgtaaaattctgaccctgaagaacgcgtatcatggctccaccgcggtgagcgcgagcatgaccggccttccgtataacagcgtgtttggcctgccgctgccgggctttctgcatctgacctgcccgcattattggcgttatggcgaagaaggcgaaaccgaagaacagtttgtcgcgcgtctggcccgtgaactggaagaaaccattcagaaggaaggcgcggataccattgcgggcttttttgcggaaccggtgatgggtgcgggcggtgttattaccccgccaaaaggctattttcaggcgattctgaccatcctgcgcaaatatgatattccggtgatcagcgatgaagtgatttgcggctttggtcgtaccggcaacacctggggctgcgtgacctatgattttaccccggatgcgattattagcagtaaaaacctaaccgcgggtttttttccagtaggagcggtgattttggggccggaactgagcaaacgtctggaaaccgcgattgaagcgatcgaagaatttgatcatggttttaccacaggcggccatccggtgggttgtgcgattgcgctgaaagcgattgatgtggtgatgaacgaaggcctggccgaaaacgtgcgtcgtctggccccgcgttttgaagaacgtctgaaacatattgcggaacgtccgaacattggcgaatatcgtggtattggctttatgtgggcgctggaagtggtgaaagataaagcgagcaaagccccgtttgatggcaacctgagcgtgagcgaacgtattgcgaacacctgcaccgatctgggactgatttgccgaccgttgggccagagcgtggttctggcaccgccgtacattctgaccgaagcgcagatggatgaaatgttcgataaactggaaaaagcgctggataaagtgtttgcggaagtggcgtaa

SEQ ID NO: 38 - protein, 453 aa, Artificial Sequence
  Engineered variant of V. fluvialis transaminase
MNKPQSWETRAETVSLYAFTHMPSLRQRGTMVVTHGEGPYIVDVHGRRYLDANSGLFNMVAGFDHKGLIDAAKAQYERFPGYHAFYGRMSDQTVMLSEKLVEVSPFDSGRVFLTNSGSEANDTMVKMLWFLHRAEGKPQKRKILTLKNAYHGSTAVSASMTGLPYNSVFGLPLPGFLHLTCPHYWRYGEEGETEEQFVARLARELEETIQKEGADTIAGFFAEPVMGAGGVITPPKGYFQAILTILRKYDIPVISDEVICGFGRTGNTWGCVTYDFTPDAIISSKNLTAGFFPVGAVILGPELSKRLETAIEAIEEFDHGFTTGGHPVGCAIALKAIDVVMNEGLAENVRRLAPRFEERLKHIAERPNIGEYRGIGFMWALEVVKDKASKAPFDGNLSVSERIANTCTDLGLICRPLGQSVVLAPPYILTEAQMDEMFDKLEKALDKVFAEVA

SEQ ID NO: 39 - DNA, 1362 bp, Artificial Sequence
  Engineered variant of V. fluvialis transaminase
atgaacaaaccgcagagctgggaaacgcgtgcggaaaccgtgagcctgtatgcctttacccacatgccgagcctacgtcagcgtggcaccatggtggtgacccatggcgaaggcccgtatatcgtggatgtgcatggccgtcgttatctggatgcgaacagcggcctgtggaacatggtggcgggctttgatcataaaggcctgattgatgcggcgaaagcgcagtatgaacgttttccgggctatcatgcgttttacggccgtatgagcgatcagaccgtgatgctgtctgaaaaactggtggaagtgagcccgtttgatagcggccgtgtgttttataccaacagcggcagcgaagcgaacgataccatggtgaaaatgctgtggtttctgcatcgtgcggaaggcaaaccgcagaaacgtaaaattctgaccctgaagaacgcgtatcatggctccaccgcggtgagcgcgagcatgaccggcatcccgtataacagcgtgtttggcctgccgctgccgggctttctgcatctgacctgcccgcattattggcgttatggcgaagaaggcgaaaccgaagaacagtttgtcgcgcgtctggcccgtgaactggaagaaaccattcagaaggaaggcgcggataccattgcgggcttttttgcggaaccggtgatgggtgcgggcggtgttattaccccgccaaaaggctattttcaggcgattctgaccatcctgcgcaaatatgatattccggtgatcagcgatgaagtgatttgcggctttggtcgtaccggcaacacctggggctgcgtgacctatgattttaccccggatgcgattattagcagtaaaaacctaaccgcgggtttttttccagtaggagcggtgattttggggccggaactgagcaaacgtctggaaaccgcgattgaagcgatcgaagaatttgatcatggttttaccacaggcggccatccggtgggttgtgcgattgcgctgaaagcgattgatgtggtgatgaacgaaggcctggccgaaaacgtgcgtcgtctggccccgcgttttgaagaacgtctgaaacatattgcggaacgtccgaacattggcgaatatcgtggtattggctttatgtgggcgctggaagtggtgaaagataaagcgagcaaagccccgtttgatggcaacctgagcgtgagcgaacgtattgcgaacacctgcaccgatctgggactgatttgccgaccgttgggccagagcgtggttctggcaccgccgtacattctgaccgaagcgcagatggatgaaatgttcgataaactggaaaaagcgctggataaagtgtttgcggaagtggcgtaa

SEQ ID NO: 40 - protein, 453 aa, Artificial Sequence
  Engineered variant of V. fluvialis transaminase
MNKPQSWETRAETVSLYAFTHMPSLRQRGTMVVTHGEGPYIVDVHGRRYLDANSGLWNMVAGFDHKGLIDAAKAQYERFPGYHAFYGRMSDQTVMLSEKLVEVSPFDSGRVFYTNSGSEANDTMVKMLWFLHRAEGKPQKRKILTLKNAYHGSTAVSASMTGIPYNSVFGLPLPGFLHLTCPHYWRYGEEGETEEQFVARLARELEETIQKEGADTIAGFFAEPVMGAGGVITPPKGYFQAILTILRKYDIPVISDEVICGFGRTGNTWGCVTYDFTPDAIISSKNLTAGFFPVGAVILGPELSKRLETAIEAIEEFDHGFTTGGHPVGCAIALKAIDVVMNEGLAENVRRLAPRFEERLKHIAERPNIGEYRGIGFMWALEVVKDKASKAPFDGNLSVSERIANTCTDLGLICRPLGQSVVLAPPYILTEAQMDEMFDKLEKALDKVFAEVA

SEQ ID NO: 41 - DNA, 1362 bp, Artificial Sequence
  Engineered variant of V. fluvialis transaminase
atgaacaaaccgcagagctgggaaacgcgtgcggaaaccgtgagcctgtatgcctttacccacatgccgagcctacgtcagcgtggcaccatggtggtgacccatggcgaaggcccgtatatcgtggatgtgcatggccgtcgttatctggatgcgaacagcggcctgttcaacatggtggcgggctttgatcataaaggcctgattgatgcggcgaaagcgcagtatgaacgttttccgggctatcatgcgttttacggcctgatgagcgatcagaccgtgatgctgtctgaaaaactggtggaagtgagcccgtttgatagcggccgtgtgttttataccaacagcggcagcgaagcgaacgataccatggtgaaaatgctgtggtttctgcatcgtgcggaaggcaaaccgcagaaacgtaaaattctgaccctgaagaacgcgtatcatggctccaccgcggtgagcgcgagcatgaccggcatcccgtataacagcgtgtttggcctgccgctgccgggctttctgcatctgacctgcccgcattattggcgttatggcgaagaaggcgaaaccgaagaacagtttgtcgcgcgtctggcccgtgaactggaagaaaccattcagaaggaaggcgcggataccattgcgggcttttttgcggaaccggtgatgggtgcgggcggtgttattaccccgccaaaaggctattttcaggcgattctgaccatcctgcgcaaatatgatattccggtgatcagcgatgaagtgatttgcggctttggtcgtaccggcaacacctggggctgcgtgacctatgattttaccccggatgcgattattagcagtaaaaacctaaccgcgggtttttttccagtaggagcggtgattttggggccggaactgagcaaacgtctggaaaccgcgattgaagcgatcgaagaatttgatcatggttttaccacaggcggccatccggtgggttgtgcgattgcgctgaaagcgattgatgtggtgatgaacgaaggcctggccgaaaacgtgcgtcgtctggccccgcgttttgaagaacgtctgaaacatattgcggaacgtccgaacattggcgaatatcgtggtattggctttatgtgggcgctggaagtggtgaaagataaagcgagcaaagccccgtttgatggcaacctgagcgtgagcgaacgtattgcgaacacctgcaccgatctgggactgatttgccgaccgttgggccagagcgtggttctggcaccgccgtacattctgaccgaagcgcagatggatgaaatgttcgataaactggaaaaagcgctggataaagtgtttgcggaagtggcgtaa

SEQ ID NO: 42 - protein, 453 aa, Artificial Sequence
  Engineered variant of V. fluvialis transaminase
MNKPQSWETRAETVSLYAFTHMPSLRQRGTMVVTHGEGPYIVDVHGRRYLDANSGLFNMVAGFDHKGLIDAAKAQYERFPGYHAFYGLMSDQTVMLSEKLVEVSPFDSGRVFYTNSGSEANDTMVKMLWFLHRAEGKPQKRKILTLKNAYHGSTAVSASMTGIPYNSVFGLPLPGFLHLTCPHYWRYGEEGETEEQFVARLARELEETIQKEGADTIAGFFAEPVMGAGGVITPPKGYFQAILTILRKYDIPVISDEVICGFGRTGNTWGCVTYDFTPDAIISSKNLTAGFFPVGAVILGPELSKRLETAIEAIEEFDHGFTTGGHPVGCAIALKAIDVVMNEGLAENVRRLAPRFEERLKHIAERPNIGEYRGIGFMWALEVVKDKASKAPFDGNLSVSERIANTCTDLGLICRPLGQSVVLAPPYILTEAQMDEMFDKLEKALDKVFAEVA

SEQ ID NO: 43 - DNA, 1362 bp, Artificial Sequence
  Engineered variant of V. fluvialis transaminase
atgaacaaaccgcagagctgggaaacgcgtgcggaaaccgtgagcctgtatgcctttacccacatgccgagcctacgtcagcgtggcaccatggtggtgacccatggcgaaggcccgtatatcgtggatgtgcatggccgtcgttatctggatgcgaacagcggcctgtggaacatggtggcgggctttgatcataaaggcctgattgatgcggcgaaagcgcagtatgaacgttttccgggctatcatgcgttttacggccgtatgagcgatcagaccgtgatgctgtctgaaaaactggtggaagtgagcccgtttgatagcggccgtgtgtttgtgaccaacagcggcagcgaagcgaacgataccatggtgaaaatgctgtggtttctgcatcgtgcggaaggcaaaccgcagaaacgtaaaattctgaccctgaagaacgcgtatcatggctccaccgcggtgagcgcgagcatgaccggcatcccgtataacagcgtgtttggcctgccgctgccgggctttctgcatctgacctgcccgcattattggcgttatggcgaagaaggcgaaaccgaagaacagtttgtcgcgcgtctggcccgtgaactggaagaaaccattcagaaggaaggcgcggataccattgcgggcttttttgcggaaccggtgatgggtgcgggcggtgttattaccccgccaaaaggctattttcaggcgattctgaccatcctgcgcaaatatgatattccggtgatcagcgatgaagtgatttgcggctttggtcgtaccggcaacacctggggctgcgtgacctatgattttaccccggatgcgattattagcagtaaaaacctaaccgcgggtttttttccagtaggagcggtgattttggggccggaactgagcaaacgtctggaaaccgcgattgaagcgatcgaagaatttgatcatggttttaccacaggcggccatccggtgggttgtgcgattgcgctgaaagcgattgatgtggtgatgaacgaaggcctggccgaaaacgtgcgtcgtctggccccgcgttttgaagaacgtctgaaacatattgcggaacgtccgaacattggcgaatatcgtggtattggctttatgtgggcgctggaagtggtgaaagataaagcgagcaaagccccgtttgatggcaacctgagcgtgagcgaacgtattgcgaacacctgcaccgatctgggactgatttgccgaccgttgggccagagcgtggttctggcaccgccgtacattctgaccgaagcgcagatggatgaaatgttcgataaactggaaaaagcgctggataaagtgtttgcggaagtggcgtaa

SEQ ID NO: 44 - protein, 453 aa, Artificial Sequence
  Engineered variant of V. fluvialis transaminase
MNKPQSWETRAETVSLYAFTHMPSLRQRGTMVVTHGEGPYIVDVHGRRYLDANSGLWNMVAGFDHKGLIDAAKAQYERFPGYHAFYGRMSDQTVMLSEKLVEVSPFDSGRVFVTNSGSEANDTMVKMLWFLHRAEGKPQKRKILTLKNAYHGSTAVSASMTGIPYNSVFGLPLPGFLHLTCPHYWRYGEEGETEEQFVARLARELEETIQKEGADTIAGFFAEPVMGAGGVITPPKGYFQAILTILRKYDIPVISDEVICGFGRTGNTWGCVTYDFTPDAIISSKNLTAGFFPVGAVILGPELSKRLETAIEAIEEFDHGFTTGGHPVGCAIALKAIDVVMNEGLAENVRRLAPRFEERLKHIAERPNIGEYRGIGFMWALEVVKDKASKAPFDGNLSVSERIANTCTDLGLICRPLGQSVVLAPPYILTEAQMDEMFDKLEKALDKVFAEVA

SEQ ID NO: 45 - DNA, 1362 bp, Artificial Sequence
  Engineered variant of V. fluvialis transaminase
atgaacaaaccgcagagctgggaaacgcgtgcggaaaccgtgagcctgtatgcctttacccacatgccgagcctacgtcagcgtggcaccatggtggtaacccatggcgaaggcccgtatatcgtggatgtgcatggccgtcgttatctggatgcgaacagcggcctgttcaacatggtggcgggctttgatcataaaggcctgattgatgcggcgaaagcgcagtatgaacgttttccgggctatcatgcgttttacggcctgatgagcgatcagaccgtgatgctgtctgaaaaactggtggaagtgagcccgtttgatagcggccgtgtgtttctgaccaacagcggcagcgaagcgaacgataccatggtgaaaatgctgtggtttctgcatcgtgcggaaggcaaaccgcagaaacgtaaaattctgaccctgaagcaggcgtatcatggctccaccgcggtgagcgcgagcatgaccggcatcccgtataacagcgtgtttggcctgccgctgccgggctttctgcatctgacctgcccgcattattggcgttatggcgaagaaggcgaaaccgaagaacagtttgtcgcgcgtctggcccgtgaactggaagaaaccattcagaaggaaggcgcggataccattgcgggcttttttgcggaaccggtgatgggtgcgggcggtgttattaccccgccaaaaggctattttcaggcgattctgaccatcctgcgcaaatatgatattccggtgatcagcgatgaagtgatttgcggctttggtcgtaccggcaacacctggggctgcgtgacctatgattttaccccggatgcgattattagcagtaaaaacctaaccgcgggtttttttccagtaggagcggtgattttggggccggaactgagcaaacgtctggaaaccgcgattgaagcgatcgaagaatttgatcatggttttaccacaggcggccatccggtgggttgtgcgattgcgctgaaagcgattgatgtggtgatgaacgaaggcctggccgaaaacgtgcgtcgtctggccccgcgttttgaagaacgtctgaaacatattgcggaacgtccgaacattggcgaatatcgtggtattggctttatgtgggcgctggaagtggtgaaagataaagcgagcaaagccccgtttgatggcaacctgagcgtgagcgaacgtattgcgaacacctgcaccgatctgggactgatttgccgaccgttgggccagagcgtggttctggcaccgccgtacattctgaccgaagcgcagatggatgaaatgttcgataaactggaaaaagcgctggataaagtgtttgcggaagtggcgtaa

SEQ ID NO: 46 - protein, 453 aa, Artificial Sequence
  Engineered variant of V. fluvialis transaminase
MNKPQSWETRAETVSLYAFTHMPSLRQRGTMVVTHGEGPYIVDVHGRRYLDANSGLFNMVAGFDHKGLIDAAKAQYERFPGYHAFYGLMSDQTVMLSEKLVEVSPFDSGRVFLTNSGSEANDTMVKMLWFLHRAEGKPQKRKILTLKQAYHGSTAVSASMTGIPYNSVFGLPLPGFLHLTCPHYWRYGEEGETEEQFVARLARELEETIQKEGADTIAGFFAEPVMGAGGVITPPKGYFQAILTILRKYDIPVISDEVICGFGRTGNTWGCVTYDFTPDAIISSKNLTAGFFPVGAVILGPELSKRLETAIEAIEEFDHGFTTGGHPVGCAIALKAIDVVMNEGLAENVRRLAPRFEERLKHIAERPNIGEYRGIGFMWALEVVKDKASKAPFDGNLSVSERIANTCTDLGLICRPLGQSVVLAPPYILTEAQMDEMFDKLEKALDKVFAEVA

SEQ ID NO: 47 - DNA, 1362 bp, Artificial Sequence
  Engineered variant of V. fluvialis transaminase
atgaacaaaccgcagagctgggaaacgcgtgcggaaaccgtgagcctgtatgcctttacccacatgccgagcctacatcagcgtggcaccatggtggtgacccatggcgaaggcccgtatatcgtggatgtgcatggccgtcgttatctggatgcgaacagcggcctgttcaacatggtggcgggctttgatcataaaggcctgattgatgcggcgaaagcgcagtatgaacgttttccgggctatcatgcgttttacggcctgatgagcgatcagaccgtgatgctgtctgaaaaactggtggaagtgagcccgtttgatagcggccgtgtgttttataccaacagcggcagcgaagcgaacgataccatggtgaaaatgctgtggtttctgcatcgtgcggaaggcaaaccgcagaaacgtaaaattctgaccctgaagcaggcgtatcatggctccaccgcggtgagcgcgagcatgaccggcatcccgtataacagcgtgtttggcctgccgctgccgggctttctgcatctgacctgcccgcattattggcgttatggcgaagaaggcgaaaccgaagaacagtttgtcgcgcgtctggcccgtgaactggaagaaaccattcagaaggaaggcgcggataccattgcgggcttttttgcggaaccggtgatgggtgcgggcggtgttattaccccgccaaaaggctattttcaggcgattctgaccatcctgcgcaaatatgatattccggtgatcagcgatgaagtgatttgcggctttggtcgtaccggcaacacctggggctgcgtgacctatgattttaccccggatgcgattattagcagtaaaaacctaaccgcgggtttttttccagtaggagcggtgattttggggccggaactgagcaaacgtctggaaaccgcgattgaagcgatcgaagaatttgatcatggttttaccacaggcggccatccggtgggttgtgcgattgcgctgaaagcgattgatgtggtgatgaacgaaggcctggccgaaaacgtgcgtcgtctggccccgcgttttgaagaacgtctgaaacatattgcggaacgtccgaacattggcgaatatcgtggtattggctttatgtgggcgctggaagtggtgaaagataaagcgagcaaagccccgtttgatggcaacctgagcgtgagcgaacgtattgcgaacacctgcaccgatctgggactgatttgccgaccgttgggccagagcgtggttctggcaccgccgtacattctgaccgaagcgcagatggatgaaatgttcgataaactggaaaaagcgctggataaagtgtttgcggaagtggcgtaa

SEQ ID NO: 48 - protein, 453 aa, Artificial Sequence
  Engineered variant of V. fluvialis transaminase
MNKPQSWETRAETVSLYAFTHMPSLHQRGTMVVTHGEGPYIVDVHGRRYLDANSGLFNMVAGFDHKGLIDAAKAQYERFPGYHAFYGLMSDQTVMLSEKLVEVSPFDSGRVFYTNSGSEANDTMVKMLWFLHRAEGKPQKRKILTLKQAYHGSTAVSASMTGIPYNSVFGLPLPGFLHLTCPHYWRYGEEGETEEQFVARLARELEETIQKEGADTIAGFFAEPVMGAGGVITPPKGYFQAILTILRKYDIPVISDEVICGFGRTGNTWGCVTYDFTPDAIISSKNLTAGFFPVGAVILGPELSKRLETAIEAIEEFDHGFTTGGHPVGCAIALKAIDVVMNEGLAENVRRLAPRFEERLKHIAERPNIGEYRGIGFMWALEVVKDKASKAPFDGNLSVSERIANTCTDLGLICRPLGQSVVLAPPYILTEAQMDEMFDKLEKALDKVFAEVA

SEQ ID NO: 49 - DNA, 1362 bp, Artificial Sequence
  Engineered variant of V. fluvialis transaminase
atgaacaaaccgcagagctgggaaacgcgtgcggaaaccgtgagcctgtatgcctttacccacatgccgagcctacgtcagcgtggcaccatggtggtgacccatggcgaaggcccgtatatcgtggatgtgcatggccgtcgttatctggatgcgaacagcggcctgttcaacatggtggcgggctttgatcataaaggcctgattgatgcggcgaaagcgcagtatgaacgttttccgggctatcatgcgttttacggcctgatgagcgatcagaccgtgatgctgtctgaaaaactggtggaagtgagcccgtttgatagcggccgtgtgtttgtgaccaacagcggcagcgaagcgaacgataccatggtgaaaatgctgtggtttctgcatcgtgcggaaggcaaaccgcagaaacgtaaaattctgaccctgaagcgtgcgtatcatggctccaccgcggtgagcgcgagcatgaccggccttccgtataacagcgtgtttggcctgccgctgccgggctttctgcatctgacctgcccgcattattggcgttatggcgaagaaggcgaaaccgaagaacagtttgtcgcgcgtctggcccgtgaactggaagaaaccattcagaaggaaggcgcggataccattgcgggcttttttgcggaaccggtgatgggtgcgggcggtgttattaccccgccaaaaggctattttcaggcgattctgaccatcctgcgcaaatatgatattccggtgatcagcgatgaagtgatttgcggctttggtcgtaccggcaacacctggggctgcgtgacctatgattttaccccggatgcgattattagcagtaaaaacctaaccgcgggtttttttccagtaggagcggtgattttggggccggaactgagcaaacgtctggaaaccgcgattgaagcgatcgaagaatttgatcatggttttaccacaggcggccatccggtgggttgtgcgattgcgctgaaagcgattgatgtggtgatgaacgaaggcctggccgaaaacgtgcgtcgtctggccccgcgttttgaagaacgtctgaaacatattgcggaacgtccgaacattggcgaatatcgtggtattggctttatgtgggcgctggaagtggtgaaagataaagcgagcaaagccccgtttgatggcaacctgagcgtgagcgaacgtattgcgaacacctgcaccgatctgggactgatttgccgaccgttgggccagagcgtggttctggcaccgccgtacattctgaccgaagcgcagatggatgaaatgttcgataaactggaaaaagcgctggataaagtgtttgcggaagtggcgtaa

SEQ ID NO: 50 - protein, 453 aa, Artificial Sequence
  Engineered variant of V. fluvialis transaminase
MNKPQSWETRAETVSLYAFTHMPSLRQRGTMVVTHGEGPYIVDVHGRRYLDANSGLFNMVAGFDHKGLIDAAKAQYERFPGYHAFYGLMSDQTVMLSEKLVEVSPFDSGRVFVTNSGSEANDTMVKMLWFLHRAEGKPQKRKILTLKRAYHGSTAVSASMTGLPYNSVFGLPLPGFLHLTCPHYWRYGEEGETEEQFVARLARELEETIQKEGADTIAGFFAEPVMGAGGVITPPKGYFQAILTILRKYDIPVISDEVICGFGRTGNTWGCVTYDFTPDAIISSKNLTAGFFPVGAVILGPELSKRLETAIEAIEEFDHGFTTGGHPVGCAIALKAIDVVMNEGLAENVRRLAPRFEERLKHIAERPNIGEYRGIGFMWALEVVKDKASKAPFDGNLSVSERIANTCTDLGLICRPLGQSVVLAPPYILTEAQMDEMFDKLEKALDKVFAEVA

SEQ ID NO: 51 - DNA, 1362 bp, Artificial Sequence
  Engineered variant of V. fluvialis transaminase
atgaacaaaccgcagagctgggaaacgcgtgcggaaaccgtgagcctgtatgcctttacccacatgccgagcctacatcagcgtggcaccatggtggtgacccatggcgaaggcccgtatatcgtggatgtgcatggccgtcgttatctggatgcgaacagcggcctgtggaacatggtggcgggctttgatcataaaggcctgattgatgcggcgaaagcgcagtatgaacgttttccgggctatcatgcgttttacggcgccatgagcgatcagaccgtgatgctgtctgaaaaactggtggaagtgagcccgtttgatagcggccgtgtgtttgtgaccaacagcggcagcgaagcgaacgataccatggtgaaaatgctgtggtttctgcatcgtgcggaaggcaaaccgcagaaacgtaaaattctgaccctgaagaacgcgtatcatggctccaccgcggtgagcgcgagcatgaccggcatcccgtataacagcgtgtttggcctgccgctgccgggctttctgcatctgacctgcccgcattattggcgttatggcgaagaaggcgaaaccgaagaacagtttgtcgcgcgtctggcccgtgaactggaagaaaccattcagaaggaaggcgcggataccattgcgggcttttttgcggaaccggtgatgggtgcgggcggtgttattaccccgccaaaaggctattttcaggcgattctgaccatcctgcgcaaatatgatattccggtgatcagcgatgaagtgatttgcggctttggtcgtaccggcaacacctggggctgcgtgacctatgattttaccccggatgcgattattagcagtaaaaacctaaccgcgggtttttttccagtaggagcggtgattttggggccggaactgagcaaacgtctggaaaccgcgattgaagcgatcgaagaatttgatcatggttttaccacaggcggccatccggtgggttgtgcgattgcgctgaaagcgattgatgtggtgatgaacgaaggcctggccgaaaacgtgcgtcgtctggccccgcgttttgaagaacgtctgaaacatattgcggaacgtccgaacattggcgaatatcgtggtattggctttatgtgggcgctggaagtggtgaaagataaagcgagcaaagccccgtttgatggcaacctgagcgtgagcgaacgtattgcgaacacctgcaccgatctgggactgatttgccgaccgttgggccagagcgtggttctggcaccgccgtacattctgaccgaagcgcagatggatgaaatgttcgataaactggaaaaagcgctggataaagtgtttgcggaagtggcgtaa

SEQ ID NO: 52 - protein, 453 aa, Artificial Sequence
  Engineered variant of V. fluvialis transaminase
MNKPQSWETRAETVSLYAFTHMPSLHQRGTMVVTHGEGPYIVDVHGRRYLDANSGLWNMVAGFDHKGLIDAAKAQYERFPGYHAFYGAMSDQTVMLSEKLVEVSPFDSGRVFVTNSGSEANDTMVKMLWFLHRAEGKPQKRKILTLKNAYHGSTAVSASMTGIPYNSVFGLPLPGFLHLTCPHYWRYGEEGETEEQFVARLARELEETIQKEGADTIAGFFAEPVMGAGGVITPPKGYFQAILTILRKYDIPVISDEVICGFGRTGNTWGCVTYDFTPDAIISSKNLTAGFFPVGAVILGPELSKRLETAIEAIEEFDHGFTTGGHPVGCAIALKAIDVVMNEGLAENVRRLAPRFEERLKHIAERPNIGEYRGIGFMWALEVVKDKASKAPFDGNLSVSERIANTCTDLGLICRPLGQSVVLAPPYILTEAQMDEMFDKLEKALDKVFAEVA

SEQ ID NO: 53 - DNA, 1362 bp, Artificial Sequence
  Engineered variant of V. fluvialis transaminase
atgaacaaaccgcagagctgggaaacgcgtgcggaaaccgtgagcctgtatgcctttacccacatgccgagcctacgtcagcgtggcaccatggtggtgacccatggcgaaggcccgtatatcgtggatgtgcatggccgtcgttatctggatgcgaacagcggcctgtggaacatggtggcgggctttgatcataaaggcctgattgatgcggcgaaagcgcagtatgaacgttttccgggctatcatgcgttttacggccgcatgagcgatcagaccgtgatgctgtctgaaaaactggtggaagtgagcccgtttgatagcggccgtgtgttttataccaacagcggcagcgaagcgaacgataccatggtgaaaatgctgtggtttctgcatcgtgcggaaggcaaaccgcagaaacgtaaaattctgaccctgaagaacgcgtatcatggctccaccgcggtgagcgcgagcatgaccggccttccgtataacagcgtgtttggcctgccgctgccgggctttctgcatctgacctgcccgcattattggcgttatggcgaagaaggcgaaaccgaagaacagtttgtcgcgcgtctggcccgtgaactggaagaaaccattcagaaggaaggcgcggataccattgcgggcttttttgcggaaccggtgatgggtgcgggcggtgttattaccccgccaaaaggctattttcaggcgattctgaccatcctgcgcaaatatgctattccggtgatcagcgatgaagtgatttgcggctttggtcgtaccggcaacacctggggctgcgtgacctatgattttaccccggatgcgattattagcagtaaaaacctaaccgcgggtttttttccagtaggagcggtgattttggggccggaactgagcaaacgtctggaaaccgcgattgaagcgatcgaagaatttgatcatggttttaccacaggcggccatccggtgggttgtgcgattgcgctgaaagcgattgatgtggtgatgaacgaaggcctggccgaaaacgtgcgtcgtctggccccgcgttttgaagaacgtctgaaacatattgcggaacgtccgaacattggcgaatatcgtggtattggctttatgtgggcgctggaagtggtgaaagataaagcgagcaaagccccgtttgatggcaacctgagcgtgagcgaacgtattgcgaacacctgcaccgatctgggactgatttgccgaccgttgggccagagcgtggttctggcaccgccgtacattctgaccgaagcgcagatggatgaaatgttcgataaactggaaaaagcgctggataaagtgtttgcggaagtggcgtaa

SEQ ID NO: 54 - protein, 453 aa, Artificial Sequence
  Engineered variant of V. fluvialis transaminase
MNKPQSWETRAETVSLYAFTHMPSLRQRGTMVVTHGEGPYIVDVHGRRYLDANSGLWNMVAGFDHKGLIDAAKAQYERFPGYHAFYGRMSDQTVMLSEKLVEVSPFDSGRVFYTNSGSEANDTMVKMLWFLHRAEGKPQKRKILTLKNAYHGSTAVSASMTGLPYNSVFGLPLPGFLHLTCPHYWRYGEEGETEEQFVARLARELEETIQKEGADTIAGFFAEPVMGAGGVITPPKGYFQAILTILRKYAIPVISDEVICGFGRTGNTWGCVTYDFTPDAIISSKNLTAGFFPVGAVILGPELSKRLETAIEAIEEFDHGFTTGGHPVGCAIALKAIDVVMNEGLAENVRRLAPRFEERLKHIAERPNIGEYRGIGFMWALEVVKDKASKAPFDGNLSVSERIANTCTDLGLICRPLGQSVVLAPPYILTEAQMDEMFDKLEKALDKVFAEVA

SEQ ID NO: 55 - DNA, 1362 bp, Artificial Sequence
  Engineered variant of V. fluvialis transaminase
atgaacaaaccgcagagctgggaaacgcgtgcggaaaccgtgagcctgtatgcctttacccacatgccgagcctacgtcagcgtggcaccatggtggtgacccatggcgaaggcccgtatatcgtggatgtgcatggccgtcgttatctggatgcgaacagcggcctgtggaacatggtggcgggctttgatcataaaggcctgattgatgcggcgaaagcgcagtatgaacgttttccgggctatcatgcgttttacggcctgatgagcgatcagaccgtgatgctgtctgaaaaactggtggaagtgagcccgtttgatagcggccgtgtgtttctgaccaacagcggcagcgaagcgaacgataccatggtgaaaatgctgtggtttctgcatcgtgcggaaggcaaaccgcagaaacgtaaaattctgaccctgaagaacgcgtatcatggctccaccgcggtgagcgcgagcatgaccggcatcccgtataacagcgtgtttggcctgccgctgccgggctttctgcatctgacctgcccgcattattggcgttatggcgaagaaggcgaaaccgaagaacagtttgtcgcgcgtctggcccgtgaactggaagaaaccattcagaaggaaggcgcggataccattgcgggcttttttgcggaaccggtgatgggtgcgggcggtgttattaccccgccaaaaggctattttcaggcgattctgaccatcctgcgcaaatatgatattccggtgatcagcgatgaagtgatttgcggctttggtcgtaccggcaacacctggggctgcgtgacctatgattttaccccggatgcgattattagcagtaaaaacctaaccgcgggtttttttccagtaggagcggtgattttggggccggaactgagcaaacgtctggaaaccgcgattgaagcgatcgaagaatttgatcatggttttaccacaggcggccatccggtgggttgtgcgattgcgctgaaagcgattgatgtggtgatgaacgaaggcctggccgaaaacgtgcgtcgtctggccccgcgttttgaagaacgtctgaaacatattgcggaacgtccgaacattggcgaatatcgtggtattggctttatgtgggcgctggaagtggtgaaagataaagcgagcaaagccccgtttgatggcaacctgagcgtgagcgaacgtattgcgaacacctgcaccgatctgggactgatttgccgaccgttgggccagagcgtggttctggcaccgccgtacattctgaccgaagcgcagatggatgaaatgttcgataaactggaaaaagcgctggataaagtgtttgcggaagtggcgtaa

SEQ ID NO: 56 - protein, 453 aa, Artificial Sequence
  Engineered variant of V. fluvialis transaminase
MNKPQSWETRAETVSLYAFTHMPSLRQRGTMVVTHGEGPYIVDVHGRRYLDANSGLWNMVAGFDHKGLIDAAKAQYERFPGYHAFYGLMSDQTVMLSEKLVEVSPFDSGRVFLTNSGSEANDTMVKMLWFLHRAEGKPQKRKILTLKNAYHGSTAVSASMTGIPYNSVFGLPLPGFLHLTCPHYWRYGEEGETEEQFVARLARELEETIQKEGADTIAGFFAEPVMGAGGVITPPKGYFQAILTILRKYDIPVISDEVICGFGRTGNTWGCVTYDFTPDAIISSKNLTAGFFPVGAVILGPELSKRLETAIEAIEEFDHGFTTGGHPVGCAIALKAIDVVMNEGLAENVRRLAPRFEERLKHIAERPNIGEYRGIGFMWALEVVKDKASKAPFDGNLSVSERIANTCTDLGLICRPLGQSVVLAPPYILTEAQMDEMFDKLEKALDKVFAEVA

SEQ ID NO: 57 - DNA, 1362 bp, Artificial Sequence
  Engineered variant of V. fluvialis transaminase
atgaacaaaccgcagagctgggaaacgcgtgcggaaaccgtgagcctgtatgcctttacccacatgccgagcctacatcagcgtggcaccatggtggtgacccatggcgaaggcccgtatatcgtggatgtgcatggccgtcgttatctggatgcgaacagcggcctgttcaacatggtggcgggctttgatcataaaggcctgattgatgcggcgaaagcgcagtatgaacgttttccgggctatcatgcgttttacggcgccatgagcgatcagaccgtgatgctgtctgaaaaactggtggaagtgagcccgtttgatagcggccgtgtgtttctgaccaacagcggcagcgaagcgaacgataccatggtgaaaatgctgtggtttctgcatcgtgcggaaggcaaaccgcagaaacgtaaaattctgaccctgaagaacgcgtatcatggctccaccgcggtgagcgcgagcatgaccggccttccgtataacagcgtgtttggcctgccgctgccgggctttctgcatctgacctgcccgcattattggcgttatggcgaagaaggcgaaaccgaagaacagtttgtcgcgcgtctggcccgtgaactggaagaaaccattcagaaggaaggcgcggataccattgcgggcttttttgcggaaccggtgatgggtgcgggcggtgttattaccccgccaaaaggctattttcaggcgattctgaccatcctgcgcaaatatgatattccggtgatcagcgatgaagtgatttgcggctttggtcgtaccggcaacacctggggctgcgtgacctatgattttaccccggatgcgattattagcagtaaaaacctaaccgcgggtttttttccagtaggagcggtgattttggggccggaactgagcaaacgtctggaaaccgcgattgaagcgatcgaagaatttgatcatggttttaccacaggcggccatccggtgggttgtgcgattgcgctgaaagcgattgatgtggtgatgaacgaaggcctggccgaaaacgtgcgtcgtctggccccgcgttttgaagaacgtctgaaacatattgcggaacgtccgaacattggcgaatatcgtggtattggctttatgtgggcgctggaagtggtgaaagataaagcgagcaaagccccgtttgatggcaacctgagcgtgagcgaacgtattgcgaacacctgcaccgatctgggactgatttgccgaccgttgggccagagcgtggttctggcaccgccgtacattctgaccgaagcgcagatggatgaaatgttcgataaactggaaaaagcgctggataaagtgtttgcggaagtggcgtaa

SEQ ID NO: 58 - protein, 453 aa, Artificial Sequence
  Engineered variant of V. fluvialis transaminase
MNKPQSWETRAETVSLYAFTHMPSLHQRGTMVVTHGEGPYIVDVHGRRYLDANSGLFNMVAGFDHKGLIDAAKAQYERFPGYHAFYGAMSDQTVMLSEKLVEVSPFDSGRVFLTNSGSEANDTMVKMLWFLHRAEGKPQKRKILTLKNAYHGSTAVSASMTGLPYNSVFGLPLPGFLHLTCPHYWRYGEEGETEEQFVARLARELEETIQKEGADTIAGFFAEPVMGAGGVITPPKGYFQAILTILRKYDIPVISDEVICGFGRTGNTWGCVTYDFTPDAIISSKNLTAGFFPVGAVILGPELSKRLETAIEAIEEFDHGFTTGGHPVGCAIALKAIDVVMNEGLAENVRRLAPRFEERLKHIAERPNIGEYRGIGFMWALEVVKDKASKAPFDGNLSVSERIANTCTDLGLICRPLGQSVVLAPPYILTEAQMDEMFDKLEKALDKVFAEVA

SEQ ID NO: 59 - DNA, 1362 bp, Artificial Sequence
  Engineered variant of V. fluvialis transaminase
atgaacaaaccgcagagctgggaaacgcgtgcggaaaccgtgagcctgtatgcctttacccacatgccgagcctacgtcagcgtggcaccatggtggtgacccatggcgaaggcccgtatatcgtggatgtgcatggccgtcgttatctggatgcgaacagcggcctgttcaacatggtggcgggctttgatcataaaggcctgattgatgcggcgaaagcgcagtatgaacgttttccgggctatcatgcgttttacggccgtatgagcgatcagaccgtgatgctgtctgaaaaactggtggaagtgagcccgtttgatagcggccgtgtgtttctgaccaacagcggcagcgaagcgaacgataccatggtgaaaatgctgtggtttctgcatcgtgcggaaggcaaaccgcagaaacgtaaaattctgaccctgaagcgtgcgtatcatggctccaccgcggtgagcgcgagcatgaccggccttccgtataacagcgtgtttggcctgccgctgccgggctttctgcatctgacctgcccgcattattggcgttatggcgaagaaggcgaaaccgaagaacagtttgtcgcgcgtctggcccgtgaactggaagaaaccattcagaaggaaggcgcggataccattgcgggcttttttgcggaaccggtgatgggtgcgggcggtgttattaccccgccaaaaggctattttcaggcgattctgaccatcctgcgcaaatatgatattccggtgatcagcgatgaagtgatttgcggctttggtcgtaccggcaacacctggggctgcgtgacctatgattttaccccggatgcgattattagcagtaaaaacctaaccgcgggtttttttccagtaggagcggtgattttggggccggaactgagcaaacgtctggaaaccgcgattgaagcgatcgaagaatttgatcatggttttaccacaggcggccatccggtgggttgtgcgattgcgctgaaagcgattgatgtggtgatgaacgaaggcctggccgaaaacgtgcgtcgtctggccccgcgttttgaagaacgtctgaaacatattgcggaacgtccgaacattggcgaatatcgtggtattggctttatgtgggcgctggaagtggtgaaagataaagcgagcaaagccccgtttgatggcaacctgagcgtgagcgaacgtattgcgaacacctgcaccgatctgggactgatttgccgaccgttgggccagagcgtggttctggcaccgccgtacattctgaccgaagcgcagatggatgaaatgttcgataaactggaaaaagcgctggataaagtgtttgcggaagtggcgtaa

SEQ ID NO: 60 - protein, 453 aa, Artificial Sequence
  Engineered variant of V. fluvialis transaminase
MNKPQSWETRAETVSLYAFTHMPSLRQRGTMVVTHGEGPYIVDVHGRRYLDANSGLFNMVAGFDHKGLIDAAKAQYERFPGYHAFYGRMSDQTVMLSEKLVEVSPFDSGRVFLTNSGSEANDTMVKMLWFLHRAEGKPQKRKILTLKRAYHGSTAVSASMTGLPYNSVFGLPLPGFLHLTCPHYWRYGEEGETEEQFVARLARELEETIQKEGADTIAGFFAEPVMGAGGVITPPKGYFQAILTILRKYDIPVISDEVICGFGRTGNTWGCVTYDFTPDAIISSKNLTAGFFPVGAVILGPELSKRLETAIEAIEEFDHGFTTGGHPVGCAIALKAIDVVMNEGLAENVRRLAPRFEERLKHIAERPNIGEYRGIGFMWALEVVKDKASKAPFDGNLSVSERIANTCTDLGLICRPLGQSVVLAPPYILTEAQMDEMFDKLEKALDKVFAEVA

SEQ ID NO: 61 - DNA, 1362 bp, Artificial Sequence
  Engineered variant of V. fluvialis transaminase
atgaacaaaccgcagagctgggaaacgcgtgcggaaaccgtgagcctgtatgcctttacccacatgccgagcctacatcagcgtggcaccatggtggtgacccatggcgaaggcccgtatatcgtggatgtgcatggccgtcgttatctggatgcgaacagcggcctgttcaacatggtggcgggctttgatcataaaggcctgattgatgcggcgaaagcgcagtatgaacgttttccgggctatcatgcgttttacggccgcatgagcgatcagaccgtgatgctgtctgaaaaactggtggaagtgagcccgtttgatagcggccgtgtgtttctgaccaacagcggcagcgaagcgaacgataccatggtgaaaatgctgtggtttctgcatcgtgcggaaggcaaaccgcagaaacgtaaaattctgaccctgaagaacgcgtatcatggctccaccgcggtgagcgcgagcatgaccggcatcccgtataacagcgtgtttggcctgccgctgccgggctttctgcatctgacctgcccgcattattggcgttatggcgaagaaggcgaaaccgaagaacagtttgtcgcgcgtctggcccgtgaactggaagaaaccattcagaaggaaggcgcggataccattgcgggcttttttgcggaaccggtgatgggtgcgggcggtgttattaccccgccaaaaggctattttcaggcgattctgaccatcctgcgcaaatatgatattccggtgatcagcgatgaagtgatttgcggctttggtcgtaccggcaacacctggggctgcgtgacctatgattttaccccggatgcgattattagcagtaaaaacctaaccgcgggtttttttccagtaggagcggtgattttggggccggaactgagcaaacgtctggaaaccgcgattgaagcgatcgaagaatttgatcatggttttaccacaggcggccatccggtgggttgtgcgattgcgctgaaagcgattgatgtggtgatgaacgaaggcctggccgaaaacgtgcgtcgtctggccccgcgttttgaagaacgtctgaaacatattgcggaacgtccgaacattggcgaatatcgtggtattggctttatgtgggcgctggaagtggtgaaagataaagcgagcaaagccccgtttgatggcaacctgagcgtgagcgaacgtattgcgaacacctgcaccgatctgggactgatttgccgaccgttgggccagagcgtggttctggcaccgccgtacattctgaccgaagcgcagatggatgaaatgttcgataaactggaaaaagcgctggataaagtgtttgcggaagtggcgtaa

SEQ ID NO: 62 - protein, 453 aa, Artificial Sequence
  Engineered variant of V. fluvialis transaminase
MNKPQSWETRAETVSLYAFTHMPSLHQRGTMVVTHGEGPYIVDVHGRRYLDANSGLFNMVAGFDHKGLIDAAKAQYERFPGYHAFYGRMSDQTVMLSEKLVEVSPFDSGRVFLTNSGSEANDTMVKMLWFLHRAEGKPQKRKILTLKNAYHGSTAVSASMTGIPYNSVFGLPLPGFLHLTCPHYWRYGEEGETEEQFVARLARELEETIQKEGADTIAGFFAEPVMGAGGVITPPKGYFQAILTILRKYDIPVISDEVICGFGRTGNTWGCVTYDFTPDAIISSKNLTAGFFPVGAVILGPELSKRLETAIEAIEEFDHGFTTGGHPVGCAIALKAIDVVMNEGLAENVRRLAPRFEERLKHIAERPNIGEYRGIGFMWALEVVKDKASKAPFDGNLSVSERIANTCTDLGLICRPLGQSVVLAPPYILTEAQMDEMFDKLEKALDKVFAEVA

SEQ ID NO: 63 - DNA, 1362 bp, Artificial Sequence
  Engineered variant of V. fluvialis transaminase
atgaacaaaccgcagagctgggaaacgcgtgcggaaacctatagcctgtatgcctttacccacatgccgagcctacatcagcgtggcaccatggtggtgacccatggcgaaggcccgtatatcgtggatgtgcatggccgtcgttatctggatgcgaacagcggcctgtggaacatggtggcgggctttgatcataaaggcctgattgatgcggcgaaagcgcagtatgaacgttttccgggctatcatgcgttttacggcctgatgagcgatcagaccgtgatgctgtctgaaaaactggtggaagtgagcccgtttgatagcggccgtgtgttttataccaacagcggcagcgaagcgaacgataccatggtgaaaatgctgtggtttctgcatcgtgcggaaggcaaaccgcagaaacgtaaaattctgaccctgaagaacgcgtatcatggctccaccgcggtgagcgcgagcatgaccggcatcccgtataacagcgtgtttggcctgccggctccgggctttctgcatctgacctgcccgcattattggcgttatggcgaagaaggcgaaaccgaagaacagtttgtcgcgcgtctggcccgtgaactggaagaaaccattcagaaggaaggcgcggataccattgcgggcttttttgcggaaccggtgatgggtgcgggcggtgttattaccccgccaaaaggctattttcaggcgattctgaccatcctgcgcaaatatgatattccggtgatcagcgatgaagtgatttgcggctttggtcgtaccggcaacacctggggctgcgtgacctatgattttaccccggatgcgattattagcgccaaaaacctaaccgcgggtttttttccagtaggagcggtgattttggggccggaactgagcaaacgtctggaaaccgcgattgaagcgatcgaagaatttgatcatggttttaccacaggcggccatccggtgggttgtgcgattgcgctgaaagcgattgatgtggtgatgaacgaaggcctggccgaaaacgtgcgtcgtctggccccgcgttttgaagaacgtctgaaacatattgcggaacgtccgaacattggcgaatatcgtggtattggctttatgtgggcgctggaagtggtgaaagataaagcgagcaaagccccgtttgatggcaacctgagcgtgggtgaacgtattgcgaacacctgcaccgatctgggactgatttgtcgaccgatgggccagagcgtggttctggtgccgccgtacattctgaccgaagcgcagatggatgaaatgttcgataaactggaaaaagcgctggataaagtgtttgcggaagtggcgtaa

SEQ ID NO: 64 - protein, 453 aa, Artificial Sequence
  Engineered variant of V. fluvialis transaminase
MNKPQSWETRAETYSLYAFTHMPSLHQRGTMVVTHGEGPYIVDVHGRRYLDANSGLWNMVAGFDHKGLIDAAKAQYERFPGYHAFYGLMSDQTVMLSEKLVEVSPFDSGRVFYTNSGSEANDTMVKMLWFLHRAEGKPQKRKILTLKNAYHGSTAVSASMTGIPYNSVFGLPAPGFLHLTCPHYWRYGEEGETEEQFVARLARELEETIQKEGADTIAGFFAEPVMGAGGVITPPKGYFQAILTILRKYDIPVISDEVICGFGRTGNTWGCVTYDFTPDAIISAKNLTAGFFPVGAVILGPELSKRLETAIEAIEEFDHGFTTGGHPVGCAIALKAIDVVMNEGLAENVRRLAPRFEERLKHIAERPNIGEYRGIGFMWALEVVKDKASKAPFDGNLSVGERIANTCTDLGLICRPMGQSVVLVPPYILTEAQMDEMFDKLEKALDKVFAEVA

SEQ ID NO: 65 - DNA, 1362 bp, Artificial Sequence
  Engineered variant of V. fluvialis transaminase
atgaacaaaccgcagagctgggaaacgcgtgcggaaacctatagcctgtatgcctttacccacatgccgagcctacatcagcgtggcaccatggtgaccacccatggcgaaggcccgtatatcgtggatgtgcatggccgtcgttatctggatgcgaacagcggcctgtggaacatggtggcgggctttgatcataaaggcctgattgatgcggcgaaagcgcagtatgaacgttttccgggctatcatgcgttttacggcctgatgagcgatcagaccgtgatgctgtctgaaaaactggtggaagtgagcccgtttgatagcggccgtgtgttttataccaacagcggcagcgaagcgaacgataccatggtgaaaatgctgtggtttctgcatcgtgcggaaggcaaaccgcagaaacgtaaaattctgaccctgaagaacgcgtatcatggctccaccgcggtgagcgcgagcatgaccggctttccgtataacagcgtgtttggcctgccggctccgggctttctgcatctgacctgcccgcattattggcgttatggcgaagaaggcgaaaccgaagaacagtttgtcgcgcgtctggcccgtgaactggaagaaaccattcagaaggaaggcgcggataccattgcgggcttttttgcggaaccggtgatgggtgcgggcggtgttattaccccgccaaaaggctattttcaggcgattctgaccatcctgcgcaaatatgatattccggtgatcagcgatgaagtgatttgcggctttggtcgtaccggcaacacctggggctgcgtgacctatgattttaccccggatgcgattattagcgccaaaaacctaaccgcgggtttttttccagtaggagcggtgattttggggccggaactgagcaaacgtctggaaaccgcgattgaagcgatcgaagaatttgatcatggttttaccacaggcggccatccggtgggttgtgcgattgcgctgaaagcgattgatgtggtgatgaacgaaggcctggccgaaaacgtgcgtcgtctggccccgcgttttgaagaacgtctgaaacatattgcggaacgtccgaacattggcgaatatcgtggtattggctttatgtgggcgctggaagccgtgaaagataaagcgagcaaagccccgtttgatggcaacctgagcgtgggtgaacgtattgcgaacacctgcaccgatctgggactgatttgccgaccgttgggccagagcgtggttctggcaccgccgtacattctgaccgaagcgcagatggatgaaatgttcgataaactggaaaaagcgctggataaagtgtttgcggaagtggcgtaa

SEQ ID NO: 66 - protein, 453 aa, Artificial Sequence
  Engineered variant of V. fluvialis transaminase
MNKPQSWETRAETYSLYAFTHMPSLHQRGTMVTTHGEGPYIVDVHGRRYLDANSGLWNMVAGFDHKGLIDAAKAQYERFPGYHAFYGLMSDQTVMLSEKLVEVSPFDSGRVFYTNSGSEANDTMVKMLWFLHRAEGKPQKRKILTLKNAYHGSTAVSASMTGFPYNSVFGLPAPGFLHLTCPHYWRYGEEGETEEQFVARLARELEETIQKEGADTIAGFFAEPVMGAGGVITPPKGYFQAILTILRKYDIPVISDEVICGFGRTGNTWGCVTYDFTPDAIISAKNLTAGFFPVGAVILGPELSKRLETAIEAIEEFDHGFTTGGHPVGCAIALKAIDVVMNEGLAENVRRLAPRFEERLKHIAERPNIGEYRGIGFMWALEAVKDKASKAPFDGNLSVGERIANTCTDLGLICRPLGQSVVLAPPYILTEAQMDEMFDKLEKALDKVFAEVA

SEQ ID NO: 67 - DNA, 1362 bp, Artificial Sequence
  Engineered variant of V. fluvialis transaminase
atgaacaaaccgcagagctgggaaacgcgtgcggaaacctatagcctgtatgcctttacccacatgccgagcctacatcagcgtggcaccatggtggtgacccatggcgaaggcccgtatatcgtggatgtgcatggccgtcgttatctggatgcgaacagcggcctgtggaacatggtggcgggctttgatcataaaggcctgattgatgcggcgaaagcgcagtatgaacgttttccgggctatcatgcgtttgatggccgtatgagcgatcagaccgtgatgctgtctgaaaaactggtggaagtgagcccgtttgatagcggccgtgtgttttataccaacagcggcagcgaagcgaacgataccatggtgaaaatgctgtggtttctgcatcgtgcggaaggcaaaccgcagaaacgtaaaattctgaccctgaagaacgcgtatcatggctccaccgcggtgagcgcgagcatgaccggctttccgtataacagcgtgtttggcctgccgctgccgggctttctgcatctgacctgcccgcattattggcgttatggcgaagaaggcgaaaccgaagaacagtttgtcgcgcgtctggcccgtgaactggaagaaaccattcagaaggaaggcgcggataccattgcgggcttttttgcggaaccggtgatgggtgcgggcggtgttattaccccgccaaaaggctattttcaggcgattctgaccatcctgcgcaaatatgatattccggtgatcagcgatgaagtgatttgcggctttggtcgtaccggcaacacctggggctgcgtgacctatgattttaccccggatgcgattattagcagtaaaaacctaaccgcgggtttttttccagtaggagcggtgattttggggccggaactgagcaaacgtctggaaaccgcgattgaagcgatcgaagaatttgatcatggttttaccacacacggccatccggtgggttgtgcgattgcgctgaaagcgattgatgtggtgatgaacgaaggcctggccgaaaacgtgcgtcgtctggccccgcgttttgaagaacgtctgaaacatattgcggaacgtccgaacattggcgaatatcgtggtattggctttatgtgggcgctggaagtggtgaaagataaagcgagcaaagccccgtttgatggcaacctgagcgtgggtgaacgtattgcgaacacctgcaccgatctgggactgatttgccgaccgttgggccagagcgtggttctggcaccgccgtacattctgaccgaagcgcagatggatgaaatgttcgataaactggaaaaagcgctggataaagtgtttgcggaagtggcgtaa

SEQ ID NO: 68 - protein, 453 aa, Artificial Sequence
  Engineered variant of V. fluvialis transaminase
MNKPQSWETRAETYSLYAFTHMPSLHQRGTMVVTHGEGPYIVDVHGRRYLDANSGLWNMVAGFDHKGLIDAAKAQYERFPGYHAFDGRMSDQTVMLSEKLVEVSPFDSGRVFYTNSGSEANDTMVKMLWFLHRAEGKPQKRKILTLKNAYHGSTAVSASMTGFPYNSVFGLPLPGFLHLTCPHYWRYGEEGETEEQFVARLARELEETIQKEGADTIAGFFAEPVMGAGGVITPPKGYFQAILTILRKYDIPVISDEVICGFGRTGNTWGCVTYDFTPDAIISSKNLTAGFFPVGAVILGPELSKRLETAIEAIEEFDHGFTTHGHPVGCAIALKAIDVVMNEGLAENVRRLAPRFEERLKHIAERPNIGEYRGIGFMWALEVVKDKASKAPFDGNLSVGERIANTCTDLGLICRPLGQSVVLAPPYILTEAQMDEMFDKLEKALDKVFAEVA

SEQ ID NO: 69 - DNA, 1362 bp, Artificial Sequence
  Engineered variant of V. fluvialis transaminase
atgaacaaaccgcagagctgggaaacgcgtgcggaaacctatagcctgtatgcctttacccacatgccgagcctacatcagcgtggcaccatggtggtgacccatggcgaaggcccgtatatcgtggatgtgcatggccgtcgttatctggatgcgaacagcggcctgtggaacatggtggcgggctttgatcataaaggcctgattgatgcggcgaaagcgcagtatgaacgttttccgggctatcatgcgtttgatggccgtatgagcgatcagaccgtgatgctgtctgaaaaactggtggaagtgagcccgtttgatagcggccgtgtgttttataccaacagcggcagcgaagcgaacgataccatggtgaaaatgctgtggtttctgcatcgtgcggaaggcaaaccgcagaaacgtaaaattctgaccctgaagaacgcgtatcatggctccaccgcggtgagcgcgagcatgaccggctttccgtataacagcaagtttggcctgccgctgccgggctttctgcatctgacctgcccgcattattggcgttatggcgaagaaggcgaaaccgaagaacagtttgtcgcgcgtctggcccgtgaactggaagaaaccattcagaaggaaggcgcggataccattgcgggcttttttgcggaaccggtgatgggtgcgggcggtgttattaccccgccaaaaggctattttcaggcgattctgaccatcctgcgcaaatatgatattccggtgatcagcgatgaagtgatttgcggctttggtcgtaccggcaacacctggggctgcgtgacctatgattttaccccggatgcgattattagcgccaaaaacctaaccgcgggtttttttccagtaggagcggtgattttggggccggaactgagcaaacgtctggaaaccgcgattgaagcgatcgaagaatttgatcatggttttaccacacacggccatccggtgggttgtgcgattgcgctgaaagcgattgatgtggtgatgaacgaaggcctggccgaaaacgtgcgtcgtctggccccgcgttttgaagaacgtctgaaacatattgcggaacgtccgaacattggcgaatatcgtggtattggctttatgtgggcgctggaagccgtgaaagataaagcgagcaaagccccgtttgatggcaacctgagcgtgggtgaacgtattgcgaacacctgcaccgatctgggactgatttgccgaccgttgggccagagcgtggttctggcaccgccgtacattctgaccgaagcgcagatggatgaaatgttcgataaactggaaaaagcgctggataaagtgtttgcggaagtggcgtaa

SEQ ID NO: 70 - protein, 453 aa, Artificial Sequence
  Engineered variant of V. fluvialis transaminase
MNKPQSWETRAETYSLYAFTHMPSLHQRGTMVVTHGEGPYIVDVHGRRYLDANSGLWNMVAGFDHKGLIDAAKAQYERFPGYHAFDGRMSDQTVMLSEKLVEVSPFDSGRVFYTNSGSEANDTMVKMLWFLHRAEGKPQKRKILTLKNAYHGSTAVSASMTGFPYNSKFGLPLPGFLHLTCPHYWRYGEEGETEEQFVARLARELEETIQKEGADTIAGFFAEPVMGAGGVITPPKGYFQAILTILRKYDIPVISDEVICGFGRTGNTWGCVTYDFTPDAIISAKNLTAGFFPVGAVILGPELSKRLETAIEAIEEFDHGFTTHGHPVGCAIALKAIDVVMNEGLAENVRRLAPRFEERLKHIAERPNIGEYRGIGFMWALEAVKDKASKAPFDGNLSVGERIANTCTDLGLICRPLGQSVVLAPPYILTEAQMDEMFDKLEKALDKVFAEVA

SEQ ID NO: 71 - DNA, 1362 bp, Artificial Sequence
  Engineered variant of V. fluvialis transaminase
atgaacaaaccgcagagctgggaaacgcgtgcggaaacctatagcctgtatgcctttacccacatgccgagcctacatcagcgtggcaccatggtggtgacccatggcgaaggcccgtatatcgtggatgtgcatggccgtcgttatctggatgcgaacagcggcctgtggaacatggtggcgggctttgatcataaaggcctgattgatgcggcgaaagcgcagtatgaacgttttccgggctatcatgcgtttgatggccgtatgagcgatcagaccgtgatgctgtctgaaaaactggtggaagtgagcccgtttgatagcggccgtgtgttttataccaacagcggcagcgaagcgaacgataccatggtgaaaatgctgtggtttctgcatcgtgcggaaggcaaaccgcagaaacgtaaaattctgaccctgaagaacgcgtatcatggctccaccgcggtgagcgcgagcatgaccggctttccgtataacagcgtgtttggcctgccggctccgggctttctgcatctgacctgcccgcattattggcgttatggcgaagaaggcgaaaccgaagaacagtttgtcgcgcgtctggcccgtgaactggaagaaaccattcagaaggaaggcgcggataccattgcgggcttttttgcggaaccggtgatgggtgcgggcggtgttattaccccgccaaaaggctattttcaggcgattctgaccatcctgcgcaaatatgatattccggtgatcagcgatgaagtgatttgcggctttggtcgtaccggcaacacctggggctgcgtgacctatgattttaccccggatgcgattattagcgccaaaaacctaaccgcgggtttttttccagtaggagcggtgattttggggccggaactgagcaaacgtctggaaaccgcgattgaagcgatcgaagaatttgatcatggttttaccacacacggccatccggtgggttgtgcgattgcgctgaaagcgattgatgtggtgatgaacgaaggcctggccgaaaacgtgcgtcgtctggccccgcgttttgaagaacgtctgaaacatattgcggaacgtccgaacattggcgaatatcgtggtattggctttatgtgggcgctggaagtggtgaaagataaagcgagcaaagccccgtttgatggcaacctgagcgtgagcgaacgtattgcgaacacctgcaccgatctgggactgatttgccgaccgttgggccagagcgtggttctggcaccgccgtacattctgaccgaagcgcagatggatgaaatgttcgataaactggaaaaagcgctggataaagtgtttgcggaagtggcgtaa

SEQ ID NO: 72 - protein, 453 aa, Artificial Sequence
  Engineered variant of V. fluvialis transaminase
MNKPQSWETRAETYSLYAFTHMPSLHQRGTMVVTHGEGPYIVDVHGRRYLDANSGLWNMVAGFDHKGLIDAAKAQYERFPGYHAFDGRMSDQTVMLSEKLVEVSPFDSGRVFYTNSGSEANDTMVKMLWFLHRAEGKPQKRKILTLKNAYHGSTAVSASMTGFPYNSVFGLPAPGFLHLTCPHYWRYGEEGETEEQFVARLARELEETIQKEGADTIAGFFAEPVMGAGGVITPPKGYFQAILTILRKYDIPVISDEVICGFGRTGNTWGCVTYDFTPDAIISAKNLTAGFFPVGAVILGPELSKRLETAIEAIEEFDHGFTTHGHPVGCAIALKAIDVVMNEGLAENVRRLAPRFEERLKHIAERPNIGEYRGIGFMWALEVVKDKASKAPFDGNLSVSERIANTCTDLGLICRPLGQSVVLAPPYILTEAQMDEMFDKLEKALDKVFAEVA

SEQ ID NO: 73 - DNA, 1362 bp, Artificial Sequence
  Engineered variant of V. fluvialis transaminase
atgaacaaaccgcagagctgggaaacgcgtgcggaaacctatagcctgtatgcctttacccacatgccgagcctacatcagcgtggcaccatggtggtgacccatggcgaaggcccgtatatcgtggatgtgcatggccgtcgttatctggatgcgaacagcggcctgtggaacatggtggcgggctttgatcataaaggcctgattgatgcggcgaaagcgcagtatgaacgttttccgggctatcatgcgtttgatggccgtatgagcgatcagaccgtgatgctgtctgaaaaactggtggaagtgagcccgtttgatagcggccgtgtgttttataccaacagcggcagcgaagcgaacgataccatggtgaaaatgctgtggtttctgcatcgtgcggaaggcaaaccgcagaaacgtaaaattctgaccctgaagaacgcgtatcatggctccaccgcggtgagcgcgagcatgaccggctttccgtataacagcgtgtttggcctgccgctgccgggctttctgcatctgacctgcccgcattattggcgttatggcgaagaaggcgaaaccgaagaacagtttgtcgcgcgtctggcccgtgaactggaagaaaccattcagaaggaaggcgcggataccattgcgggcttttttgcggaaccggtgatgggtgcgggcggtgttattaccccgccaaaaggctattttcaggcgattctgaccatcctgcgcaaatatgatattccggtgatcagcgatgaagtgatttgcggctttggtcgtaccggcaacacctggggctgcgtgacctatgattttaccccggatgcgattattagcagtaaaaacctaaccgcgggtttttttccagtaggagcggtgattttggggccggaactgagcaaacgtctggaaaccgcgattgaagcgatcgaagaatttgatcatggttttaccacaggcggccatccggtgggttgtgcgattgcgctgaaagcgattgatgtggtgatgaacgaaggcctggccgaaaacgtgcgtcgtctggccccgcgttttgaagaacgtctgaaacatattgcggaacgtccgaacattggcgaatatcgtggtattggctttatgtgggcgctggaagccgtgaaagataaagcgagcaaagccccgtttgatggcaacctgagcgtgggtgaacgtattgcgaacacctgcaccgatctgggactgatttgccgaccgttgggccagagcgtggttctggcaccgccgtacattctgaccgaagcgcagatggatgaaatgttcgataaactggaaaaagcgctggataaagtgtttgcggaagtggcgtaa

SEQ ID NO: 74 - protein, 453 aa, Artificial Sequence
  Engineered variant of V. fluvialis transaminase
MNKPQSWETRAETYSLYAFTHMPSLHQRGTMVVTHGEGPYIVDVHGRRYLDANSGLWNMVAGFDHKGLIDAAKAQYERFPGYHAFDGRMSDQTVMLSEKLVEVSPFDSGRVFYTNSGSEANDTMVKMLWFLHRAEGKPQKRKILTLKNAYHGSTAVSASMTGFPYNSVFGLPLPGFLHLTCPHYWRYGEEGETEEQFVARLARELEETIQKEGADTIAGFFAEPVMGAGGVITPPKGYFQAILTILRKYDIPVISDEVICGFGRTGNTWGCVTYDFTPDAIISSKNLTAGFFPVGAVILGPELSKRLETAIEAIEEFDHGFTTGGHPVGCAIALKAIDVVMNEGLAENVRRLAPRFEERLKHIAERPNIGEYRGIGFMWALEAVKDKASKAPFDGNLSVGERIANTCTDLGLICRPLGQSVVLAPPYILTEAQMDEMFDKLEKALDKVFAEVA

SEQ ID NO: 75 - DNA, 1362 bp, Artificial Sequence
  Engineered variant of V. fluvialis transaminase
atgaacaaaccgcagagctgggaaacgcgtgcggaaacctatagcctgtatgcctttacccacatgccgagcctacatcagcgtggcaccatggtggtgacccatggcgaaggcccgtatatcgtggatgtgcatggccgtcgttatctggatgcgaacagcggcctgtggaacatggtggcgggctttgatcataaaggcctgattgatgcggcgaaagcgcagtatgaacgttttccgggctatcatgcgtttgatggccgtatgagcgatcagaccgtgatgctgtctgaaaaactggtggaagtgagcccgtttgatagcggccgtgtgttttataccaacagcggcagcgaagcgaacgataccatggtgaaaatgctgtggtttctgcatcgtgcggaaggcaaaccgcagaaacgtaaaattctgaccctgaagaacgcgtatcatggctccaccgcggtgagcgcgagcatgaccggctttccgtataacagcgtgtttggcctgccggctccgggctttctgcatctgacctgcccgcattattggcgttatggcgaagaaggcgaaaccgaagaacagtttgtcgcgcgtctggcccgtgaactggaagaaaccattcagaaggaaggcgcggataccattgcgggcttttttgcggaaccggtgatgggtgcgggcggtgttattaccccgccaaaaggctattttcaggcgattctgaccatcctgcgcaaatatgatattccggtgatcagcgatgaagtgatttgcggctttggtcgtaccggcaacacctggggctgcgtgacctatgattttaccccggatgcgattattagcagtaaaaacctaaccgcgggtttttttccagtaggagcggtgattttggggccggaactgagcaaacgtctggaaaccgcgattgaagcgatcgaagaatttgatcatggttttaccacaggcggccatccggtgggttgtgcgattgcgctgaaagcgattgatgtggtgatgaacgaaggcctggccgaaaacgtgcgtcgtctggccccgcgttttgaagaacgtctgaaacatattgcggaacgtccgaacattggcgaatatcgtggtattggctttatgtgggcgctggaagtggtgaaagataaagcgagcaaagccccgtttgatggcaacctgagcgtgggtgaacgtattgcgaacacctgcaccgatctgggactgatttgccgaccgttgggccagagcgtggttctggcaccgccgtacattctgaccgaagcgcagatggatgaaatgttcgataaactggaaaaagcgctggataaagagtttgcggaagtggcgtaa

SEQ ID NO: 76 - protein, 453 aa, Artificial Sequence
  Engineered variant of V. fluvialis transaminase
MNKPQSWETRAETYSLYAFTHMPSLHQRGTMVVTHGEGPYIVDVHGRRYLDANSGLWNMVAGFDHKGLIDAAKAQYERFPGYHAFDGRMSDQTVMLSEKLVEVSPFDSGRVFYTNSGSEANDTMVKMLWFLHRAEGKPQKRKILTLKNAYHGSTAVSASMTGFPYNSVFGLPAPGFLHLTCPHYWRYGEEGETEEQFVARLARELEETIQKEGADTIAGFFAEPVMGAGGVITPPKGYFQAILTILRKYDIPVISDEVICGFGRTGNTWGCVTYDFTPDAIISSKNLTAGFFPVGAVILGPELSKRLETAIEAIEEFDHGFTTGGHPVGCAIALKAIDVVMNEGLAENVRRLAPRFEERLKHIAERPNIGEYRGIGFMWALEVVKDKASKAPFDGNLSVGERIANTCTDLGLICRPLGQSVVLAPPYILTEAQMDEMFDKLEKALDKEFAEVA

SEQ ID NO: 77 - DNA, 1362 bp, Artificial Sequence
  Engineered variant of V. fluvialis transaminase
atgaacaaaccgcagagctgggaaacgcgtgcggaaacctatagcctgtatgcctttacccacatgccgagcctacatcagcgtggcaccatggtggtgacccatggcgaaggcccgtatatcgtggatgtgcatggccgtcgttatctggatgcgaacagcggcctgtggaacatggtggcgggctttgatcataaaggcctgattgatgcggcgaaagcgcagtatgaacgttttccgggctatcatgcgtttgatggccgtatgagcgatcagaccgtgatgctgtctgaaaaactggtggaagtgagcccgtttgatagcggccgtgtgttttataccaacagcggcagcgaagcgaacgataccatggtgaaaatgctgtggtttctgcatcgtgcggaaggcaaaccgcagaaacgtaaaattctgaccctgaagaacgcgtatcatggctccaccgcggtgagcgcgagcatgaccggctttccgtataacagcgtgtttggcctgccgctgccgggctttctgcatctgacctgcccgcattattggcgttatggcgaagaaggcgaaaccgaagaacagtttgtcgcgcgtctggcccgtgaactggaagaaaccattcagaaggaaggcgcggataccattgcgggcttttttgcggaaccggtgatgggtgcgggcggtgttattaccccgccaaaaggctattttcaggcgattctgaccatcctgcgcaaatatgatattccggtgatcagcgatgaagtgatttgcggctttggtcgtaccggcaacacctggggctgcgtgacctatgattttaccccggatgcgattattagcgccaaaaacctaaccgcgggtttttttccagtaggagcggtgattttggggccggaactgagcaaacgtctggaaaccgcgattgaagcgatcgaagaatttgatcatggttttaccacacacggccatccggtgggttgtgcgattgcgctgaaagcgattgatgtggtgatgaacgaaggcctggccgaaaacgtgcgtcgtctggccccgcgttttgaagaacgtctgaaacatattgcggaacgtccgaacattggcgaatatcgtggtattggctttatgtgggcgctggaagtggtgaaagataaagcgagcaaagccccgtttgatggcaacctgagcgtgggtgaacgtattgcgaacacctgcaccgatctgggactgatttgccgaccgttgggccagagcgtggttctggcaccgccgtacattctgaccgaagcgcagatggatgaaatgttcgataaactggaaaaagcgctggataaagtgtttgcggaagtggcgtaa

SEQ ID NO: 78 - protein, 453 aa, Artificial Sequence
  Engineered variant of V. fluvialis transaminase
MNKPQSWETRAETYSLYAFTHMPSLHQRGTMVVTHGEGPYIVDVHGRRYLDANSGLWNMVAGFDHKGLIDAAKAQYERFPGYHAFDGRMSDQTVMLSEKLVEVSPFDSGRVFYTNSGSEANDTMVKMLWFLHRAEGKPQKRKILTLKNAYHGSTAVSASMTGFPYNSVFGLPLPGFLHLTCPHYWRYGEEGETEEQFVARLARELEETIQKEGADTIAGFFAEPVMGAGGVITPPKGYFQAILTILRKYDIPVISDEVICGFGRTGNTWGCVTYDFTPDAIISAKNLTAGFFPVGAVILGPELSKRLETAIEAIEEFDHGFTTHGHPVGCAIALKAIDVVMNEGLAENVRRLAPRFEERLKHIAERPNIGEYRGIGFMWALEVVKDKASKAPFDGNLSVGERIANTCTDLGLICRPLGQSVVLAPPYILTEAQMDEMFDKLEKALDKVFAEVA

SEQ ID NO: 79 - DNA, 1362 bp, Artificial Sequence
  Engineered variant of V. fluvialis transaminase
atgaacaaaccgcagagctgggaaacgcgtgcggaaacctatagcctgtatgcctttacccacatgccgagcctacatcagcgtggcaccatggtggtgacccatggcgaaggcccgtatatcgtggatgtgcatggccgtcgttatctggatgcgaacagcggcctgtggaacatggtggcgggctttgatcataaaggcctgattgatgcggcgaaagcgcagtatgaacgttttccgggctatcatgcgtttgatggccgtatgagcgatcagaccgtgatgctgtctgaaaaactggtggaagtgagcccgtttgatagcggccgtgtgttttataccaacagcggcagcgaagcgaacgataccatggtgaaaatgctgtggtttctgcatcgtgcggaaggcaaaccgcagaaacgtaaaattctgaccctgaagaacgcgtatcatggctccaccgcggtgagcgcgagcatgaccggctttccgtataacagcgtgtttggcctgccggctccgggctttctgcatctgacctgcccgcattattggcgttatggcgaagaaggcgaaaccgaagaacagtttgtcgcgcgtctggcccgtgaactggaagaaaccattcagaaggaaggcgcggataccattgcgggcttttttgcggaaccggtgatgggtgcgggcggtgttattaccccgccaaaaggctattttcaggcgattctgaccatcctgcgcaaatatgatattccggtgatcagcgatgaagtgatttgcggctttggtcgtaccggcaacacctggggctgcgtgacctatgattttaccccggatgcgattattagcgccaaaaacctaaccgcgggtttttttccagtaggagcggtgattttggggccggaactgagcaaacgtctggaaaccgcgattgaagcgatcgaagaatttgatcatggttttaccacacacggccatccggtgggttgtgcgattgcgctgaaagcgattgatgtggtgatgaacgaaggcctggccgaaaacgtgcgtcgtctggccccgcgttttgaagaacgtctgaaacatattgcggaacgtccgaacattggcgaatatcgtggtattggctttatgtgggcgctggaagtggtgaaagataaagcgagcaaagccccgtttgatggcaacctgagcgtgggtgaacgtattgcgaacacctgcaccgatctgggactgatttgccgaccgctgggccagagcgtggttctggcaccgccgtacattctgaccgaagcgcagatggatgaaatgttcgataaactggaaaaagcgctggataaagtgtttgcggaagtggcgtaa

SEQ ID NO: 80 - protein, 453 aa, Artificial Sequence
  Engineered variant of V. fluvialis transaminase
MNKPQSWETRAETYSLYAFTHMPSLHQRGTMVVTHGEGPYIVDVHGRRYLDANSGLWNMVAGFDHKGLIDAAKAQYERFPGYHAFDGRMSDQTVMLSEKLVEVSPFDSGRVFYTNSGSEANDTMVKMLWFLHRAEGKPQKRKILTLKNAYHGSTAVSASMTGFPYNSVFGLPAPGFLHLTCPHYWRYGEEGETEEQFVARLARELEETIQKEGADTIAGFFAEPVMGAGGVITPPKGYFQAILTILRKYDIPVISDEVICGFGRTGNTWGCVTYDFTPDAIISAKNLTAGFFPVGAVILGPELSKRLETAIEAIEEFDHGFTTHGHPVGCAIALKAIDVVMNEGLAENVRRLAPRFEERLKHIAERPNIGEYRGIGFMWALEVVKDKASKAPFDGNLSVGERIANTCTDLGLICRPLGQSVVLAPPYILTEAQMDEMFDKLEKALDKVFAEVA

SEQ ID NO: 81 - DNA, 1362 bp, Artificial Sequence
  Engineered variant of V. fluvialis transaminase
atgaacaaaccgcagagctgggaaacgcgtgcggaaacctatagcctgtatgcctttacccacatgccgagcctacatcagcgtggcaccatggtggtgacccatggcgaaggcccgtatctggtggatgtgcatggccgtcgttatctggatgcgaacagcggcctgtataacatggtggcgggctttgatcataaaggcctgattgcggcggcgaaagcgcagtatgaacgttttccgggctatcatgcgttttacggccgtatgagcgatcagaccgtgatgctgtctgaaaaactggtggaagtgagcccgtttccaagcggccgtgtgttttataccaacagcggcagcgaagcgaacgataccatggtgaaaatgctgtggtttctgtttcgtgcggaaggcaaaccgcagaaacgtaaaattctgaccctgaagaacgcgtatcatggctccaccgcggtgagcgcgagcatgaccggccttccgtataacagcgtgtttggcctgccgctgccgggctttctgcatctgacctgcccgcattattggcgttatggcgaagaaggcgaaaccgaagaacagtttgtcgcgcgtctggcccgtgaactggaagaaaccattcagaaggaaggcgcggataccattgcgggcttttttgcggaaccggtgatgggtgcgggcggtgttattaccccgccaaaaggctattttcaggcgattctgaccatcctgcgcaaatatgatattccggtgatcagcgatgaagtgatttgcggctttggtcgtaccggcaacacctggggctgcgtgacctatgattttaccccggatgcgattattagcagtaaaaacctaaccgcgggtttttttccagtaggagcggtgattttggggccggaactgagcaaacgtctggaaaccgcgattgaagcgaatgaggaatttgatcatggttttaccacaggcggccatccggtgggttgtgcgattgcgctgaaagcgattgatgtggtgatgaacgaaggcctggccgaaaacgtgcgtcgtctggccccgcgttttgaagaacgtctgaaacatattgcggaacgtccgaacattggcgaatatcgtggtattggctttatgtgggcgctggaagtggtgaaagataaagcgagcaaagccccgtttgatggtaacctggttgtgagcgaacgtattgcgaacacctgcaccgatctgggactgatttgccgaccgttgggccagagcgtggttctggcaccgccgtacattctgaccgaagcgcagatggatgaaatgttcgataaactggaaaaagcgctggataaagtgtttgcggatgtggcgtaa

SEQ ID NO: 82 - protein, 453 aa, Artificial Sequence
  Engineered variant of V. fluvialis transaminase
MNKPQSWETRAETYSLYAFTHMPSLHQRGTMVVTHGEGPYLVDVHGRRYLDANSGLYNMVAGFDHKGLIAAAKAQYERFPGYHAFYGRMSDQTVMLSEKLVEVSPFPSGRVFYTNSGSEANDTMVKMLWFLFRAEGKPQKRKILTLKNAYHGSTAVSASMTGLPYNSVFGLPLPGFLHLTCPHYWRYGEEGETEEQFVARLARELEETIQKEGADTIAGFFAEPVMGAGGVITPPKGYFQAILTILRKYDIPVISDEVICGFGRTGNTWGCVTYDFTPDAIISSKNLTAGFFPVGAVILGPELSKRLETAIEANEEFDHGFTTGGHPVGCAIALKAIDVVMNEGLAENVRRLAPRFEERLKHIAERPNIGEYRGIGFMWALEVVKDKASKAPFDGNLVVSERIANTCTDLGLICRPLGQSVVLAPPYILTEAQMDEMFDKLEKALDKVFADVA

SEQ ID NO: 83 - DNA, 1362 bp, Artificial Sequence
  Engineered variant of V. fluvialis transaminase
atgaacaaaccgcagagctgggaaacgcgtgcggaaacctatagcctgtatgcctttacccacatgccgagcctacatcagcgtggcaccatggtggtgacccatggcgaaggcccgtatctggtggatgtgcatggcaaccgttatctggatgcgaacagcggcctgtataacatggtggcgggctttgatcataaaggcctgattgatgcggcgaaagcgcagtatgaacgttttccgggctatcatgcgttttacggccgtatgagcgatcagaccgtgatgctgtctgaaaaactggtggaagtgagcccgtttgatagcggccgtgtgttttataccaacagcggcagcgaagcgaacgataccatggtgaaaatgctgtggtttctgcatcgtgcggaaggcaaaccgcagaaacgtaaaattctgaccctgaagaacgcgtatcatggctccaccgcggtgagcgcgagcatgaccggccttccgtataacagcgtgtttggcctgccgctgccgggctttctgcatctgacctgcccgcattattggcgttatggcgaagaaggcgaaaccgaagaacagtttgtcgcgcgtctggcccgtgaactggaagaaaccattcagaaggaaggcgcggataccattgcgggcttttttgcggaaccggtgatgggtgcgggcggtgttattaccccgccaaaaggctattttcaggcgattctgaccatcctgcgcaaatatgatattccggtgatcagcgatgaagtgatttgcggctttggtcgtaccggcaacacctggggctgcgtgacctatgattttaccccggatgcgattattagcagtaaaaacctaaccgcgggtttttttccagtaggagcggtgattttggggccggaactgagcaaacgtctggaaaccgcgattgaagcgattggggaatttgatcatggttttaccacaggcggccatccggtgggttgtgcgattgcgctgaaagcgattgatgtggtgatgaacgaaggcctggccgaaaacgtgcgtcgtctggccccgcgttttgaagaacgtctgaaacatattgcggaacgtccgaacattggcgaatatcgtggtattggctttatgtgggcgctggaagtggtgaaagataaagcgagcaaagccccgtttgatggtaacctggttgtgagcgaacgtattgcgaacacctgcaccgatctgggactgatttgccgaccgttgggccagagcgtggttatcgcgccgccgtacattctgaccgaagcgcagatggatgaaatgttcgataaactggaaaaagcgctggataaagtgtttgcggaagtggcgtaa

SEQ ID NO: 84 - protein, 453 aa, Artificial Sequence
  Engineered variant of V. fluvialis transaminase
MNKPQSWETRAETYSLYAFTHMPSLHQRGTMVVTHGEGPYLVDVHGNRYLDANSGLYNMVAGFDHKGLIDAAKAQYERFPGYHAFYGRMSDQTVMLSEKLVEVSPFDSGRVFYTNSGSEANDTMVKMLWFLHRAEGKPQKRKILTLKNAYHGSTAVSASMTGLPYNSVFGLPLPGFLHLTCPHYWRYGEEGETEEQFVARLARELEETIQKEGADTIAGFFAEPVMGAGGVITPPKGYFQAILTILRKYDIPVISDEVICGFGRTGNTWGCVTYDFTPDAIISSKNLTAGFFPVGAVILGPELSKRLETAIEAIGEFDHGFTTGGHPVGCAIALKAIDVVMNEGLAENVRRLAPRFEERLKHIAERPNIGEYRGIGFMWALEVVKDKASKAPFDGNLVVSERIANTCTDLGLICRPLGQSVVIAPPYILTEAQMDEMFDKLEKALDKVFAEVA

SEQ ID NO: 85 - DNA, 1362 bp, Artificial Sequence
  Engineered variant of V. fluvialis transaminase
atgaacaaaccgcagagctgggaaacgcgtgcggaaacctatagcctgtatgcctttacccacatgccgagcctacatcagcgtggcaccatggtggtgacccatggcgaaggcccgtatctggtggatgtgcatggccgtcgttatctggatgcgaacagcggcctgtataacatggtggcgggctttgatcataaaggcctgattgatgcggcgaaagcgcagtatgaacgttttccgggctatcatgcgttttacggccgtatgagcgatcagaccgtgatgctgtctgaaaaactggtggaagtgagcccgtttgatagcggccgtgtgttttataccaacagcggcagcgaagcgaacgataccatggtgaaaatgctgtggtttctgcatcgtgcggaaggcaaaccgcagaaacgtaaaattctgaccctgaagaacgcgtatcatggctccaccgcggtgagcgcgagcatgaccggccttccgtataacagcgtgtttggcctgccgctgccgggctttctgcatctgacctgcccgcattattggcgttatggcgaagaaggcgaaaccgaagaacagtttgtcgcgcgtctggcccgtgaactggaagaaaccattcagaaggaaggcgcggataccattgcgggcttttttgcggaaccggtgatgggtgcgggcggtgttattaccccgccaaaaggctattttcaggcgattctgaccatcctgcgcaaatatgatattccggtgatcagcgatgaagtgatttgcggctttggtcgtaccggcaacacctggggctgcgtgacctatgattttaccccggatgcgattattagcagtaaaaacctaaccgcgggtttttttccagtaggagcggtgattttggggccggaactgagcaaacgtctggaaaccgcgattgaagcgattggggaatttgatcatggttttaccacaggcggccatccggtgggttgtgcgattgcgctgaaagcgattgatgtggtgatgaacgaaggcctggccgaaaacgtgcgtcgtctggccccgcgttttgaagaacgtctgaaacatattgcggaacgtccgaacattggcgaatatcgtggtattggctttatgtgggcgctggaagtggtgaaagataaagcgagcaaagccccgtttgatggtaacctggttgtgagcgaacgtattgcgaacacctgcaccgatctgggactgatttgccgaccgttgggccagagcgtggttctggcgccgccgtacattctgaccgaagcgcagatggatgaaatgttcgataaactggaaaaagcgctggataaagtgtttgcggaagtggcgtaa

SEQ ID NO: 86 - protein, 453 aa, Artificial Sequence
  Engineered variant of V. fluvialis transaminase
MNKPQSWETRAETYSLYAFTHMPSLHQRGTMVVTHGEGPYLVDVHGRRYLDANSGLYNMVAGFDHKGLIDAAKAQYERFPGYHAFYGRMSDQTVMLSEKLVEVSPFDSGRVFYTNSGSEANDTMVKMLWFLHRAEGKPQKRKILTLKNAYHGSTAVSASMTGLPYNSVFGLPLPGFLHLTCPHYWRYGEEGETEEQFVARLARELEETIQKEGADTIAGFFAEPVMGAGGVITPPKGYFQAILTILRKYDIPVISDEVICGFGRTGNTWGCVTYDFTPDAIISSKNLTAGFFPVGAVILGPELSKRLETAIEAIGEFDHGFTTGGHPVGCAIALKAIDVVMNEGLAENVRRLAPRFEERLKHIAERPNIGEYRGIGFMWALEVVKDKASKAPFDGNLVVSERIANTCTDLGLICRPLGQSVVLAPPYILTEAQMDEMFDKLEKALDKVFAEVA

SEQ ID NO: 87 - DNA, 1362 bp, Artificial Sequence
  Engineered variant of V. fluvialis transaminase
atgaacaaaccgcagagctgggaaacgcgtgcggaaacctatagcctgtatgcctttacccacatgccgagcctacatcagcgtggcaccatggtggtgacccatggcgaaggcccgtatctggtggatgtgcatggccgtcgttatctggatgcgaacagcggcctgtataacatggtggcgggctttgatcataaaggcctgattgatgcggcgaaagcgcagtatgaacgttttccgggctatcatgcgttttacggccgtatgagcgatcagaccgtgatgctgtctgaaaaactggtggaagtgagcccgtttccaagcggccgtgtgttttataccaacagcggcagcgaagcgaacgataccatggtgaaaatgctgtggtttctgtttcgtgcggaaggcaaaccgcagaaacgtaaaattctgaccctgaagaacgcgtatcatggctccaccgcggtgagcgcgagcatgaccggccttccgtataacagcgtgtttggcctgccgctgccgggctttctgcatctgacctgcccgcattattggcgttatggcgaagaaggcgaaaccgaagaacagtttgtcgcgcgtctggcccgtgaactggaagaaaccattcagaaggaaggcgcggataccattgcgggcttttttgcggaaccggtgatgggtgcgggcggtgttattaccccgccaaaaggctattttcaggcgattctgaccatcctgcgcaaatatgatattccggtgatcagcgatgaagtgatttgcggctttggtcgtaccggcaacacctggggctgcgtgacctatgattttaccccggatgcgattattagcagtaaaaacctaaccgcgggtttttttccagtaggagcggtgattttggggccggaactgagcaaacgtctggaaaccgcgattgaagcgattggggaatttgatcatggttttaccacaggcggccatccggtgggttgtgcgattgcgctgaaagcgattgatgtggtgatgaacgaaggcctggccgaaaacgtgcgtcgtctggccccgcgttttgaagaacgtctgaaacatattgcggaacgtccgaacattggcgaatatcgtggtattggctttatgtgggcgctggaagtggtgaaagataaagcgagcaaagccccgtttgatccaaacctgtgggtgagcgaacgtattgcgaacacctgcaccgatctgggactgatttgccgaccgttgggccagagcgtggttctggcgccgccgtacattctgacggaagcgcagatggatgaaatgttcgataaactggaaaaagcgctggataaagtgtttgcggaagtggcgtaa

SEQ ID NO: 88 - protein, 453 aa, Artificial Sequence
  Engineered variant of V. fluvialis transaminase
MNKPQSWETRAETYSLYAFTHMPSLHQRGTMVVTHGEGPYLVDVHGRRYLDANSGLYNMVAGFDHKGLIDAAKAQYERFPGYHAFYGRMSDQTVMLSEKLVEVSPFPSGRVFYTNSGSEANDTMVKMLWFLFRAEGKPQKRKILTLKNAYHGSTAVSASMTGLPYNSVFGLPLPGFLHLTCPHYWRYGEEGETEEQFVARLARELEETIQKEGADTIAGFFAEPVMGAGGVITPPKGYFQAILTILRKYDIPVISDEVICGFGRTGNTWGCVTYDFTPDAIISSKNLTAGFFPVGAVILGPELSKRLETAIEAIGEFDHGFTTGGHPVGCAIALKAIDVVMNEGLAENVRRLAPRFEERLKHIAERPNIGEYRGIGFMWALEVVKDKASKAPFDPNLWVSERIANTCTDLGLICRPLGQSVVLAPPYILTEAQMDEMFDKLEKALDKVFAEVA

SEQ ID NO: 89 - DNA, 1362 bp, Artificial Sequence
  Engineered variant of V. fluvialis transaminase
atgaacaaaccgcagagctgggaaacgcgtgcggaaacctatagcctgtatgcctttacccacatgccgagcctacatcagcgtggcaccatggtggtgacccatggcgaaggcccgtatctggtggatgtgcatggccgtcgttatctggatgcgaacagcggcctgtggaacatggtggcgggctttgatcataaaggcctgattgatgcggcgaaagcgcagtatgaacgttttccgggctatcatgcgttttacggccgtatgagcgatcagaccgtgatgctgtctgaaaaactggtggaagtgagcccgtttccaagcggccgtgtgttttataccaacagcggcagcgaagcgaacgataccatggtgaaaatgctgtggtttctgtttcgtgcggaaggcaaaccgcagaaacgtaaaattctgaccctgaagaacgcgtatcatggctccaccgcggtgagcgcgagcatgaccggccttccgtataacagcgtgtttggcctgccgctgccgggctttctgcatctgacctgcccgcattattggcgttatggcgaagaaggcgaaaccgaagaacagtttgtcgcgcgtctggcccgtgaactggaagaaaccattcagaaggaaggcgcggataccattgcgggcttttttgcggaaccggtgatgggtgcgggcggtgttattaccccgccaaaaggctattttcaggcgattctgaccatcctgcgcaaatatgatattccggtgatcagcgatgaagtgatttgcggctttggtcgtaccggcaacacctggggctgcgtgacctatgattttaccccggatgcgattattagcagtaaaaacctaaccgcgggtttttttccagtaggagcggtgattttggggccggaactgagcaaacgtctggaaaccgcgattgaagcgattgaagaatttgatcatggttttaccacaggcggccatccggtgggttgtgcgattgcgctgaaagcgattgatgtggtgatgaacgaaggcctggccgaaaacgtgcgtcgtctggccccgcgttttgaagaacgtctgaaacatattgcggaacgtccgaacattggcgaatatcgtggtattggctttatgtgggcgctggaagtggtgaaagataaagcgagcaaagccccgtttgatggtaacctggttgtgagcgaacgtattgcgaacacctgcaccgatctgggactgatttgccgaccgttgggccagagcgtggttctggcgccgccgtacattctgaccgaagcgcagatggatgaaatgttcgataaactggaaaaagcgctggataaagtgtttgcggatgtggcgtaa

SEQ ID NO: 90 - protein, 453 aa, Artificial Sequence
  Engineered variant of V. fluvialis transaminase
MNKPQSWETRAETYSLYAFTHMPSLHQRGTMVVTHGEGPYLVDVHGRRYLDANSGLWNMVAGFDHKGLIDAAKAQYERFPGYHAFYGRMSDQTVMLSEKLVEVSPFPSGRVFYTNSGSEANDTMVKMLWFLFRAEGKPQKRKILTLKNAYHGSTAVSASMTGLPYNSVFGLPLPGFLHLTCPHYWRYGEEGETEEQFVARLARELEETIQKEGADTIAGFFAEPVMGAGGVITPPKGYFQAILTILRKYDIPVISDEVICGFGRTGNTWGCVTYDFTPDAIISSKNLTAGFFPVGAVILGPELSKRLETAIEAIEEFDHGFTTGGHPVGCAIALKAIDVVMNEGLAENVRRLAPRFEERLKHIAERPNIGEYRGIGFMWALEVVKDKASKAPFDGNLVVSERIANTCTDLGLICRPLGQSVVLAPPYILTEAQMDEMFDKLEKALDKVFADVA

SEQ ID NO: 91 - DNA, 1362 bp, Artificial Sequence
  Engineered variant of V. fluvialis transaminase
atgaacaaaccgcagagctgggaaacgcgtgcggaaacctatagcctgtatgcctttacccacatgccgagcctacatcagcgtggcaccatggtggtgacccatggcgaaggcccgtatctggtggatgtgcatggccgtcgttatctggatgcgaacagcggcctgtataacatggtggcgggctttgatcataaaggcctgattgatgcggcgaaagcgcagtatgaacgttttccgggctatcatgcgttttacggccgtatgagcgatcagaccgtgatgctgtctgaaaaactggtggaagtgagcccgtttccaagcggccgtgtgttttataccaacagcggcagcgaagcgaacgataccatggtgaaaatgctgtggtttctgtttcgtgcggaaggcaaaccgcagaaacgtaaaattctgaccctgaagaacgcgtatcatggctccaccgcggtgagcgcgagcatgaccggccttccgtataacagcgtgtttggcctgccgctgccgggctttctgcatctgacctgcccgcattattggcgttatggcgaagaaggcgaaaccgaagaacagtttgtcgcgcgtctggcccgtgaactggaagaaaccattcagaaggaaggcgcggataccattgcgggcttttttgcggaaccggtgatgggtgcgggcggtgttattaccccgccaaaaggctattttcaggcgattctgaccatcctgcgcaaatatgatattccggtgatcagcgatgaagtgatttgcggctttggtcgtaccggcaacacctggggctgcgtgacctatgattttaccccggatgcgattattagcagtaaaaacctaaccgcgggtttttttccagtaggagcggtgattttggggccggaactgagcaaacgtctggaaaccgcgattgaagcgaatggggaatttgatcatggttttaccacaggcggccatccggtgggttgtgcgattgcgctgaaagcgattgatgtggtgatgaacgaaggcctggccgaaaacgtgcgtcgtctggccccgcgttttgaagaacgtctgaaacatattgcggaacgtccgaacattggcgaatatcgtggtattggctttatgtgggcgctggaagtggtgaaagataaagcgagcaaagccccgtttgatggtaacctggttgtgagcgaacgtattgcgaacacctgcaccgatctgggactgatttgccgaccgttgggccagagcgtggttatcgcgccgccgtacattctgaccgaagcgcagatggatgaaatgttcgataaactggaaaaagcgctggataaagtgtttgcggatgtggcgtaa

SEQ ID NO: 92 - protein, 453 aa, Artificial Sequence
  Engineered variant of V. fluvialis transaminase
MNKPQSWETRAETYSLYAFTHMPSLHQRGTMVVTHGEGPYLVDVHGRRYLDANSGLYNMVAGFDHKGLIDAAKAQYERFPGYHAFYGRMSDQTVMLSEKLVEVSPFPSGRVFYTNSGSEANDTMVKMLWFLFRAEGKPQKRKILTLKNAYHGSTAVSASMTGLPYNSVFGLPLPGFLHLTCPHYWRYGEEGETEEQFVARLARELEETIQKEGADTIAGFFAEPVMGAGGVITPPKGYFQAILTILRKYDIPVISDEVICGFGRTGNTWGCVTYDFTPDAIISSKNLTAGFFPVGAVILGPELSKRLETAIEANGEFDHGFTTGGHPVGCAIALKAIDVVMNEGLAENVRRLAPRFEERLKHIAERPNIGEYRGIGFMWALEVVKDKASKAPFDGNLVVSERIANTCTDLGLICRPLGQSVVIAPPYILTEAQMDEMFDKLEKALDKVFADVA

SEQ ID NO: 93 - DNA, 1362 bp, Artificial Sequence
  Engineered variant of V. fluvialis transaminase
atgaacaaaccgcagagctgggaaacgcgtgcggaaacctatagcctgtatgcctttacccacatgccgagcctacatcagcgtggcaccatggtggtgacccatggcgaaggcccgtatctggtggatgtgcatggccgtcgttatctggatgcgaacagcggcctgtataacatggtggcgggctttgatcataaaggcctgattgatgcggcgaaagcgcagtatgaacgttttccgggctatcatgcgttttacggccgtatgagcgatcagaccgtgatgctgtctgaaaaactggtggaagtgagcccgtttccaagcggccgtgtgttttataccaacagcggcagcgaagcgaacgataccatggtgaaaatgctgtggtttctgtttcgtgcggaaggcaaaccgcagaaacgtaaaattctgaccctgaagaacgcgtatcatggctccaccgcggtgagcgcgagcatgaccggccttccgtataacagcgtgtttggcctgccgctgccgggctttctgcatctgacctgcccgcattattggcgttatggcgaagaaggcgaaaccgaagaacagtttgtcgcgcgtctggcccgtgaactggaagaaaccattcagaaggaaggcgcggataccattgcgggcttttttgcggaaccggtgatgggtgcgggcggtgttattaccccgccaaaaggctattttcaggcgattctgaccatcctgcgcaaatatgatattccggtgatcagcgatgaagtgatttgcggctttggtcgtaccggcaacacctggggctgcgtgacctatgattttaccccggatgcgattattagcagtaaaaacctaaccgcgggtttttttccagtaggagcggtgattttggggccggaactgagcaaacgtctggaaaccgcgattgaagcgattggggaatttgatcatggttttaccacaggcggccatccggtgggttgtgcgattgcgctgaaagcgattgatgtggtgatgaacgaaggcctggccgaaaacgtgcgtcgtctggccccgcgttttgaagaacgtctgaaacatattgcggaacgtccgaacattggcgaatatcgtggtattggctttatgtgggcgctggaagtggtgaaagataaagcgagcaaagccccgtttgatggtaacctggttgtgagcgaacgtattgcgaacacctgcaccgatctgggactgatttgccgaccgttgggccagagcgtggttatcgcgccgccgtacattctgaccgaagcgcagatggatgaaatgttcgataaactggaaaaagcgctggataaagtgtttgcggaagtggcgtaa

SEQ ID NO: 94 - protein, 453 aa, Artificial Sequence
  Engineered variant of V. fluvialis transaminase
MNKPQSWETRAETYSLYAFTHMPSLHQRGTMVVTHGEGPYLVDVHGRRYLDANSGLYNMVAGFDHKGLIDAAKAQYERFPGYHAFYGRMSDQTVMLSEKLVEVSPFPSGRVFYTNSGSEANDTMVKMLWFLFRAEGKPQKRKILTLKNAYHGSTAVSASMTGLPYNSVFGLPLPGFLHLTCPHYWRYGEEGETEEQFVARLARELEETIQKEGADTIAGFFAEPVMGAGGVITPPKGYFQAILTILRKYDIPVISDEVICGFGRTGNTWGCVTYDFTPDAIISSKNLTAGFFPVGAVILGPELSKRLETAIEAIGEFDHGFTTGGHPVGCAIALKAIDVVMNEGLAENVRRLAPRFEERLKHIAERPNIGEYRGIGFMWALEVVKDKASKAPFDGNLVVSERIANTCTDLGLICRPLGQSVVIAPPYILTEAQMDEMFDKLEKALDKVFAEVA

SEQ ID NO: 95 - DNA, 1362 bp, Artificial Sequence
  Engineered variant of V. fluvialis transaminase
atgaacaaaccgcagagctgggaaacgcgtgcggaaacctatagcctgtatgcctttacccacatgccgagcctacatcagcgtggcaccatggtggtgacccatggcgaaggcccgtatctggtggatgtgcatggccgtcgttatctggatgcgaacagcggcctgtataacatggtggcgggctttgatcataaaggcctgattgcggcggcgaaagcgcagtatgaacgttttccgggctatcatgcgttttacggccgtatgagcgatcagaccgtgatgctgtctgaaaaactggtggaagtgagcccgtttccaagcggccgtgtgttttataccaacagcggcagcgaagcgaacgataccatggtgaaaatgctgtggtttctgtttcgtgcggaaggcaaaccgcagaaacgtaaaattctgaccctgaagaacgcgtatcatggctccaccgcggtgagcgcgagcatgaccggccttccgtataacagcgtgtttggcctgccgctgccgggctttctgcatctgacctgcccgcattattggcgttatggcgaagaaggcgaaaccgaagaacagtttgtcgcgcgtctggcccgtgaactggaagaaaccattcagaaggaaggcgcggataccattgcgggcttttttgcggaaccggtgatgggtgcgggcggtgttattaccccgccaaaaggctattttcaggcgattctgaccatcctgcgcaaatatgatattccggtgatcagcgatgaagtgatttgcggctttggtcgtaccggcaacacctggggctgcgtgacctatgattttaccccggatgcgattattagcagtaaaaacctaaccgcgggtttttttccagtaggagcggtgattttggggccggaactgagcaaacgtctggaaaccgcgattgaagcgaatgaggaatttgatcatggttttaccacaggcggccatccggtgggttgtgcgattgcgctgaaagcgattgatgtggtgatgaacgaaggcctggccgaaaacgtgcgtcgtctggccccgcgttttgaagaacgtctgaaacatattgcggaacgtccgaacattggcgaatatcgtggtattggctttatgtgggcgctggaagtggtgaaagataaagcgagcaaagccccgtttgatggtaacctgtgggtgagcgaacgtattgcgaacacctgcaccgatctgggactgatttgccgaccgttgggcagcagcgtggttctggcgccgccgtacattctgaccgaagcgcagatggatgaaatgttcgataaactggaaaaagcgctggataaagtgtttgcggaagtggcgtaa

SEQ ID NO: 96 - protein, 453 aa, Artificial Sequence
  Engineered variant of V. fluvialis transaminase
MNKPQSWETRAETYSLYAFTHMPSLHQRGTMVVTHGEGPYLVDVHGRRYLDANSGLYNMVAGFDHKGLIAAAKAQYERFPGYHAFYGRMSDQTVMLSEKLVEVSPFPSGRVFYTNSGSEANDTMVKMLWFLFRAEGKPQKRKILTLKNAYHGSTAVSASMTGLPYNSVFGLPLPGFLHLTCPHYWRYGEEGETEEQFVARLARELEETIQKEGADTIAGFFAEPVMGAGGVITPPKGYFQAILTILRKYDIPVISDEVICGFGRTGNTWGCVTYDFTPDAIISSKNLTAGFFPVGAVILGPELSKRLETAIEANEEFDHGFTTGGHPVGCAIALKAIDVVMNEGLAENVRRLAPRFEERLKHIAERPNIGEYRGIGFMWALEVVKDKASKAPFDGNLWVSERIANTCTDLGLICRPLGSSVVLAPPYILTEAQMDEMFDKLEKALDKVFAEVA

SEQ ID NO: 97 - DNA, 1362 bp, Artificial Sequence
  Engineered variant of V. fluvialis transaminase
atgaacaaaccgcagagctgggaaacgcgtgcggaaacctatagcctgtatgcctttacccacatgccgagcctacatcagcgtggcacctcagtggtaacccatggcgaaggcccgtatatcgtggatgtgcatggccgtcgttatctggatgcgaacagcggcctgttcaacatggtggcgggctttgatcataaaggcctgattgatgcggcgaaagcgcagtatgaacgttttccgggctatcatgcgttttacggccgtatgagcgatcagaccgtgatgctgtctgaaaaactggtggaagtgagcccgtttgatagcggccgtgtgttttataccaacagcggcagcgaagcgaacgataccatggtgaaaatgctgtggtttctgcatcgtgcggaaggcaaaccgcagaaacgtaaaattctgaccctgaagaacgcgtatcatggctccaccgcggtgagcgcgagcatgaccggcatcccgtataacagcgtgtttggcctgccgctgccgggctttctgcatctgacctgcccgcattattggcgttatggcgaagaaggcgaaaccgaagaacagtttgtcgcgcgtctggcccgtgaactggaagaaaccattcagaaggaaggcgcggataccattgcgggcttttttgcggaaccggtgatgggtgcgggcggtgttattaccccgccaaaaggctattttcaggcgattctgaccatcctgcgcaaatatgatattccggtgatcagcgatgaagtgatttgcggctttggtcgtaccggcaacacctggggctgcgtgacctatgattttaccccggatgcgattattagcagtaaaaacctaaccgcgggtttttttccagtaggagcggtgattttggggccggaactgagcaaacgtctggaaaccgcgattgaagcgaatgaggaatttgatcatggttttaccacaggcggccatccggtgggttgtgcgattgcgctgaaagcgattgatgtggtgatgaacgaaggcctgctggaaaacgtgcgtcgtctggccccgcgttttgaagaacgtctgaaacatattgcggaacgtccgaacattggcgaatatcgtggtattggctttatgtgggcgctggaagtggtgaaagataaagcgagcaaagccccgtttgatccaaacctgtgggtgagcgaacgtattgcgaacacctgcaccgatctgggactgatttgccgaccgttgggccagagcgtggttctggcgccgccgtacattctgaccgaagcgcagatggatgaaatgttcgataaactggaaaaagcgctggataaagtgtttgcggatgtggcgtaa

SEQ ID NO: 98 - protein, 453 aa, Artificial Sequence
  Engineered variant of V. fluvialis transaminase
MNKPQSWETRAETYSLYAFTHMPSLHQRGTSVVTHGEGPYIVDVHGRRYLDANSGLFNMVAGFDHKGLIDAAKAQYERFPGYHAFYGRMSDQTVMLSEKLVEVSPFDSGRVFYTNSGSEANDTMVKMLWFLHRAEGKPQKRKILTLKNAYHGSTAVSASMTGIPYNSVFGLPLPGFLHLTCPHYWRYGEEGETEEQFVARLARELEETIQKEGADTIAGFFAEPVMGAGGVITPPKGYFQAILTILRKYDIPVISDEVICGFGRTGNTWGCVTYDFTPDAIISSKNLTAGFFPVGAVILGPELSKRLETAIEANEEFDHGFTTGGHPVGCAIALKAIDVVMNEGLLENVRRLAPRFEERLKHIAERPNIGEYRGIGFMWALEVVKDKASKAPFDPNLWVSERIANTCTDLGLICRPLGQSVVLAPPYILTEAQMDEMFDKLEKALDKVFADVA

SEQ ID NO: 99 - DNA, 1362 bp, Artificial Sequence
  Engineered variant of V. fluvialis transaminase
atgaacaaaccgcagagctgggaaacgcgtgcggaaacctatagcctgtatgcctttacccacatgccgagcctacatcagcgtggcacctcagtggtaacccatggcgaaggcccgtatatcgtggatgtgcatggccgtcgttatctggatgcgaacagcggcctgttcaacatggtggcgggctttgatcataaaggcctgattgatgcggcgaaagcgcagtatgaacgttttccgggctatcatgcgttttacggccgtatgagcgatcagaccgtgatgctgtctgaaaaactggtggaagtgagcccgtttgatagcggccgtgtgttttataccaacagcggcagcgaagcgaacgataccatggtgaaaatgctgtggtttctgcatcgtgcggaaggcaaaccgcagaaacgtaaaattctgaccctgaagaacgcgtatcatggctccaccgcggtgagcgcgagcatgaccggcatcccgtataacagcgtgtttggcctgccgctgccgggctttctgcatctgacctgcccgcattattggcgttatggcgaagaaggcgaaaccgaagaacagtttgtcgcgcgtctggcccgtgaactggaagaaaccattcagaaggaaggcgcggataccattgcgggcttttttgcggaaccggtgatgggtgcgggcggtgttattaccccgccaaaaggctattttcaggcgattctgaccatcctgcgcaaatatgatattccggtgatcagcgatgaagtgatttgcggctttggtcgtaccggcaacacctggggctgcgtgacctatgattttaccccggatgcgattattagcagtaaaaacctaaccgcgggtttttttccagtaggagcggtgattttggggccggaactgagcaaacgtctggaaaccgcgattgaagcgattggggaatttgatcatggttttaccacaggcggccatccggtgggttgtgcgattgcgctgaaagcgattgatgtggtgatgaacgaaggcctgctggaaaacgtgcgtcgtctggccccgcgttttgaagaacgtctgaaacatattgcggaacgtccgaacattggcgaatatcgtggtattggctttatgtgggcgctggaagtggtgaaagataaagcgagcaaagccccgtttgatggtaacctgttggtgagcgaacgtattgcgaacacctgcaccgatctgggactgatttgccgaccgttgggcagcagcgtggttctggcgccgccgtacattctgaccgaagcgcagatggatgaaatgttcgataaactggaaaaagcgctggataaagtgtttgcggaagtggcgtaa

SEQ ID NO: 100 - protein, 453 aa, Artificial Sequence
  Engineered variant of V. fluvialis transaminase
MNKPQSWETRAETYSLYAFTHMPSLHQRGTSVVTHGEGPYIVDVHGRRYLDANSGLFNMVAGFDHKGLIDAAKAQYERFPGYHAFYGRMSDQTVMLSEKLVEVSPFDSGRVFYTNSGSEANDTMVKMLWFLHRAEGKPQKRKILTLKNAYHGSTAVSASMTGIPYNSVFGLPLPGFLHLTCPHYWRYGEEGETEEQFVARLARELEETIQKEGADTIAGFFAEPVMGAGGVITPPKGYFQAILTILRKYDIPVISDEVICGFGRTGNTWGCVTYDFTPDAIISSKNLTAGFFPVGAVILGPELSKRLETAIEAIGEFDHGFTTGGHPVGCAIALKAIDVVMNEGLLENVRRLAPRFEERLKHIAERPNIGEYRGIGFMWALEVVKDKASKAPFDGNLLVSERIANTCTDLGLICRPLGSSVVLAPPYILTEAQMDEMFDKLEKALDKVFAEVA

SEQ ID NO: 101 - DNA, 1362 bp, Artificial Sequence
  Engineered variant of V. fluvialis transaminase
atgaacaaaccgcagagctgggaaacgcgtgcggaaacctatagcctgtatgcctttacccacatgccgagcctacatcagcgtggcacctcagtggtaacccatggcgaaggcccgtatctggtggatgtgcatggccgtcgttatctggatgcgaacagcggcctgttcaacatggtggcgggctttgatcataaaggcctgattgatgcggcgaaagcgcagtatgaacgttttccgggctatcatgcgttttacggcgccatgagcgatcagaccgtgatgctgtctgaaaaactggtggaagtgagcccgtttgatagcggccgtgtgttttataccaacagcggcagcgaagcgaacgataccatggtgaaaatgctgtggtttctgcatcgtgcggaaggcaaaccgcagaaacgtaaaattctgaccctgaagaacgcgtatcatggctccaccgcggtgagcgcgagcatgaccggcatcccgtataacagcagctttggcctgccgctgccgggctttctgcatctgacctgcccgcattattggcgttatggcgaagaaggcgaaaccgaagaacagtttgtcgcgcgtctggcccgtgaactggaagaaaccattcagaaggaaggcgcggataccattgcgggcttttttgcggaaccggtgatgggtgcgggcggtgttattaccccgccaaaaggctattttcaggcgattctgaccatcctgcgcaaatatgatattccggtgatcagcgatgaagtgatttgcggctttggtcgtaccggcaacacctggggctgcgtgacctatgattttaccccggatgcgattattagcagtaaaaacctaaccgcgggtttttttccagtaggagcggtgattttggggccggaactgagcaaacgtctggaaaccgcgattgaagcgatcgaagaatttgatcatggttttaccacaggcggccatccggtgggttgtgcgattgcgctgaaagcgattgatgtggtgatgaacgaaggcctgctggaaaacgtgcgtcgtctggccccgcgttttgaagaacgtctgaaacatattgcggaacgtccgaacattggcgaatatcgtggtattggctttatgtgggcgctggaagtggtgaaagataaagcgagcaaagccccgtttgatggtaacctggttgtgagcgaacgtattgcgaacacctgcaccgatctgggactgatttgccgaccgttgggccagagcgtggttctggcgccgccgtacattctgaccgaagcgcagatggatgaaatgttcgataaactggaaaaagcgctggataaagtgtttgcggatgtggcgtaa

SEQ ID NO: 102 - protein, 453 aa, Artificial Sequence
  Engineered variant of V. fluvialis transaminase
MNKPQSWETRAETYSLYAFTHMPSLHQRGTSVVTHGEGPYLVDVHGRRYLDANSGLFNMVAGFDHKGLIDAAKAQYERFPGYHAFYGAMSDQTVMLSEKLVEVSPFDSGRVFYTNSGSEANDTMVKMLWFLHRAEGKPQKRKILTLKNAYHGSTAVSASMTGIPYNSSFGLPLPGFLHLTCPHYWRYGEEGETEEQFVARLARELEETIQKEGADTIAGFFAEPVMGAGGVITPPKGYFQAILTILRKYDIPVISDEVICGFGRTGNTWGCVTYDFTPDAIISSKNLTAGFFPVGAVILGPELSKRLETAIEAIEEFDHGFTTGGHPVGCAIALKAIDVVMNEGLLENVRRLAPRFEERLKHIAERPNIGEYRGIGFMWALEVVKDKASKAPFDGNLVVSERIANTCTDLGLICRPLGQSVVLAPPYILTEAQMDEMFDKLEKALDKVFADVA

SEQ ID NO: 103 - DNA, 1362 bp, Artificial Sequence
  Engineered variant of V. fluvialis transaminase
atgaacaaaccgcagagctgggaaacgcgtgcggaaacctatagcctgtatgcctttacccacatgccgagcctacatcagcgtggcacctcagtggtaacccatggcgaaggcccgtatatcgtggatgtgcatggccgtcgttatctggatgcgaacagcggcctgttcaacatggtggcgggctttgatcataaaggcctgattgatgcggcgaaagcgcagtatgaacgttttccgggctatcatgcgttttacggccgtatgagcgatcagaccgtgatgctgtctgaaaaactggtggaagtgagcccgtttgatagcggccgtgtgttttataccaacagcggcagcgaagcgaacgataccatggtgaaaatgctgtggtttctgcatcgtgcggaaggcaaaccgcagaaacgtaaaattctgaccctgaagaacgcgtatcatggctccaccgcggtgagcgcgagcatgaccggccttccgtataacagcagctttggcctgccgctgccgggctttctgcatctgacctgcccgcattattggcgttatggcgaagaaggcgaaaccgaagaacagtttgtcgcgcgtctggcccgtgaactggaagaaaccattcagaaggaaggcgcggataccattgcgggcttttttgcggaaccggtgatgggtgcgggcggtgttattaccccgccaaaaggctattttcaggcgattctgaccatcctgcgcaaatatgatattccggtgatcagcgatgaagtgatttgcggctttggtcgtaccggcaacacctggggctgcgtgacctatgattttaccccggatgcgattattagcagtaaaaacctaaccgcgggtttttttccagtaggagcggtgattttggggccggaactgagcaaacgtctggaaaccgcgattgaagcgattggggaatttgatcatggttttaccacaggcggccatccggtgggttgtgcgattgcgctgaaagcgattgatgtggtgatgaacgaaggcctgctggaaaacgtgcgtcgtctggccccgcgttttgaagaacgtctgaaacatattgcggaacgtccgaacattggcgaatatcgtggtattggctttatgtgggcgctggaagtggtgaaagataaagcgagcaaagccccgtttgatggtaacctggttgtgagcgaacgtattgcgaacacctgcaccgatctgggactgatttgccgaccgttgggcagcagcgtggttctggcgccgccgtacattctgaccgaagcgcagatggatgaaatgttcgataaactggaaaaagcgctggataaagtgtttgcggaagtggcgtaa

SEQ ID NO: 104 - protein, 453 aa, Artificial Sequence
  Engineered variant of V. fluvialis transaminase
MNKPQSWETRAETYSLYAFTHMPSLHQRGTSVVTHGEGPYIVDVHGRRYLDANSGLFNMVAGFDHKGLIDAAKAQYERFPGYHAFYGRMSDQTVMLSEKLVEVSPFDSGRVFYTNSGSEANDTMVKMLWFLHRAEGKPQKRKILTLKNAYHGSTAVSASMTGLPYNSSFGLPLPGFLHLTCPHYWRYGEEGETEEQFVARLARELEETIQKEGADTIAGFFAEPVMGAGGVITPPKGYFQAILTILRKYDIPVISDEVICGFGRTGNTWGCVTYDFTPDAIISSKNLTAGFFPVGAVILGPELSKRLETAIEAIGEFDHGFTTGGHPVGCAIALKAIDVVMNEGLLENVRRLAPRFEERLKHIAERPNIGEYRGIGFMWALEVVKDKASKAPFDGNLVVSERIANTCTDLGLICRPLGSSVVLAPPYILTEAQMDEMFDKLEKALDKVFAEVA

SEQ ID NO: 105 - DNA, 1362 bp, Artificial Sequence
  Engineered variant of V. fluvialis transaminase
atgaacaaaccgcagagctgggaaacgcgtgcggaaacctatagcctgtatgcctttacccacatgccgagcctacatcagcgtggcacctcagtggtaacccatggcgaaggcccgtatatcgtggatgtgcatggccgtcgttatctggatgcgaacagcggcctgttcaacatggtggcgggctttgatcataaaggcctgattgatgcggcgaaagcgcagtatgaacgttttccgggctatcatgcgttttacggccgtatgagcgatcagaccgtgatgctgtctgaaaaactggtggaagtgagcccgtttgatagcggccgtgtgttttataccaacagcggcagcgaagcgaacgataccatggtgaaaatgctgtggtttctgcatcgtgcggaaggcaaaccgcagaaacgtaaaattctgaccctgaagaacgcgtatcatggctccaccgcggtgagcgcgagcatgaccggccttccgtataacagcgtgtttggcctgccgctgccgggctttctgcatctgacctgcccgcattattggcgttatggcgaagaaggcgaaaccgaagaacagtttgtcgcgcgtctggcccgtgaactggaagaaaccattcagaaggaaggcgcggataccattgcgggcttttttgcggaaccggtgatgggtgcgggcggtgttattaccccgccaaaaggctattttcaggcgattctgaccatcctgcgcaaatatgatattccggtgatcagcgatgaagtgatttgcggctttggtcgtaccggcaacacctggggctgcgtgacctatgattttaccccggatgcgattattagcagtaaaaacctaaccgcgggtttttttccagtaggagcggtgattttggggccggaactgagcaaacgtctggaaaccgcgattgaagcgaatgaggaatttgatcatggttttaccacaggcggccatccggtgggttgtgcgattgcgctgaaagcgattgatgtggtgatgaacgaaggcctggccgaaaacgtgcgtcgtctggccccgcgttttgaagaacgtctgaaacatattgcggaacgtccgaacattggcgaatatcgtggtattggctttatgtgggcgctggaagtggtgaaagataaagcgagcaaagccccgtttgatggtaacctgtgggtgagcgaacgtattgcgaacacctgcaccgatctgggactgatttgccgaccgttgggccagagcgtggttctggcaccgccgtacattctgaccgaagcgcagatggatgaaatgttcgataaactggaaaaagcgctggataaagtgtttgcggaagtggcgtaa

SEQ ID NO: 106 - protein, 453 aa, Artificial Sequence
  Engineered variant of V. fluvialis transaminase
MNKPQSWETRAETYSLYAFTHMPSLHQRGTSVVTHGEGPYIVDVHGRRYLDANSGLFNMVAGFDHKGLIDAAKAQYERFPGYHAFYGRMSDQTVMLSEKLVEVSPFDSGRVFYTNSGSEANDTMVKMLWFLHRAEGKPQKRKILTLKNAYHGSTAVSASMTGLPYNSVFGLPLPGFLHLTCPHYWRYGEEGETEEQFVARLARELEETIQKEGADTIAGFFAEPVMGAGGVITPPKGYFQAILTILRKYDIPVISDEVICGFGRTGNTWGCVTYDFTPDAIISSKNLTAGFFPVGAVILGPELSKRLETAIEANEEFDHGFTTGGHPVGCAIALKAIDVVMNEGLAENVRRLAPRFEERLKHIAERPNIGEYRGIGFMWALEVVKDKASKAPFDGNLWVSERIANTCTDLGLICRPLGQSVVLAPPYILTEAQMDEMFDKLEKALDKVFAEVA

SEQ ID NO: 107 - DNA, 1362 bp, Artificial Sequence
  Engineered variant of V. fluvialis transaminase
atgaacaaaccgcagagctgggaaacgcgtgcggaaacctatagcctgtatgcctttacccacatgccgagcctacatcagcgtggcacctcagtggtaacccatggcgaaggcccgtatatcgtggatgtgcatggccgtcgttatctggatgcgaacagcggcctgttcaacatggtggcgggctttgatcataaaggcctgattgatgcggcgaaagcgcagtatgaacgttttccgggctatcatgcgttttacggccgtatgagcgatcagaccgtgatgctgtctgaaaaactggtggaagtgagcccgtttgatagcggccgtgtgttttataccaacagcggcagcgaagcgaacgataccatggtgaaaatgctgtggtttctgcatcgtgcggaaggcaaaccgcagaaacgtaaaattctgaccctgaagaacgcgtatcatggctccaccgcggtgagcgcgagcatgaccggccttccgtataacagcgtgtttggcctgccgctgccgggctttctgcatctgacctgcccgcattattggcgttatggcgaagaaggcgaaaccgaagaacagtttgtcgcgcgtctggcccgtgaactggaagaaaccattcagaaggaaggcgcggataccattgcgggcttttttgcggaaccggtgatgggtgcgggcggtgttattaccccgccaaaaggctattttcaggcgattctgaccatcctgcgcaaatatgatattccggtgatcagcgatgaagtgatttgcggctttggtcgtaccggcaacacctggggctgcgtgacctatgattttaccccggatgcgattattagcagtaaaaacctaaccgcgggtttttttccagtaggagcggtgattttggggccggaactgagcaaacgtctggaaaccgcgattgaagcgatcgaagaatttgatcatggttttaccacaggcggccatccggtgggttgtgcgattgcgctgaaagcgattgatgtggtgatgaacgaaggcctggccgaaaacgtgcgtcgtctggccccgcgttttgaagaacgtctgaaacatattgcggaacgtccgaacattggcgaatatcgtggtattggctttatgtgggcgctggaagtggtgaaagataaagcgagcaaagccccgtttgatggcaacctgagcgtgagcgaacgtattgcgaacacctgcaccgatctgggactgatttgccgaccgttgggccagagcgtggttctggcaccgccgtacattctgaccgaagcgcagatggatgaaatgttcgataaactggaaaaagcgctggataaagtgtttgcggaagtggcgtaa

SEQ ID NO: 108 - protein, 453 aa, Artificial Sequence
  Engineered variant of V. fluvialis transaminase
MNKPQSWETRAETYSLYAFTHMPSLHQRGTSVVTHGEGPYIVDVHGRRYLDANSGLFNMVAGFDHKGLIDAAKAQYERFPGYHAFYGRMSDQTVMLSEKLVEVSPFDSGRVFYTNSGSEANDTMVKMLWFLHRAEGKPQKRKILTLKNAYHGSTAVSASMTGLPYNSVFGLPLPGFLHLTCPHYWRYGEEGETEEQFVARLARELEETIQKEGADTIAGFFAEPVMGAGGVITPPKGYFQAILTILRKYDIPVISDEVICGFGRTGNTWGCVTYDFTPDAIISSKNLTAGFFPVGAVILGPELSKRLETAIEAIEEFDHGFTTGGHPVGCAIALKAIDVVMNEGLAENVRRLAPRFEERLKHIAERPNIGEYRGIGFMWALEVVKDKASKAPFDGNLSVSERIANTCTDLGLICRPLGQSVVLAPPYILTEAQMDEMFDKLEKALDKVFAEVA

SEQ ID NO: 109 - DNA, 1362 bp, Artificial Sequence
  Engineered variant of V. fluvialis transaminase
atgaacaaaccgcagagctgggaaacgcgtgcggaaacctatagcctgtatgcctttacccacatgccgagcctacatcagcgtggcacctcagtggtaacccatggcgaaggcccgtatatcgtggatgtgcatggccgtcgttatctggatgcgaacagcggcctgttcaacatggtggcgggctttgatcataaaggcctgattgatgcggcgaaagcgcagtatgaacgttttccgggctatcatgcgttttacggccgtatgagcgatcagaccgtgatgctgtctgaaaaactggtggaagtgagcccgtttgatagcggccgtgtgttttataccaacagcggcagcgaagcgaacgataccatggtgaaaatgctgtggtttctgcatcgtgcggaaggcaaaccgcagaaacgtaaaattctgaccctgaagaacgcgtatcatggctccaccgcggtgagcgcgagcatgaccggcatcccgtataacagcaagtttggcctgccgctgccgggctttctgcatctgacctgcccgcattattggcgttatggcgaagaaggcgaaaccgaagaacagtttgtcgcgcgtctggcccgtgaactggaagaaaccattcagaaggaaggcgcggataccattgcgggcttttttgcggaaccggtgatgggtgcgggcggtgttattaccccgccaaaaggctattttcaggcgattctgaccatcctgcgcaaatatgatattccggtgatcagcgatgaagtgatttgcggctttggtcgtaccggcaacacctggggctgcgtgacctatgattttaccccggatgcgattattagcagtaaaaacctaaccgcgggtttttttccagtaggagcggtgattttggggccggaactgagcaaacgtctggaaaccgcgattgaagcgattggggaatttgatcatggttttaccacaggcggccatccggtgggttgtgcgattgcgctgaaagcgattgatgtggtgatgaacgaaggcctgctggaaaacgtgcgtcgtctggccccgcgttttgaagaacgtctgaaacatattgcggaacgtccgaacattggcgaatatcgtggtattggctttatgtgggcgctggaagtggtgaaagataaagcgagcaaagccccgtttgatggtaacctgtgggtgagcgaacgtattgcgaacacctgcaccgatctgggactgatttgccgaccgttgggccagagcgtggttctggcgccgccgtacattctgaccgaagcgcagatggatgaaatgttcgataaactggaaaaagcgctggataaagtgtttgcggatgtggcgtaa

SEQ ID NO: 110 - protein, 453 aa, Artificial Sequence
  Engineered variant of V. fluvialis transaminase
MNKPQSWETRAETYSLYAFTHMPSLHQRGTSVVTHGEGPYIVDVHGRRYLDANSGLFNMVAGFDHKGLIDAAKAQYERFPGYHAFYGRMSDQTVMLSEKLVEVSPFDSGRVFYTNSGSEANDTMVKMLWFLHRAEGKPQKRKILTLKNAYHGSTAVSASMTGIPYNSKFGLPLPGFLHLTCPHYWRYGEEGETEEQFVARLARELEETIQKEGADTIAGFFAEPVMGAGGVITPPKGYFQAILTILRKYDIPVISDEVICGFGRTGNTWGCVTYDFTPDAIISSKNLTAGFFPVGAVILGPELSKRLETAIEAIGEFDHGFTTGGHPVGCAIALKAIDVVMNEGLLENVRRLAPRFEERLKHIAERPNIGEYRGIGFMWALEVVKDKASKAPFDGNLWVSERIANTCTDLGLICRPLGQSVVLAPPYILTEAQMDEMFDKLEKALDKVFADVA

SEQ ID NO: 111 - DNA, 1362 bp, Artificial Sequence
  Engineered variant of V. fluvialis transaminase
atgaacaaaccgcagagctgggaaacgcgtgcggaaaccgtgagcctgtatgcctttacccacatgccgagcctacatcagcgtggcacctcagtggtaacccatggcgaaggcccgtatatcgtggatgtgcatggccgtcgttatctggatgcgaacagcggcctgttcaacatggtggcgggctttgatcataaaggcctgattgatgcggcgaaagcgcagtatgaacgttttccgggctatcatgcgttttacggccgtatgagcgatcagaccgtgatgctgtctgaaaaactggtggaagtgagcccgtttgatagcggccgtgtgttttataccaacagcggcagcgaagcgaacgataccatggtgaaaatgctgtggtttctgcatcgtgcggaaggcaaaccgcagaaacgtaaaattctgaccctgaagaacgcgtatcatggctccaccgcggtgagcgcgagcatgaccggccttccgtataacagcgtgtttggcctgccgctgccgggctttctgcatctgacctgcccgcattattggcgttatggcgaagaaggcgaaaccgaagaacagtttgtcgcgcgtctggcccgtgaactggaagaaaccattcagaaggaaggcgcggataccattgcgggcttttttgcggaaccggtgatgggtgcgggcggtgttattaccccgccaaaaggctattttcaggcgattctgaccatcctgcgcaaatatgatattccggtgatcagcgatgaagtgatttgcggctttggtcgtaccggcaacacctggggctgcgtgacctatgattttaccccggatgcgattattagcagtaaaaacctaaccgcgggtttttttccagtaggagcggtgattttggggccggaactgagcaaacgtctggaaaccgcgattgaagcgaatgaggaatttgatcatggttttaccacaggcggccatccggtgggttgtgcgattgcgctgaaagcgattgatgtggtgatgaacgaaggcctgctggaaaacgtgcgtcgtctggccccgcgttttgaagaacgtctgaaacatattgcggaacgtccgaacattggcgaatatcgtggtattggctttatgtgggcgctggaagtggtgaaagataaagcgagcaaagccccgtttgatggtaacctggttgtgagcgaacgtattgcgaacacctgcaccgatctgggactgatttgccgaccgttgggccagagcgtggttctggcgccgccgtacattctgaccgaagcgcagatggatgaaatgttcgataaactggaaaaagcgctggataaagtgtttgcggaagtggcgtaa

SEQ ID NO: 112 - protein, 453 aa, Artificial Sequence
  Engineered variant of V. fluvialis transaminase
MNKPQSWETRAETVSLYAFTHMPSLHQRGTSVVTHGEGPYIVDVHGRRYLDANSGLFNMVAGFDHKGLIDAAKAQYERFPGYHAFYGRMSDQTVMLSEKLVEVSPFDSGRVFYTNSGSEANDTMVKMLWFLHRAEGKPQKRKILTLKNAYHGSTAVSASMTGLPYNSVFGLPLPGFLHLTCPHYWRYGEEGETEEQFVARLARELEETIQKEGADTIAGFFAEPVMGAGGVITPPKGYFQAILTILRKYDIPVISDEVICGFGRTGNTWGCVTYDFTPDAIISSKNLTAGFFPVGAVILGPELSKRLETAIEANEEFDHGFTTGGHPVGCAIALKAIDVVMNEGLLENVRRLAPRFEERLKHIAERPNIGEYRGIGFMWALEVVKDKASKAPFDGNLVVSERIANTCTDLGLICRPLGQSVVLAPPYILTEAQMDEMFDKLEKALDKVFAEVA

SEQ ID NO: 113 - DNA, 1362 bp, Artificial Sequence
  Engineered variant of V. fluvialis transaminase
atgaacaaaccgcagagctgggaaacgcgtgcggaaacctatagcctgtatgcctttacccacatgccgagcctacatcagcgtggcacctcagtggtaacccatggcgaaggcccgtatatcgtggatgtgcatggccgtcgttatctggatgcgaacagcggcctgttcaacatggtggcgggctttgatcataaaggcctgattgatgcggcgaaagcgcagtatgaacgttttccgggctatcatgcgttttacggccgtatgagcgatcagaccgtgatgctgtctgaaaaactggtggaagtgagcccgtttgatagcggccgtgtgttttataccaacagcggcagcgaagcgaacgataccatggtgaaaatgctgtggtttctgcatcgtgcggaaggcaaaccgcagaaacgtaaaattctgaccctgaagaacgcgtatcatggctccaccgcggtgagcgcgagcatgaccggcatcccgtataacagcgtgtttggcctgccgctgccgggctttctgcatctgacctgcccgcattattggcgttatggcgaagaaggcgaaaccgaagaacagtttgtcgcgcgtctggcccgtgaactggaagaaaccattcagaaggaaggcgcggataccattgcgggcttttttgcggaaccggtgatgggtgcgggcggtgttattaccccgccaaaaggctattttcaggcgattctgaccatcctgcgcaaatatgatattccggtgatcagcgatgaagtgatttgcggctttggtcgtaccggcaacacctggggctgcgtgacctatgattttaccccggatgcgattattagcagtaaaaacctaaccgcgggtttttttccagtaggagcggtgattttggggccggaactgagcaaacgtctggaaaccgcgattgaagcgattggggaatttgatcatggttttaccacaggcggccatccggtgggttgtgcgattgcgctgaaagcgattgatgtggtgatgaacgaaggcctgctggaaaacgtgcgtcgtctggccccgcgttttgaagaacgtctgaaacatattgcggaacgtccgaacattggcgaatatcgtggtattggctttatgtgggcgctggaagtggtgaaagataaagcgagcaaagccccgtttgatggtaacctgttggtgagcgaacgtattgcgaacacctgcaccgatctgggactgatttgccgaccgttgggccagagcgtggttctggcgccgccgtacattctgaccgaagcgcagatggatgaaatgttcgataaactggaaaaagcgctggataaagtgtttgcggaagtggcgtaa

SEQ ID NO: 114 - protein, 453 aa, Artificial Sequence
  Engineered variant of V. fluvialis transaminase
MNKPQSWETRAETYSLYAFTHMPSLHQRGTSVVTHGEGPYIVDVHGRRYLDANSGLFNMVAGFDHKGLIDAAKAQYERFPGYHAFYGRMSDQTVMLSEKLVEVSPFDSGRVFYTNSGSEANDTMVKMLWFLHRAEGKPQKRKILTLKNAYHGSTAVSASMTGIPYNSVFGLPLPGFLHLTCPHYWRYGEEGETEEQFVARLARELEETIQKEGADTIAGFFAEPVMGAGGVITPPKGYFQAILTILRKYDIPVISDEVICGFGRTGNTWGCVTYDFTPDAIISSKNLTAGFFPVGAVILGPELSKRLETAIEAIGEFDHGFTTGGHPVGCAIALKAIDVVMNEGLLENVRRLAPRFEERLKHIAERPNIGEYRGIGFMWALEVVKDKASKAPFDGNLLVSERIANTCTDLGLICRPLGQSVVLAPPYILTEAQMDEMFDKLEKALDKVFAEVA

SEQ ID NO: 115 - DNA, 1362 bp, Artificial Sequence
  Engineered variant of V. fluvialis transaminase
atgaacaaaccgcagagctgggaaacgcgtgcggaaacctatagcctgtatgcctttacccacatgccgagcctacatcagcgtggcacctcagtggtaacccatggcgaaggcccgtatatcgtggatgtgcatggccgtcgttatctggatgcgaacagcggcctgtggaacatggtggcgggctttgatcataaaggcctgattgatgcggcgaaagcgcagtatgaacgttttccgggctatcatgcgttttacggccgtatgagcgatcagaccgtgatgctgtctgaaaaattggtggaagtgagcccgtttgatagcggccgtgtgttttataccaacagcggcagcgaagcgaacgataccatggtgaaaatgctgtggtttctgcatcgtgcggaaggcaaaccgcagaaacgtaaaattctgaccctgaagaacgcgtatcatggctccaccgcggtgagcgcgagcatgaccggcatcccgtataacagcgtgtttggcctgccgctgccgggctttctgcatctgacctgcccgcattattggcgttatggcgaagaaggcgaaaccgaagaacagtttgtcgcgcgtctggcccgtgaactggaagaaaccattcagaaggaaggcgcggataccattgcgggcttttttgcggaaccggtgatgggtgcgggcggtgttattaccccgccaaaaggctattttcaggcgattctgaccatcctgcgcaaatatgatattccggtgatcagcgatgaagtgatttgcggctttggtcgtaccggcaacacctggggctgcgtgacctatgattttaccccggatgcgattattagcagtaaaaacctaaccgcgggtttttttccagtaggagcggtgattttggggccggaactgagcaaacgtctggaaaccgcgattgaagcgattggggaatttgatcatggttttaccacaggcggccatccggtgggttgtgcgattgcgctgaaagcgattgatgtggtgatgaacgaaggcctgctggaaaacgtgcgtcgtctggccccgcgttttgaagaacgtctgaaacatattgcggaacgtccgaacattggcgaatatcgtggtattggctttatgtgggcgctggaagtggtgaaagataaagcgagcaaagccccgtttgatggtaacctggttgtgagcgaacgtattgcgaacacctgcaccgatctgggactgatttgccgaccgttgggccagagcgtggttctggcaccgccgtacattctgaccgaagcgcagatggatgaaatgttcgataaactggaaaaagcgctggataaagtgtttgcggatgtggcgtaa

SEQ ID NO: 116 - protein, 453 aa, Artificial Sequence
  Engineered variant of V. fluvialis transaminase
MNKPQSWETRAETYSLYAFTHMPSLHQRGTSVVTHGEGPYIVDVHGRRYLDANSGLWNMVAGFDHKGLIDAAKAQYERFPGYHAFYGRMSDQTVMLSEKLVEVSPFDSGRVFYTNSGSEANDTMVKMLWFLHRAEGKPQKRKILTLKNAYHGSTAVSASMTGIPYNSVFGLPLPGFLHLTCPHYWRYGEEGETEEQFVARLARELEETIQKEGADTIAGFFAEPVMGAGGVITPPKGYFQAILTILRKYDIPVISDEVICGFGRTGNTWGCVTYDFTPDAIISSKNLTAGFFPVGAVILGPELSKRLETAIEAIGEFDHGFTTGGHPVGCAIALKAIDVVMNEGLLENVRRLAPRFEERLKHIAERPNIGEYRGIGFMWALEVVKDKASKAPFDGNLVVSERIANTCTDLGLICRPLGQSVVLAPPYILTEAQMDEMFDKLEKALDKVFADVA

SEQ ID NO: 117 - DNA, 1362 bp, Artificial Sequence
  Engineered variant of V. fluvialis transaminase
atgaacaaaccgcagagctgggaaacgcgtgcggaaacctatagcctgtatgcctttacccacatgccgagcctacatcagcgtggcacctcagtggtaacccatggcgaaggcccgtatatcgtggatgtgcatggccgtcgttatctggatgcgaacagcggcctgttcaacatggtggcaggctttgatcataaaggcctgattgatgcggcgaaagcgcagtatgaacgttttccgggctatcatgcgttttacggccgtatgagcgatcagaccgtgatgctgtctgaaaaactggtggaagtgagcccgtttgatagcggccgtgtgttttataccaacagcggcagcgaagcgaacgataccatggtgaaaatgctgtggtttctgcatcgtgcggaaggcaaaccgcagaaacgtaaaattctgaccctgaagaacgcgtatcatggctccaccgcggtgagcgcgagcatgaccggcatcccgtataacagcgtgtttggcctgccgctgccgggctttctgcatctgacctgcccgcattattggcgttatggcgaagaaggcgaaaccgaagaacagtttgtcgcgcgtctggcccgtgaactggaagaaaccattcagaaggaaggcgcggataccattgcgggcttttttgcggaaccggtgatgggtgcgggcggtgttattaccccgccaaaaggctattttcaggcgattctgaccatcctgcgcaaatatgatattccggtgatcagcgatgaagtgatttgcggctttggtcgtaccggcaacacctggggctgcgtgacctatgattttaccccggatgcgattattagcagtaaaaacctaaccgcgggtttttttccagtaggagcggtgattttggggccggaactgagcaaacgtctggaaaccgcgattgaagcgattggggaatttgatcatggttttaccacaggcggccatccggtgggttgtgcgattgcgctgaaagcgattgatgtggtgatgaacgaaggcctgctggaaaacgtgcgtcgtctggccccgcgttttgaagaacgtctgaaacatattgcggaacgtccgaacattggcgaatatcgtggtattggctttatgtgggcgctggaagtggtgaaagataaagcgagcaaagccccgtttgatggtaacctgtgggtgagcgaacgtattgcgaacacctgcaccgatctgggactgatttgccgaccgttgggccagagcgtggttctggcgccgccgtacattctgaccgaagcgcagatggatgaaatgttcgataaactggaaaaagcgctggataaagtgtttgcggatgtggcgtaa

SEQ ID NO: 118 - protein, 453 aa, Artificial Sequence
  Engineered variant of V. fluvialis transaminase
MNKPQSWETRAETYSLYAFTHMPSLHQRGTSVVTHGEGPYIVDVHGRRYLDANSGLFNMVAGFDHKGLIDAAKAQYERFPGYHAFYGRMSDQTVMLSEKLVEVSPFDSGRVFYTNSGSEANDTMVKMLWFLHRAEGKPQKRKILTLKNAYHGSTAVSASMTGIPYNSVFGLPLPGFLHLTCPHYWRYGEEGETEEQFVARLARELEETIQKEGADTIAGFFAEPVMGAGGVITPPKGYFQAILTILRKYDIPVISDEVICGFGRTGNTWGCVTYDFTPDAIISSKNLTAGFFPVGAVILGPELSKRLETAIEAIGEFDHGFTTGGHPVGCAIALKAIDVVMNEGLLENVRRLAPRFEERLKHIAERPNIGEYRGIGFMWALEVVKDKASKAPFDGNLWVSERIANTCTDLGLICRPLGQSVVLAPPYILTEAQMDEMFDKLEKALDKVFADVA

SEQ ID NO: 119 - DNA, 1362 bp, Artificial Sequence
  Engineered variant of V. fluvialis transaminase
atgaacaaaccgcagagctgggaaacgcgtgcggaaacctatagcctgtatgcctttacccacatgccgagcctacatcagcgtggcacctcagtggtaacccatggcgaaggcccgtatatcgtggatgtgcatggccgtcgttatctggatgcgaacagcggcctgttcaacatggtggcgggctttgatcataaaggcctgattgatgcggcgaaagcgcagtatgaacgttttccgggctatcatgcgttttacggccgtatgagcgatcagaccgtgatgctgtctgaaaaactggtggaagtgagcccgtttgatagcggccgtgtgttttataccaacagcggcagcgaagcgaacgataccatggtgaaaatgctgtggtttctgcatcgtgcggaaggcaaaccgcagaaacgtaaaattctgaccctgaagaacgcgtatcatggctccaccgcggtgagcgcgagcatgaccggcatcccgtataacagcgtgtttggcctgccgctgccgggctttctgcatctgacctgcccgcattattggcgttatggcgaagaaggcgaaaccgaagaacagtttgtcgcgcgtctggcccgtgaactggaagaaaccattcagaaggaaggcgcggataccattgcgggcttttttgcggaaccggtgatgggtgcgggcggtgttattaccccgccaaaaggctattttcaggcgattctgaccatcctgcgcaaatatgatattccggtgatcagcgatgaagtgatttgcggctttggtcgtaccggcaacacctggggctgcgtgacctatgattttaccccggatgcgattattagcagtaaaaacctaaccgcgggtttttttccagtaggagcggtgattttggggccggaactgagcaaacgtctggaaaccgcgattgaagcgattggggaatttgatcatggttttaccacaggcggccatccggtgggttgtgcgattgcgctgaaagcgattgatgtggtgatgaacgaaggcctgctggaaaacgtgcgtcgtctggccccgcgttttgaagaacgtctgaaacatattgcggaacgtccgaacattggcgaatatcgtggtattggctttatgtgggcgctggaagtggtgaaagataaagcgagcaaagccccgtttgatggtaacctggttgtgagcgaacgtattgcgaacacctgcaccgatctgggactgatttgccgaccgttgggccagagcgtggttctggcgccgccgtacattctgaccgaagcgcagatggatgaaatgttcgataaactggaaaaagcgctggataaagtgtttgcggaagtggcgtaa

SEQ ID NO: 120 - protein, 453 aa, Artificial Sequence
  Engineered variant of V. fluvialis transaminase
MNKPQSWETRAETYSLYAFTHMPSLHQRGTSVVTHGEGPYIVDVHGRRYLDANSGLFNMVAGFDHKGLIDAAKAQYERFPGYHAFYGRMSDQTVMLSEKLVEVSPFDSGRVFYTNSGSEANDTMVKMLWFLHRAEGKPQKRKILTLKNAYHGSTAVSASMTGIPYNSVFGLPLPGFLHLTCPHYWRYGEEGETEEQFVARLARELEETIQKEGADTIAGFFAEPVMGAGGVITPPKGYFQAILTILRKYDIPVISDEVICGFGRTGNTWGCVTYDFTPDAIISSKNLTAGFFPVGAVILGPELSKRLETAIEAIGEFDHGFTTGGHPVGCAIALKAIDVVMNEGLLENVRRLAPRFEERLKHIAERPNIGEYRGIGFMWALEVVKDKASKAPFDGNLVVSERIANTCTDLGLICRPLGQSVVLAPPYILTEAQMDEMFDKLEKALDKVFAEVA

SEQ ID NO: 121 - DNA, 1362 bp, Artificial Sequence
  Engineered variant of V. fluvialis transaminase
atgaacaaaccgcagagctgggaaacgcgtgcggaaacctatagcctgtatgcctttacccacatgccgagcctacatcagcgtggcaccatggtggtgacccatggcgaaggcccgtatatcgtggatgtgcatggccgtcgttatctggatgcgaacagcggcctgttcaacatggtggcgggctttgatcataaaggcctgattgatgcggcgaaagcgcagtatgaacgttttccgggctatcatgcgttttacggccgtatgagcgatcagaccgtgatgctgtctgaaaaactggtggaagtgagcccgtttgatagcggccgtgtgttttataccaacagcggcagcgaagcgaacgataccatggtgaaaatgctgtggtttctgcatcgtgcggaaggcaaaccgcagaaacgtaaaattctgaccctgaagaacgcgtatcatggctccaccgcggtgagcgcgagcatgaccggccttccgtataacagcgtgtttggcctgccgctgccgggctttctgcatctgacctgcccgcattattggcgttatggcgaagaaggcgaaaccgaagaacagtttgtcgcgcgtctggcccgtgaactggaagaaaccattcagaaggaaggcgcggataccattgcgggcttttttgcggaaccggtgatgggtgcgggcggtgttattaccccgccaaaaggctattttcaggcgattctgaccatcctgcgcaaatatgatattccggtgatcagcgatgaagtgatttgcggctttggtcgtaccggcaacacctggggctgcgtgacctatgattttaccccggatgcgattattagcagtaaaaacctaaccgcgggtttttttccagtaggagcggtgattttggggccggaactgagcaaacgtctggaaaccgcgattgaagcgattgaggaatttgatcatggttttaccacaggcggccatccggtgggttgtgcgattgcgctgaaagcgattgatgtggtgatgaacgaaggcctgctggaaaacgtgcgtcgtctggccccgcgttttgaagaacgtctgaaacatattgcggaacgtccgaacattggcgaatatcgtggtattggctttatgtgggcgctggaagtggtgaaagataaagcgagcaaagccccgtttgatggtaacctgttggtgagcgaacgtattgcgaacacctgcaccgatctgggactgatttgccgaccgttgggccagagcgtggttctggcgccgccgtacattctgaccgaagcgcagatggatgaaatgttcgataaactggaaaaagcgctggataaagtgtttgcggaagtggcgtaa

SEQ ID NO: 122 - protein, 453 aa, Artificial Sequence
  Engineered variant of V. fluvialis transaminase
MNKPQSWETRAETYSLYAFTHMPSLHQRGTMVVTHGEGPYIVDVHGRRYLDANSGLFNMVAGFDHKGLIDAAKAQYERFPGYHAFYGRMSDQTVMLSEKLVEVSPFDSGRVFYTNSGSEANDTMVKMLWFLHRAEGKPQKRKILTLKNAYHGSTAVSASMTGLPYNSVFGLPLPGFLHLTCPHYWRYGEEGETEEQFVARLARELEETIQKEGADTIAGFFAEPVMGAGGVITPPKGYFQAILTILRKYDIPVISDEVICGFGRTGNTWGCVTYDFTPDAIISSKNLTAGFFPVGAVILGPELSKRLETAIEAIEEFDHGFTTGGHPVGCAIALKAIDVVMNEGLLENVRRLAPRFEERLKHIAERPNIGEYRGIGFMWALEVVKDKASKAPFDGNLLVSERIANTCTDLGLICRPLGQSVVLAPPYILTEAQMDEMFDKLEKALDKVFAEVA

SEQ ID NO: 123 - DNA, 1362 bp, Artificial Sequence
  Engineered variant of V. fluvialis transaminase
atgaacaaaccgcagagctgggaaacgcgtgcggaaacctatagcctgtatgcctttacccacatgccgagcctacatcagcgtggcaccatggtggtgacccatggcgaaggcccgtatatcgtggatgtgcatggccgtcgttatctggatgcgaacagcggcctgttcaacatggtggcgggctttgatcataaaggcctgattgatgcggcgaaagcgcagtatgaacgttttccgggctatcatgcgttttacggccgtatgagcgatcagaccgtgatgctgtctgaaaaactggtggaagtgagcccgtttgatagcggccgtgtgttttataccaacagcggcagcgaagcgaacgataccatggtgaaaatgctgtggtttctgcatcgtgcggaaggcaaaccgcagaaacgtaaaattctgaccctgaagaacgcgtatcatggctccaccgcggtgagcgcgagcatgaccggccttccgtataacagcaagtttggcctgccgctgccgggctttctgcatctgacctgcccgcattattggcgttatggcgaagaaggcgaaaccgaagaacagtttgtcgcgcgtctggcccgtgaactggaagaaaccattcagaaggaaggcgcggataccattgcgggcttttttgcggaaccggtgatgggtgcgggcggtgttattaccccgccaaaaggctattttcaggcgattctgaccatcctgcgcaaatatgatattccggtgatcagcgatgaagtgatttgcggctttggtcgtaccggcaacacctggggctgcgtgacctatgattttaccccggatgcgattattagcagtaaaaacctaaccgcgggtttttttccagtaggagcggtgattttggggccggaactgagcaaacgtctggaaaccgcgattgaagcgaatggggaatttgatcatggttttaccacaggcggccatccggtgggttgtgcgattgcgctgaaagcgattgatgtggtgatgaacgaaggcctgctggaaaacgtgcgtcgtctggccccgcgttttgaagaacgtctgaaacatattgcggaacgtccgaacattggcgaatatcgtggtattggctttatgtgggcgctggaagtggtgaaagataaagcgagcaaagccccgtttgatggtaacctggttgtgagcgaacgtattgcgaacacctgcaccgatctgggactgatttgccgaccgttgggccagagcgtggttctggcgccgccgtacattctgaccgaagcgcagatggatgaaatgttcgataaactggaaaaagcgctggataaagtgtttgcggaagtggcgtaa

SEQ ID NO: 124 - protein, 453 aa, Artificial Sequence
  Engineered variant of V. fluvialis transaminase
MNKPQSWETRAETYSLYAFTHMPSLHQRGTMVVTHGEGPYIVDVHGRRYLDANSGLFNMVAGFDHKGLIDAAKAQYERFPGYHAFYGRMSDQTVMLSEKLVEVSPFDSGRVFYTNSGSEANDTMVKMLWFLHRAEGKPQKRKILTLKNAYHGSTAVSASMTGLPYNSKFGLPLPGFLHLTCPHYWRYGEEGETEEQFVARLARELEETIQKEGADTIAGFFAEPVMGAGGVITPPKGYFQAILTILRKYDIPVISDEVICGFGRTGNTWGCVTYDFTPDAIISSKNLTAGFFPVGAVILGPELSKRLETAIEANGEFDHGFTTGGHPVGCAIALKAIDVVMNEGLLENVRRLAPRFEERLKHIAERPNIGEYRGIGFMWALEVVKDKASKAPFDGNLVVSERIANTCTDLGLICRPLGQSVVLAPPYILTEAQMDEMFDKLEKALDKVFAEVA

SEQ ID NO: 125 - DNA, 1362 bp, Artificial Sequence
  Engineered variant of V. fluvialis transaminase
atgaacaaaccgcagagctgggaaacgcgtgcggaaacctatagcctgtatgcctttacccacatgccgagcctacatcagcgtggcacctcagtggtaacccatggcgaaggcccgtatatcgtggatgtgcatggccgtcgttatctggatgcgaacagcggcctgttcaacatggtggcgggctttgatcataaaggcctgattgatgcggcgaaagcgcagtatgaacgttttccgggctatcatgcgttttacggccgtatgagcgatcagaccgtgatgctgtctgaaaaactggtggaagtgagcccgtttgatagcggccgtgtgttttataccaacagcggcagcgaagcgaacgataccatggtgaaaatgctgtggtttctgcatcgtgcggaaggcaaaccgcagaaacgtaaaattctgaccctgaagaacgcgtatcatggctccaccgcggtgagcgcgagcatgaccggcatcccgtataacagcgtgtttggcctgccgctgccgggctttctgcatctgacctgcccgcattattggcgttatggcgaagaaggcgaaaccgaagaacagtttgtcgcgcgtctggcccgtgaactggaagaaaccattcagaaggaaggcgcggataccattgcgggcttttttgcggaaccggtgatgggtgcgggcggtgttattaccccgccaaaaggctattttcaggcgattctgaccatcctgcgcaaatatgatattccggtgatcagcgatgaagtgatttgcggctttggtcgtaccggcaacacctggggctgcgtgacctatgattttaccccggatgcgattattagcagtaaaaacctaaccgcgggtttttttccagtaggagcggtgattttggggccggaactgagcaaacgtctggaaaccgcgattgaagcgattggggaatttgatcatggttttaccacaggcggccatccggtgggttgtgcgattgcgctgaaagcgattgatgtggtgatgaacgaaggcctgctggaaaacgtgcgtcgtctggccccgcgttttgaagaacgtctgaaacatattgcggaacgtccgaacattggcgaatatcgtggtattggctttatgtgggcgctggaagtggtgaaagataaagcgagcaaagccccgtttgatggtaacctggttgtgagcgaacgtattgcgaacacctgcaccgatctgggactgatttgccgaccgttgggccagagcgtggttatcgcgccgccgtacattctgaccgaagcgcagatggatgaaatgttcgataaactggaaaaagcgctggataaagtgtttgcggaagtggcgtaa

SEQ ID NO: 126 - protein, 453 aa, Artificial Sequence
  Engineered variant of V. fluvialis transaminase
MNKPQSWETRAETYSLYAFTHMPSLHQRGTSVVTHGEGPYIVDVHGRRYLDANSGLFNMVAGFDHKGLIDAAKAQYERFPGYHAFYGRMSDQTVMLSEKLVEVSPFDSGRVFYTNSGSEANDTMVKMLWFLHRAEGKPQKRKILTLKNAYHGSTAVSASMTGIPYNSVFGLPLPGFLHLTCPHYWRYGEEGETEEQFVARLARELEETIQKEGADTIAGFFAEPVMGAGGVITPPKGYFQAILTILRKYDIPVISDEVICGFGRTGNTWGCVTYDFTPDAIISSKNLTAGFFPVGAVILGPELSKRLETAIEAIGEFDHGFTTGGHPVGCAIALKAIDVVMNEGLLENVRRLAPRFEERLKHIAERPNIGEYRGIGFMWALEVVKDKASKAPFDGNLVVSERIANTCTDLGLICRPLGQSVVIAPPYILTEAQMDEMFDKLEKALDKVFAEVA

SEQ ID NO: 127 - DNA, 1362 bp, Artificial Sequence
  Engineered variant of V. fluvialis transaminase
atgaacaaaccgcagagctgggaaacgcgtgcggaaacctatagcctgtatgcctttacccacatgccgagcctacatcagcgtggcacctcagtggtaacccatggcgaaggcccgtatatcgtggatgtgcatggccgtcgttatctggatgcgaacagcggcctgttcaacatggtggcgggctttgatcataaaggcctgattgatgcggcgaaagcgcagtatgaacgttttccgggctatcatgcgttttacggccgtatgagcgatcagaccgtgatgctgtctgaaaaactggtggaagtgagcccgtttgatagcggccgtgtgttttataccaacagcggcagcgaagcgaacgataccatggtgaaaatgctgtggtttctgcatcgtgcggaaggcaaaccgcagaaacgtaaaattctgaccctgaagaacgcgtatcatggctccaccgcggtgagcgcgagcatgaccggccttccgtataacagcgtgtttggcctgccgctgccgggctttctgcatctgacctgcccgcattattggcgttatggcgaagaaggcgaaaccgaagaacagtttgtcgcgcgtctggcccgtgaactggaagaaaccattcagaaggaaggcgcggataccattgcgggcttttttgcggaaccggtgatgggtgcgggcggtgttattaccccgccaaaaggctattttcaggcgattctgaccatcctgcgcaaatatgatattccggtgatcagcgatgaagtgatttgcggctttggtcgtaccggcaacacctggggctgcgtgacctatgattttaccccggatgcgattattagcagtaaaaacctaaccgcgggtttttttccagtaggagcggtgattttggggccggaactgagcaaacgtctggaaaccgcgattgaagcgaatggggaatttgatcatggttttaccacaggcggccatccggtgggttgtgcgattgcgctgaaagcgattgatgtggtgatgaacgaaggcctgctggaaaacgtgcgtcgtctggccccgcgttttgaagaacgtctgaaacatattgcggaacgtccgaacattggcgaatatcgtggtattggctttatgtgggcgctggaagtggtgaaagataaagcgagcaaagccccgtttgatggtaacctggttgtgagcgaacgtattgcgaacacctgcaccgatctgggactgatttgccgaccgttgggcagcagcgtggttctggcgccgccgtacattctgaccgaagcgcagatggatgaaatgttcgataaactggaaaaagcgctggataaagtgtttgcggaagtggcgtaa

SEQ ID NO: 128 - protein, 453 aa, Artificial Sequence
  Engineered variant of V. fluvialis transaminase
MNKPQSWETRAETYSLYAFTHMPSLHQRGTSVVTHGEGPYIVDVHGRRYLDANSGLFNMVAGFDHKGLIDAAKAQYERFPGYHAFYGRMSDQTVMLSEKLVEVSPFDSGRVFYTNSGSEANDTMVKMLWFLHRAEGKPQKRKILTLKNAYHGSTAVSASMTGLPYNSVFGLPLPGFLHLTCPHYWRYGEEGETEEQFVARLARELEETIQKEGADTIAGFFAEPVMGAGGVITPPKGYFQAILTILRKYDIPVISDEVICGFGRTGNTWGCVTYDFTPDAIISSKNLTAGFFPVGAVILGPELSKRLETAIEANGEFDHGFTTGGHPVGCAIALKAIDVVMNEGLLENVRRLAPRFEERLKHIAERPNIGEYRGIGFMWALEVVKDKASKAPFDGNLVVSERIANTCTDLGLICRPLGSSVVLAPPYILTEAQMDEMFDKLEKALDKVFAEVA

SEQ ID NO: 129 - DNA, 1362 bp, Artificial Sequence
  Engineered variant of V. fluvialis transaminase
atgaacaaaccgcagagctgggaaacgcgtgcggaaaccgtgagcctgtatgcctttacccacatgccgagcctacgtcagcgtggcaccatggtggtgacccatggcgaaggcccgtatatcgtggatgtgcatggccgtcgttatctggatgcgaacagcggcctgtggaacatggtggcgggctttgatcataaaggcctgattgatgcggcgaaagcgcagtatgaacgttttccgggctatcatgcgttttacggccgtatgagcgatcagaccgtgatgctgtctgaaaaactggtggaagtgagcccgtttgatagcggccgtgtgttttataccaacagcggcagcgaagcgaacgataccatggtgaaaatgctgtggtttctgcatcgtgcggaaggcaaaccgcagaaacgtaaaattctgaccctgaagaacgcgtatcatggctccaccgcggtgagcgcgagcatgaccggcatcccgtataacagcgtgtttggcctgccgctgccgggctttctgcatctgacctgcccgcattattggcgttatggcgaagaaggcgaaaccgaagaacagtttgtcgcgcgtctggcccgtgaactggaagaaaccattcagaaggaaggcgcggataccattgcgggcttttttgcggaaccggtgatgggtgcgggcggtgttattaccccgccaaaaggctattttcaggcgattctgaccatcctgcgcaaatatgatattccggtgatcagcgatgaagtgatttgcggctttggtcgtaccggcaacacctggggctgcgtgacctatgattttaccccggatgcgattattagcgccaaaaacctaaccgcgggtttttttccagtaggagcggtgattttggggccggaactgagcaaacgtctggaaaccgcgattgaagcgatcgaagaatttgatcatggttttaccacaggcggccatccggtgggttgtgcgattgcgctgaaagcgattgatgtggtgatgaacgaaggcctggccgaaaacgtgcgtcgtctggccccgcgttttgaagaacgtctgaaacatattgcggaacgtccgaacattggcgaatatcgtggtattggctttatgtgggcgctggaagtggtgaaagataaagcgagcaaagccccgtttgatggcaacctgagcgtgggtgaacgtattgcgaacacctgcaccgatctgggactgatttgtcgaccgatgggccagaacgtggttctggcaccgccgtacattctgaccgaagcgcagatggatgaaatgttcgataaactggaaaaagcgctggataaagtgtttgcggaagtggcgtaa

SEQ ID NO: 130 - protein, 453 aa, Artificial Sequence
  Engineered variant of V. fluvialis transaminase
MNKPQSWETRAETVSLYAFTHMPSLRQRGTMVVTHGEGPYIVDVHGRRYLDANSGLWNMVAGFDHKGLIDAAKAQYERFPGYHAFYGRMSDQTVMLSEKLVEVSPFDSGRVFYTNSGSEANDTMVKMLWFLHRAEGKPQKRKILTLKNAYHGSTAVSASMTGIPYNSVFGLPLPGFLHLTCPHYWRYGEEGETEEQFVARLARELEETIQKEGADTIAGFFAEPVMGAGGVITPPKGYFQAILTILRKYDIPVISDEVICGFGRTGNTWGCVTYDFTPDAIISAKNLTAGFFPVGAVILGPELSKRLETAIEAIEEFDHGFTTGGHPVGCAIALKAIDVVMNEGLAENVRRLAPRFEERLKHIAERPNIGEYRGIGFMWALEVVKDKASKAPFDGNLSVGERIANTCTDLGLICRPMGQNVVLAPPYILTEAQMDEMFDKLEKALDKVFAEVA

SEQ ID NO: 131 - DNA, 1362 bp, Artificial Sequence
  Engineered variant of V. fluvialis transaminase
atgaacaaaccgcagagctgggaaacgcgtgcggaaaccgtgagcctgtatgcctttacccacatgccgagcctacatcagcgtggcaccatggtggtaacccatggcgaaggcccgtatatcgtggatgtgcatggccgtcgttatctggatgcgaacagcggcctgtggaacatggtggcgggctttgatcataaaggcctgattgatgcggcgaaagcgcagtatgaacgttttccgggctatcatgcgttttacggccgtatgagcgatcagaccgtgatgctgtctgaaaaactggtggaagtgagcccgtttgatagcggccgtgtgttttataccaacagcggcagcgaagcgaacgataccatggtgaaaatgctgtggtttctgcatcgtgcggaaggcaaaccgcagaaacgtaaaattctgaccctgaagaacgcgtatcatggctccaccgcggtgagcgcgagcatgaccggccttccgtataacagcgtgtttggcctgccggctccgggctttctgcatctgacctgcccgcattattggcgttatggcgaagaaggcgaaaccgaagaacagtttgtcgcgcgtctggcccgtgaactggaagaaaccattcagaaggaaggcgcggataccattgcgggcttttttgcggaaccggtgatgggtgcgggcggtgttattaccccgccaaaaggctattttcaggcgattctgaccatcctgcgcaaatatgatattccggtgatcagcgatgaagtgatttgcggctttggtcgtaccggcaacacctggggctgcgtgacctatgattttaccccggatgcgattattagcagtaaaaacctaaccgcgggtttttttccagtaggagcggtgattttggggccggaactgagcaaacgtctggaaaccgcgattgaagcgatcgaagaatttgatcatggttttaccacaggcggccatccggtgggttgtgcgattgcgctgaaagcgattgatgtggtgatgaacgaaggcctggccgaaaacgtgcgtcgtctggccccgcgttttgaagaacgtctgaaacatattgcggaacgtccgaacattggcgaatatcgtggtattggctttatgtgggcgctggaagtggtgaaagataaagcgagcaaagccccgtttgatggcaacctgagcgtgggtgaacgtattgcgaacacctgcaccgatctgggactgatttgtcgaccgctgggccagaacgtggttctggcaccgccgtacattctgaccgaagcgcagatggatgaaatgttcgataaactggaaaaagcgctggataaagtgtttgcggaagtggcgtaa

SEQ ID NO: 132 - protein, 453 aa, Artificial Sequence
  Engineered variant of V. fluvialis transaminase
MNKPQSWETRAETVSLYAFTHMPSLHQRGTMVVTHGEGPYIVDVHGRRYLDANSGLWNMVAGFDHKGLIDAAKAQYERFPGYHAFYGRMSDQTVMLSEKLVEVSPFDSGRVFYTNSGSEANDTMVKMLWFLHRAEGKPQKRKILTLKNAYHGSTAVSASMTGLPYNSVFGLPAPGFLHLTCPHYWRYGEEGETEEQFVARLARELEETIQKEGADTIAGFFAEPVMGAGGVITPPKGYFQAILTILRKYDIPVISDEVICGFGRTGNTWGCVTYDFTPDAIISSKNLTAGFFPVGAVILGPELSKRLETAIEAIEEFDHGFTTGGHPVGCAIALKAIDVVMNEGLAENVRRLAPRFEERLKHIAERPNIGEYRGIGFMWALEVVKDKASKAPFDGNLSVGERIANTCTDLGLICRPLGQNVVLAPPYILTEAQMDEMFDKLEKALDKVFAEVA

SEQ ID NO: 133 - DNA, 1362 bp, Artificial Sequence
  Engineered variant of V. fluvialis transaminase
atgaacaaaccgcagagctgggaaacgcgtgcggaaaccgtgagcctgtatgcctttacccacatgccgagcctacatcagcgtggcaccatggtggtaacccatggcgaaggcccgtatatcgtggatgtgcatggccgtcgttatctggatgcgaacagcggcctgtggaacatggtggcgggctttgatcataaaggcctgattgatgcggcgaaagcgcagtatgaacgttttccgggctatcatgcgttttacggccgcatgagcgatcagaccgtgatgctgtctgaaaaactggtggaagtgagcccgtttgatagcggccgtgtgtttctgaccaacagcggcagcgaagcgaacgataccatggtgaaaatgctgtggtttctgcatcgtgcggaaggcaaaccgcagaaacgtaaaattctgaccctgaagaacgcgtatcatggctccaccgcggtgagcgcgagcatgaccggccttccgtataacagcgtgtttggcctgccgctgccgggctttctgcatctgacctgcccgcattattggcgttatggcgaagaaggcgaaaccgaagaacagtttgtcgcgcgtctggcccgtgaactggaagaaaccattcagaaggaaggcgcggataccattgcgggcttttttgcggaaccggtgatgggtgcgggcggtgttattaccccgccaaaaggctattttcaggcgattctgaccatcctgcgcaaatatgatattccggtgatcagcgatgaagtgatttgcggctttggtcgtaccggcaacacctggggctgcgtgacctatgattttaccccggatgcgattattagcgccaaaaacctaaccgcgggtttttttccagtaggagcggtgattttggggccggaactgagcaaacgtctggaaaccgcgattgaagcgatcgaagaatttgatcatggttttaccacaggcggccatccggtgggttgtgcgattgcgctgaaagcgattgatgtggtgatgaacgaaggcctggccgaaaacgtgcgtcgtctggccccgcgttttgaagaacgtctgaaacatattgcggaacgtccgaacattggcgaatatcgtggtattggctttatgtgggcgctggaagtggtgaaagataaagcgagcaaagccccgtttgatggcaacctgagcgtgagcgaacgtattgcgaacacctgcaccgatctgggactgatttgccgaccgttgggccagagcgtggttctggtgccgccgtacattctgaccgaagcgcagatggatgaaatgttcgataaactggaaaaagcgctggataaagtgtttgcggaagtggcgtaa

SEQ ID NO: 134 - protein, 453 aa, Artificial Sequence
  Engineered variant of V. fluvialis transaminase
MNKPQSWETRAETVSLYAFTHMPSLHQRGTMVVTHGEGPYIVDVHGRRYLDANSGLWNMVAGFDHKGLIDAAKAQYERFPGYHAFYGRMSDQTVMLSEKLVEVSPFDSGRVFLTNSGSEANDTMVKMLWFLHRAEGKPQKRKILTLKNAYHGSTAVSASMTGLPYNSVFGLPLPGFLHLTCPHYWRYGEEGETEEQFVARLARELEETIQKEGADTIAGFFAEPVMGAGGVITPPKGYFQAILTILRKYDIPVISDEVICGFGRTGNTWGCVTYDFTPDAIISAKNLTAGFFPVGAVILGPELSKRLETAIEAIEEFDHGFTTGGHPVGCAIALKAIDVVMNEGLAENVRRLAPRFEERLKHIAERPNIGEYRGIGFMWALEVVKDKASKAPFDGNLSVSERIANTCTDLGLICRPLGQSVVLVPPYILTEAQMDEMFDKLEKALDKVFAEVA

SEQ ID NO: 135 - DNA, 1362 bp, Artificial Sequence
  Engineered variant of V. fluvialis transaminase
atgaacaaaccgcagagctgggaaacgcgtgcggaaaccgtgagcctgtatgcctttacccacatgccgagcctacatcagcgtggcaccatggtggtaacccatggcgaaggcccgtatatcgtggatgtgcatggccgtcgttatctggatgcgaacagcggcctgtggaacatggtggcgggctttgatcataaaggcctgattgatgcggcgaaagcgcagtatgaacgttttccgggctatcatgcgttttacggcctgatgagcgatcagaccgtgatgctgtctgaaaaactggtggaagtgagcccgtttgatagcggccgtgtgttttataccaacagcggcagcgaagcgaacgataccatggtgaaaatgctgtggtttctgcatcgtgcggaaggcaaaccgcagaaacgtaaaattctgaccctgaagaacgcgtatcatggctccaccgcggtgagcgcgagcatgaccggccttccgtataacagcgtgtttggcctgccgctgccgggctttctgcatctgacctgcccgcattattggcgttatggcgaagaaggcgaaaccgaagaacagtttgtcgcgcgtctggcccgtgaactggaagaaaccattcagaaggaaggcgcggataccattgcgggcttttttgcggaaccggtgatgggtgcgggcggtgttattaccccgccaaaaggctattttcaggcgattctgaccatcctgcgcaaatatgatattccggtgatcagcgatgaagtgatttgcggctttggtcgtaccggcaacacctggggctgcgtgacctatgattttaccccggatgcgattattagcagtaaaaacctaaccgcgggtttttttccagtaggagcggtgattttggggccggaactgagcaaacgtctggaaaccgcgattgaagcgatcgaagaatttgatcatggttttaccacacacggccatccggtgggttgtgcgattgcgctgaaagcgattgatgtggtgatgaacgaaggcctggccgaaaacgtgcgtcgtctggccccgcgttttgaagaacgtctgaaacatattgcggaacgtccgaacattggcgaatatcgtggtattggctttatgtgggcgctggaagtggtgaaagataaagcgagcaaagccccgtttgatggcaacctgagcgtgggtgaacgtattgcgaacacctgcaccgatctgggactgatttgtcgaccgatgggccagagcgtggttctggcaccgccgtacattctgaccgaagcgcagatggatgaaatgttcgataaactggaaaaagcgctggataaagtgtttgcggaagtggcgtaa

SEQ ID NO: 136 - protein, 453 aa, Artificial Sequence
  Engineered variant of V. fluvialis transaminase
MNKPQSWETRAETVSLYAFTHMPSLHQRGTMVVTHGEGPYIVDVHGRRYLDANSGLWNMVAGFDHKGLIDAAKAQYERFPGYHAFYGLMSDQTVMLSEKLVEVSPFDSGRVFYTNSGSEANDTMVKMLWFLHRAEGKPQKRKILTLKNAYHGSTAVSASMTGLPYNSVFGLPLPGFLHLTCPHYWRYGEEGETEEQFVARLARELEETIQKEGADTIAGFFAEPVMGAGGVITPPKGYFQAILTILRKYDIPVISDEVICGFGRTGNTWGCVTYDFTPDAIISSKNLTAGFFPVGAVILGPELSKRLETAIEAIEEFDHGFTTHGHPVGCAIALKAIDVVMNEGLAENVRRLAPRFEERLKHIAERPNIGEYRGIGFMWALEVVKDKASKAPFDGNLSVGERIANTCTDLGLICRPMGQSVVLAPPYILTEAQMDEMFDKLEKALDKVFAEVA

SEQ ID NO: 137 - DNA, 1362 bp, Artificial Sequence
  Engineered variant of V. fluvialis transaminase
atgaacaaaccgcagagctgggaaacgcgtgcggaaaccgtgagcctgtatgcctttacccacatgccgagcctacgtcagcgtggcaccatggtggtgacccatggcgaaggcccgtatatcgtggatgtgcatggccgtcgttatctggatgcgaacagcggcctgttcaacatggtggcgggctttgatcataaaggcctgattgatgcggcgaaagcgcagtatgaacgttttccgggctatcatgcgttttacggccgtatgagcgatcagaccgtgatgctgtctgaaaaactggtggaagtgagcccgtttgatagcggccgtgtgtttctgaccaacagcggcagcgaagcgaacgataccatggtgaaaatgctgtggtttctgcatcgtgcggaaggcaaaccgcagaaacgtaaaattctgaccctgaagaacgcgtatcatggctccaccgcggtgagcgcgagcatgaccggccttccgtataacagcgtgtttggcctgccgctgccgggctttctgcatctgacctgcccgcattattggcgttatggcgaagaaggcgaaaccgaagaacagtttgtcgcacgtctggcccgtgaactggaagaaaccattcagaaggaaggcgcggataccattgcgggcttttttgcggaaccggtgatgggtgcgggcggtgttattaccccgccaaaaggctattttcaggcgattctgaccatcctgcgcaaatatgatattccggtgatcagcgatgaagtgatttgcggctttggtcgtaccggcaacacctggggctgcgtgacctatgattttaccccggatgcgattattagcgccaaaaacctaaccgcgggtttttttccagtaggagcggtgattttggggccggaactgagcaaacgtctggaaaccgcgattgaagcgatcgaagaatttgatcatggttttaccacaggcggccatccggtgggttgtgcgattgcgctgaaagcgattgatgtggtgatgaacgaaggcctggccgaaaacgtgcgtcgtctggccccgcgttttgaagaacgtctgaaacatattgcggaacgtccgaacattggcgaatatcgtggtattggctttatgtgggcgctggaagtggtgaaagataaagcgagcaaagccccgtttgatggcaacctgagcgtgagcgaacgtattgcgaacacctgcaccgatctgggactgatttgccgaccgttgggccagagcgtggttctggcaccgccgtacattctgaccgaagcgcagatggatgaaatgttcgataaactggaaaaagcgctggataaagtgtttgcggaagtggcgtaa

SEQ ID NO: 138 - protein, 453 aa, Artificial Sequence
  Engineered variant of V. fluvialis transaminase
MNKPQSWETRAETVSLYAFTHMPSLRQRGTMVVTHGEGPYIVDVHGRRYLDANSGLFNMVAGFDHKGLIDAAKAQYERFPGYHAFYGRMSDQTVMLSEKLVEVSPFDSGRVFLTNSGSEANDTMVKMLWFLHRAEGKPQKRKILTLKNAYHGSTAVSASMTGLPYNSVFGLPLPGFLHLTCPHYWRYGEEGETEEQFVARLARELEETIQKEGADTIAGFFAEPVMGAGGVITPPKGYFQAILTILRKYDIPVISDEVICGFGRTGNTWGCVTYDFTPDAIISAKNLTAGFFPVGAVILGPELSKRLETAIEAIEEFDHGFTTGGHPVGCAIALKAIDVVMNEGLAENVRRLAPRFEERLKHIAERPNIGEYRGIGFMWALEVVKDKASKAPFDGNLSVSERIANTCTDLGLICRPLGQSVVLAPPYILTEAQMDEMFDKLEKALDKVFAEVA

SEQ ID NO: 139 - DNA, 1362 bp, Artificial Sequence
  Engineered variant of V. fluvialis transaminase
atgaacaaaccgcagagctgggaaacgcgtgcggaaaccgtgagcctgtatgcctttacccacatgccgagcctacgtcagcgtggcaccatggtggtgacccatggcgaaggcccgtatatcgtggatgtgcatggccgtcgttatctggatgcgaacagcggcctgtggaacatggtggcgggctttgatcataaaggcctgattgatgcggcgaaagcgcagtatgaacgttttccgggctatcatgcgttttacggccgtatgagcgatcagaccgtgatgctgtctgaaaaactggtggaagtgagcccgtttgatagcggccgtgtgttttataccaacagcggcagcgaagcgaacgataccatggtgaaaatgctgtggtttctgcatcgtgcggaaggcaaaccgcagaaacgtaaaattctgaccctgaagaacgcgtatcatggctccaccgcggtgagcgcgagcatgaccggccttccgtataacagcgtgtttggcctgccgctgccgggctttctgcatctgacctgcccgcattattggcgttatggcgaagaaggcgaaaccgaagaacagtttgtcgcgcgtctggcccgtgaactggaagaaaccattcagaaggaaggcgcggataccattgcgggcttttttgcggaaccggtgatgggtgcgggcggtgttattaccccgccaaaaggctattttcaggcgattctgaccatcctgcgcaaatatgatattccggtgatcagcgatgaagtgatttgcggctttggtcgtaccggcaacacctggggctgcgtgacctatgattttaccccggatgcgattattagcgccaaaaacctaaccgcgggtttttttccagtaggagcggtgattttggggccggaactgagcaaacgtctggaaaccgcgattgaagcgatcgaagaatttgatcatggttttaccacaggcggccatccggtgggttgtgcgattgcgctgaaagcgattgatgtggtgatgaacgaaggcctggccgaaaacgtgcgtcgtctggccccgcgttttgaagaacgtctgaaacatattgcggaacgtccgaacattggcgaatatcgtggtattggctttatgtgggcgctggaagccgtgaaagataaagcgagcaaagccccgtttgatggcaacctgagcgtgggtgaacgtattgcgaacacctgcaccgatctgggactgatttgccgaccgttgggccagagcgtggttctggcaccgccgtacattctgaccgaagcgcagatggatgaaatgttcgataaactggaaaaagcgctggataaagtgtttgcggaagtggcgtaa

SEQ ID NO: 140 - protein, 453 aa, Artificial Sequence
  Engineered variant of V. fluvialis transaminase
MNKPQSWETRAETVSLYAFTHMPSLRQRGTMVVTHGEGPYIVDVHGRRYLDANSGLWNMVAGFDHKGLIDAAKAQYERFPGYHAFYGRMSDQTVMLSEKLVEVSPFDSGRVFYTNSGSEANDTMVKMLWFLHRAEGKPQKRKILTLKNAYHGSTAVSASMTGLPYNSVFGLPLPGFLHLTCPHYWRYGEEGETEEQFVARLARELEETIQKEGADTIAGFFAEPVMGAGGVITPPKGYFQAILTILRKYDIPVISDEVICGFGRTGNTWGCVTYDFTPDAIISAKNLTAGFFPVGAVILGPELSKRLETAIEAIEEFDHGFTTGGHPVGCAIALKAIDVVMNEGLAENVRRLAPRFEERLKHIAERPNIGEYRGIGFMWALEAVKDKASKAPFDGNLSVGERIANTCTDLGLICRPLGQSVVLAPPYILTEAQMDEMFDKLEKALDKVFAEVA

SEQ ID NO: 141 - DNA, 1362 bp, Artificial Sequence
  Engineered variant of V. fluvialis transaminase
atgaacaaaccgcagagctgggaaacgcgtgcggaaaccgtgagcctgtatgcctttacccacatgccgagcctacgtcagcgtggcaccatggtggtgacccatggcgaaggcccgtatatcgtggatgtgcatggccgtcgttatctggatgcgaacagcggcctgtggaacatggtggcgggctttgatcataaaggcctgattgatgcggcgaaagcgcagtatgaacgttttccgggctatcatgcgttttacggccgcatgagcgatcagaccgtgatgctgtctgaaaaactggtggaagtgagcccgtttgatagcggccgtgtgtttctgaccaacagcggcagcgaagcgaacgataccatggtgaaaatgctgtggtttctgcatcgtgcggaaggcaaaccgcagaaacgtaaaattctgaccctgaagaacgcgtatcatggctccaccgcggtgagcgcgagcatgaccggccttccgtataacagcgtgtttggcctgccgctgccgggctttctgcatctgacctgcccgcattattggcgttatggcgaagaaggcgaaaccgaagaacagtttgtcgcgcgtctggcccgtgaactggaagaaaccattcagaaggaaggcgcggataccattgcgggcttttttgcggaaccggtgatgggtgcgggcggtgttattaccccgccaaaaggctattttcaggcgattctgaccatcctgcgcaaatatgatattccggtgatcagcgatgaagtgatttgcggctttggtcgtaccggcaacacctggggctgcgtgacctatgattttaccccggatgcgattattagcagtaaaaacctaaccgcgggtttttttccagtaggagcggtgattttggggccggaactgagcaaacgtctggaaaccgcgattgaagcgatcgaagaatttgatcatggttttaccacaggcggccatccggtgggttgtgcgattgcgctgaaagcgattgatgtggtgatgaacgaaggcctggccgaaaacgtgcgtcgtctggccccgcgttttgaagaacgtctgaaacatattgcggaacgtccgaacattggcgaatatcgtggtattggctttatgtgggcgctggaagccgtgaaagataaagcgagcaaagccccgtttgatggcaacctgagcgtgagcgaacgtattgcgaacacctgcaccgatctgggactgatttgccgaccgttgggccagagcgtggttctggtgccgccgtacattctgaccgaagcgcagatggatgaaatgttcgataaactggaaaaagcgctggataaagtgtttgcggaagtggcgtaa

SEQ ID NO: 142 - protein, 453 aa, Artificial Sequence
  Engineered variant of V. fluvialis transaminase
MNKPQSWETRAETVSLYAFTHMPSLRQRGTMVVTHGEGPYIVDVHGRRYLDANSGLWNMVAGFDHKGLIDAAKAQYERFPGYHAFYGRMSDQTVMLSEKLVEVSPFDSGRVFLTNSGSEANDTMVKMLWFLHRAEGKPQKRKILTLKNAYHGSTAVSASMTGLPYNSVFGLPLPGFLHLTCPHYWRYGEEGETEEQFVARLARELEETIQKEGADTIAGFFAEPVMGAGGVITPPKGYFQAILTILRKYDIPVISDEVICGFGRTGNTWGCVTYDFTPDAIISSKNLTAGFFPVGAVILGPELSKRLETAIEAIEEFDHGFTTGGHPVGCAIALKAIDVVMNEGLAENVRRLAPRFEERLKHIAERPNIGEYRGIGFMWALEAVKDKASKAPFDGNLSVSERIANTCTDLGLICRPLGQSVVLVPPYILTEAQMDEMFDKLEKALDKVFAEVA

SEQ ID NO: 143 - DNA, 1362 bp, Artificial Sequence
  Engineered variant of V. fluvialis transaminase
atgaacaaaccgcagagctgggaaacgcgtgcggaaacctatagcctgtatgcctttacccacatgccgagcctacatcagcgtggcaccatggtggtgacccatggcgaaggcccgtatatcgtggatgtgcatggccgtcgttatctggatgcgaacagcggcctgtggaacatggtggcgggctttgatcataaaggcctgattgatgcggcgaaagcgcagtatgaacgttttccgggctatcatgcgttttacggcctgatgagcgatcagaccgtgatgctgtctgaaaaactggtggaagtgagcccgtttgatagcggccgtgtgttttataccaacagcggcagcgaagcgaacgataccatggtgaaaatgctgtggtttctgcatcgtgcggaaggcaaaccgcagaaacgtaaaattctgaccctgaagaacgcgtatcatggctccaccgcggtgagcgcgagcatgaccggccttccgtataacagcgtgtttggcctgccgctgccgggctttctgcatctgacctgcccgcattattggcgttatggcgaagaaggcgaaaccgaagaacagtttgtcgcgcgtctggcccgtgaactggaagaaaccattcagaaggaaggcgcggataccattgcgggcttttttgcggaaccggtgatgggtgcgggcggtgttattaccccgccaaaaggctattttcaggcgattctgaccatcctgcgcaaatatgatattccggtgatcagcgatgaagtgatttgcggctttggtcgtaccggcaacacctggggctgcgtgacctatgattttaccccggatgcgattattagcagtaaaaacctaaccgcgggtttttttccagtaggagcggtgattttggggccggaactgagcaaacgtctggaaaccgcgattgaagcgatcgaagaatttgatcatggttttaccacaggcggccatccggtgggttgtgcgattgcgctgaaagcgattgatgtggtgatgaacgaaggcctggccgaaaacgtgcgtcgtctggccccgcgttttgaagaacgtctgaaacatattgcggaacgtccgaacattggcgaatatcgtggtattggctttatgtgggcgctggaagtggtgaaagataaagcgagcaaagccccgtttgatggcaacctgagcgtgagcgaacgtattgcgaacacctgcaccgatctgggactgatttgccgaccgttgggccagagcgtggttctggcaccgccgtacattctgaccgaagcgcagatggatgaaatgttcgataaactggaaaaagcgctggataaagtgtttgcggaagtggcgtaa

SEQ ID NO: 144 - protein, 453 aa, Artificial Sequence
  Engineered variant of V. fluvialis transaminase
MNKPQSWETRAETYSLYAFTHMPSLHQRGTMVVTHGEGPYIVDVHGRRYLDANSGLWNMVAGFDHKGLIDAAKAQYERFPGYHAFYGLMSDQTVMLSEKLVEVSPFDSGRVFYTNSGSEANDTMVKMLWFLHRAEGKPQKRKILTLKNAYHGSTAVSASMTGLPYNSVFGLPLPGFLHLTCPHYWRYGEEGETEEQFVARLARELEETIQKEGADTIAGFFAEPVMGAGGVITPPKGYFQAILTILRKYDIPVISDEVICGFGRTGNTWGCVTYDFTPDAIISSKNLTAGFFPVGAVILGPELSKRLETAIEAIEEFDHGFTTGGHPVGCAIALKAIDVVMNEGLAENVRRLAPRFEERLKHIAERPNIGEYRGIGFMWALEVVKDKASKAPFDGNLSVSERIANTCTDLGLICRPLGQSVVLAPPYILTEAQMDEMFDKLEKALDKVFAEVA

SEQ ID NO: 145 - DNA, 1362 bp, Artificial Sequence
  Engineered variant of V. fluvialis transaminase
atgaacaaaccgcagagctgggaaacgcgtgcggaaaccgtgagcctgtatgcctttacccacatgccgagcctacgtcagcgtggcaccatggtggtgacccatggcgaaggcccgtatatcgtggatgtgcatggccgtcgttatctggatgcgaacagcggcctgtggaacatggtggcgggctttgatcataaaggcctgattgatgcggcgaaagcgcagtatgaacgttttccgggctatcatgcgttttacggccgtatgagcgatcagaccgtgatgctgtctgaaaaactggtggaagtgagcccgtttgatagcggccgtgtgttttataccaacagcggcagcgaagcgaacgataccatggtgaaaatgctgtggtttctgcatcgtgcggaaggcaaaccgcagaaacgtaaaattctgaccctgaagcaggcgtatcatggctccaccgcggtgagcgcgagcatgaccggcatcccgtataacagcgtgtttggcctgccgctgccgggctttctgcatctgacctgcccgcattattggcgttatggcgaagaaggcgaaaccgaagaacagtttgtcgcgcgtctggcccgtgaactggaagaaaccattcagaaggaaggcgcggataccattgcgggcttttttgcggaaccggtgatgggtgcgggcggtgttattaccccgccaaaaggctattttcaggcgattctgaccatcctgcgcaaatatgatattccggtgatcagcgatgaagtgatttgcggctttggtcgtaccggcaacacctggggctgcgtgacctatgattttaccccggatgcgattattagcgccaaaaacctaaccgcgggtttttttccagtaggagcggtgattttggggccggaactgagcaaacgtctggaaaccgcgattgaagcgatcgaagaatttgatcatggttttaccacaggcggccatccggtgggttgtgcgattgcgctgaaagcgattgatgtggtgatgaacgaaggcctggccgaaaacgtgcgtcgtctggccccgcgttttgaagaacgtctgaaacatattgcggaacgtccgaacattggcgaatatcgtggtattggctttatgtgggcgctggaagccgtgaaagataaagcgagcaaagccccgtttgatggcaacctgagcgtgggtgaacgtattgcgaacacctgcaccgatctgggactgatttgtcgaccgctgggccagaacgtggttctggcaccgccgtacattctgaccgaagcgcagatggatgaaatgttcgataaactggaaaaagcgctggataaagtgtttgcggaagtggcgtaa

SEQ ID NO: 146 - protein, 453 aa, Artificial Sequence
  Engineered variant of V. fluvialis transaminase
MNKPQSWETRAETVSLYAFTHMPSLRQRGTMVVTHGEGPYIVDVHGRRYLDANSGLWNMVAGFDHKGLIDAAKAQYERFPGYHAFYGRMSDQTVMLSEKLVEVSPFDSGRVFYTNSGSEANDTMVKMLWFLHRAEGKPQKRKILTLKQAYHGSTAVSASMTGIPYNSVFGLPLPGFLHLTCPHYWRYGEEGETEEQFVARLARELEETIQKEGADTIAGFFAEPVMGAGGVITPPKGYFQAILTILRKYDIPVISDEVICGFGRTGNTWGCVTYDFTPDAIISAKNLTAGFFPVGAVILGPELSKRLETAIEAIEEFDHGFTTGGHPVGCAIALKAIDVVMNEGLAENVRRLAPRFEERLKHIAERPNIGEYRGIGFMWALEAVKDKASKAPFDGNLSVGERIANTCTDLGLICRPLGQNVVLAPPYILTEAQMDEMFDKLEKALDKVFAEVA

SEQ ID NO: 147 - DNA, 1362 bp, Artificial Sequence
  Engineered variant of V. fluvialis transaminase
atgaacaaaccgcagagctgggaaacgcgtgcggaaaccgtgagcctgtatgcctttacccacatgccgagcctacatcagcgtggcaccatggtgaccacccatggcgaaggcccgtatatcgtggatgtgcatggccgtcgttatctggatgcgaacagcggcctgttcaacatggtggcgggctttgatcataaaggcctgattgatgcggcgaaagcgcagtatgaacgttttccgggctatcatgcgttttacggccgtatgagcgatcagaccgtgatgctgtctgaaaaactggtggaagtgagcccgtttgatagcggccgtgtgtttctgaccaacagcggcagcgaagcgaacgataccatggtgaaaatgctgtggtttctgcatcgtgcggaaggcaaaccgcagaaacgtaaaattctgaccctgaagaacgcgtatcatggctccaccgcggtgagcgcgagcatgaccggccttccgtataacagcgtgtttggcctgccgctgccgggctttctgcatctgacctgcccgcattattggcgttatggcgaagaaggcgaaaccgaagaacagtttgtcgcgcgtctggcccgtgaactggaagaaaccattcagaaggaaggcgcggataccattgcgggcttttttgcggaaccggtgatgggtgcgggcggtgttattaccccgccaaaaggctattttcaggcgattctgaccatcctgcgcaaatatgatattccggtgatcagcgatgaagtgatttgcggctttggtcgtaccggcaacacctggggctgcgtgacctatgattttaccccggatgcgattattagcagtaaaaacctaaccgcgggtttttttccagtaggagcggtgattttggggccggaactgagcaaacgtctggaaaccgcgattgaagcgatcgaagaatttgatcatggttttaccacaggcggccatccggtgggttgtgcgattgcgctgaaagcgattgatgtggtgatgaacgaaggcctggccgaaaacgtgcgtcgtctggccccgcgttttgaagaacgtctgaaacatattgcggaacgtccgaacattggcgaatatcgtggtattggctttatgtgggcgctggaagtggtgaaagataaagcgagcaaagccccgtttgatggcaacctgagcgtgagcgaacgtattgcgaacacctgcaccgatctgggactgatttgccgaccgttgggccagagcgtggttctggcaccgccgtacattctgaccgaagcgcagatggatgaaatgttcgataaactggaaaaagcgctggataaagtgtttgcggaagtggcgtaa

SEQ ID NO: 148 - protein, 453 aa, Artificial Sequence
  Engineered variant of V. fluvialis transaminase
MNKPQSWETRAETVSLYAFTHMPSLHQRGTMVTTHGEGPYIVDVHGRRYLDANSGLFNMVAGFDHKGLIDAAKAQYERFPGYHAFYGRMSDQTVMLSEKLVEVSPFDSGRVFLTNSGSEANDTMVKMLWFLHRAEGKPQKRKILTLKNAYHGSTAVSASMTGLPYNSVFGLPLPGFLHLTCPHYWRYGEEGETEEQFVARLARELEETIQKEGADTIAGFFAEPVMGAGGVITPPKGYFQAILTILRKYDIPVISDEVICGFGRTGNTWGCVTYDFTPDAIISSKNLTAGFFPVGAVILGPELSKRLETAIEAIEEFDHGFTTGGHPVGCAIALKAIDVVMNEGLAENVRRLAPRFEERLKHIAERPNIGEYRGIGFMWALEVVKDKASKAPFDGNLSVSERIANTCTDLGLICRPLGQSVVLAPPYILTEAQMDEMFDKLEKALDKVFAEVA

SEQ ID NO: 149 - DNA, 1362 bp, Artificial Sequence
  Engineered variant of V. fluvialis transaminase
atgaacaaaccgcagagctgggaaacgcgtgcggaaaccgtgagcctgtatgcctttacccacatgccgagcctacatcagcgtggcaccatggtggtaacccatggcgaaggcccgtatatcgtggatgtgcatggccgtcgttatctggatgcgaacagcggcctgttcaacatggtggcgggctttgatcataaaggcctgattgatgcggcgaaagcgcagtatgaacgttttccgggctatcatgcgttttacggcctgatgagcgatcagaccgtgatgctgtctgaaaaactggtggaagtgagcccgtttgatagcggccgtgtgtttctgaccaacagcggcagcgaagcgaacgataccatggtgaaaatgctgtggtttctgcatcgtgcggaaggcaaaccgcagaaacgtaaaattctgaccctgaagcaggcgtatcatggctccaccgcggtgagcgcgagcatgaccggcatcccgtataacagcgtgtttggcctgccggctccgggctttctgcatctgacctgcccgcattattggcgttatggcgaagaaggcgaaaccgaagaacagtttgtcgcgcgtctggcccgtgaactggaagaaaccattcagaaggaaggcgcggataccattgcgggcttttttgcggaaccggtgatgggtgcgggcggtgttattaccccgccaaaaggctattttcaggcgattctgaccatcctgcgcaaatatgatattccggtgatcagcgatgaagtgatttgcggctttggtcgtaccggcaacacctggggctgcgtgacctatgattttaccccggatgcgattattagcagtaaaaacctaaccgcgggtttttttccagtaggagcggtgattttggggccggaactgagcaaacgtctggaaaccgcgattgaagcgatcgaagaatttgatcatggttttaccacaggcggccatccggtgggttgtgcgattgcgctgaaagcgattgatgtggtgatgaacgaaggcctggccgaaaacgtgcgtcgtctggccccgcgttttgaagaacgtctgaaacatattgcggaacgtccgaacattggcgaatatcgtggtattggctttatgtgggcgctggaagccgtgaaagataaagcgagcaaagccccgtttgatggcaacctgagcgtgggtgaacgtattgcgaacacctgcaccgatctgggactgatttgccgaccgttgggccagagcgtggttctggcaccgccgtacattctgaccgaagcgcagatggatgaaatgttcgataaactggaaaaagcgctggataaagtgtttgcggaagtggcgtaa

SEQ ID NO: 150 - protein, 453 aa, Artificial Sequence
  Engineered variant of V. fluvialis transaminase
MNKPQSWETRAETVSLYAFTHMPSLHQRGTMVVTHGEGPYIVDVHGRRYLDANSGLFNMVAGFDHKGLIDAAKAQYERFPGYHAFYGLMSDQTVMLSEKLVEVSPFDSGRVFLTNSGSEANDTMVKMLWFLHRAEGKPQKRKILTLKQAYHGSTAVSASMTGIPYNSVFGLPAPGFLHLTCPHYWRYGEEGETEEQFVARLARELEETIQKEGADTIAGFFAEPVMGAGGVITPPKGYFQAILTILRKYDIPVISDEVICGFGRTGNTWGCVTYDFTPDAIISSKNLTAGFFPVGAVILGPELSKRLETAIEAIEEFDHGFTTGGHPVGCAIALKAIDVVMNEGLAENVRRLAPRFEERLKHIAERPNIGEYRGIGFMWALEAVKDKASKAPFDGNLSVGERIANTCTDLGLICRPLGQSVVLAPPYILTEAQMDEMFDKLEKALDKVFAEVA

SEQ ID NO: 151 - DNA, 1362 bp, Artificial Sequence
  Engineered variant of V. fluvialis transaminase
atgaacaaaccgcagagctgggaaacgcgtgcggaaacctatagcctgtatgcctttacccacatgccgagcctacatcagcgtggcaccatggtggtgacccatggcgaaggcccgtatatcgtggatgtgcatggccgtcgttatctggatgcgaacagcggcctgttcaacatggtggcgggctttgatcataaaggcctgattgatgcggcgaaagcgcagtatgaacgttttccgggctatcatgcgttttacggccgtatgagcgatcagaccgtgatgctgtctgaaaaactggtggaagtgagcccgtttgatagcggccgtgtgttttataccaacagcggcagcgaagcgaacgataccatggtgaaaatgctgtggtttctgcatcgtgcggaaggcaaaccgcagaaacgtaaaattctgaccctgaagaacgcgtatcatggctccaccgcggtgagcgcgagcatgaccggccttccgtataacagcgtgtttggcctgccgctgccgggctttctgcatctgacctgcccgcattattggcgttatggcgaagaaggcgaaaccgaagaacagtttgtcgcgcgtctggcccgtgaactggaagaaaccattcagaaggaaggcgcggataccattgcgggcttttttgcggaaccggtgatgggtgcgggcggtgttattaccccgccaaaaggctattttcaggcgattctgaccatcctgcgcaaatatgatattccggtgatcagcgatgaagtgatttgcggctttggtcgtaccggcaacacctggggctgcgtgacctatgattttaccccggatgcgattattagcagtaaaaacctaaccgcgggtttttttccagtaggagcggtgattttggggccggaactgagcaaacgtctggaaaccgcgattgaagcgatcgaagaatttgatcatggttttaccacaggcggccatccggtgggttgtgcgattgcgctgaaagcgattgatgtggtgatgaacgaaggcctggccgaaaacgtgcgtcgtctggccccgcgttttgaagaacgtctgaaacatattgcggaacgtccgaacattggcgaatatcgtggtattggctttatgtgggcgctggaagtggtgaaagataaagcgagcaaagccccgtttgatggcaacctgagcgtgagcgaacgtattgcgaacacctgcaccgatctgggactgatttgccgaccgttgggccagagcgtggttctggcaccgccgtacattctgaccgaagcgcagatggatgaaatgttcgataaactggaaaaagcgctggataaagtgtttgcggaagtggcgtaa

SEQ ID NO: 152 - protein, 453 aa, Artificial Sequence
  Engineered variant of V. fluvialis transaminase
MNKPQSWETRAETYSLYAFTHMPSLHQRGTMVVTHGEGPYIVDVHGRRYLDANSGLFNMVAGFDHKGLIDAAKAQYERFPGYHAFYGRMSDQTVMLSEKLVEVSPFDSGRVFYTNSGSEANDTMVKMLWFLHRAEGKPQKRKILTLKNAYHGSTAVSASMTGLPYNSVFGLPLPGFLHLTCPHYWRYGEEGETEEQFVARLARELEETIQKEGADTIAGFFAEPVMGAGGVITPPKGYFQAILTILRKYDIPVISDEVICGFGRTGNTWGCVTYDFTPDAIISSKNLTAGFFPVGAVILGPELSKRLETAIEAIEEFDHGFTTGGHPVGCAIALKAIDVVMNEGLAENVRRLAPRFEERLKHIAERPNIGEYRGIGFMWALEVVKDKASKAPFDGNLSVSERIANTCTDLGLICRPLGQSVVLAPPYILTEAQMDEMFDKLEKALDKVFAEVA

SEQ ID NO: 153 - DNA, 1362 bp, Artificial Sequence
  Engineered variant of V. fluvialis transaminase
atgaacaaaccgcagagctgggaaacgcgtgcggaaaccgtgagcctgtatgcctttacccacatgccgagcctacgtcagcgtggcaccatggtggtgacccatggcgaaggcccgtatatcgtggatgtgcatggccgtcgttatctggatgcgaacagcggcctgtggaacatggtggcgggctttgatcataaaggcctgattgatgcggcgaaagcgcagtatgaacgttttccgggctatcatgcgttttacggccgtatgagcgatcagaccgtgatgctgtctgaaaaactggtggaagtgagcccgtttgatagcggccgtgtgttttataccaacagcggcagcgaagcgaacgataccatggtgaaaatgctgtggtttctgcatcgtgcggaaggcaaaccgcagaaacgtaaaattctgaccctgaagaacgcgtatcatggctccaccgcggtgagcgcgagcatgaccggccttccgtataacagcgtgtttggcctgccgctgccgggctttctgcatctgacctgcccgcattattggcgttatggcgaagaaggcgaaaccgaagaacagtttgtcgcgcgtctggcccgtgaactggaagaaaccattcagaaggaaggcgcggataccattgcgggcttttttgcggaaccggtgatgggtgcgggcggtgttattaccccgccaaaaggctattttcaggcgattctgaccatcctgcgcaaatatgatattccggtgatcagcgatgaagtgatttgcggctttggtcgtaccggcaacacctggggctgcgtgacctatgattttaccccggatgcgattattagcgccaaaaacctaaccgcgggtttttttccagtaggagcggtgattttggggccggaactgagcaaacgtctggaaaccgcgattgaagcgatcgaagaatttgatcatggttttaccacacacggccatccggtgggttgtgcgattgcgctgaaagcgattgatgtggtgatgaacgaaggcctggccgaaaacgtgcgtcgtctggccccgcgttttgaagaacgtctgaaacatattgcggaacgtccgaacattggcgaatatcgtggtattggctttatgtgggcgctggaagtggtgaaagataaagcgagcaaagccccgtttgatggcaacctgagcgtgggtgaacgtattgcgaacacctgcaccgatctgggactgatttgccgaccgttgggccagagcgtggttctggcaccgccgtacattctgaccgaagcgcagatggatgaaatgttcgataaactggaaaaagcgctggataaagtgtttgcggaagtggcgtaa

SEQ ID NO: 154 - protein, 453 aa, Artificial Sequence
  Engineered variant of V. fluvialis transaminase
MNKPQSWETRAETVSLYAFTHMPSLRQRGTMVVTHGEGPYIVDVHGRRYLDANSGLWNMVAGFDHKGLIDAAKAQYERFPGYHAFYGRMSDQTVMLSEKLVEVSPFDSGRVFYTNSGSEANDTMVKMLWFLHRAEGKPQKRKILTLKNAYHGSTAVSASMTGLPYNSVFGLPLPGFLHLTCPHYWRYGEEGETEEQFVARLARELEETIQKEGADTIAGFFAEPVMGAGGVITPPKGYFQAILTILRKYDIPVISDEVICGFGRTGNTWGCVTYDFTPDAIISAKNLTAGFFPVGAVILGPELSKRLETAIEAIEEFDHGFTTHGHPVGCAIALKAIDVVMNEGLAENVRRLAPRFEERLKHIAERPNIGEYRGIGFMWALEVVKDKASKAPFDGNLSVGERIANTCTDLGLICRPLGQSVVLAPPYILTEAQMDEMFDKLEKALDKVFAEVA